European Patent Application EP 4 317 174 A1, published February 7, 2024. Title: Peptide and composition comprising the peptide. Applicant: PeptiAID Inc. Japan as represented by National Institute of Infectious Diseases. The sequence listing filed with the application follows.

SEQUENCE LISTING (218 sequences)

SEQ ID NO: 1 - protein, 12 aa, Artificial Sequence
  artificial peptide
  MUTAGEN (1)..(1): Xaa stands for Ala, Glu, N-methyl-alanine or N-methyl-glutamic acid
  MUTAGEN (2)..(2): Xaa stands for N-methyl amino acid
  MUTAGEN (3)..(3): Xaa stands for Ser or alpha-methyl-alanine
  MUTAGEN (4)..(4): Xaa stands for beta-cyclohexyl-L-alanine
  MUTAGEN (5)..(5): Xaa stands for an amino acid having a side chain of unsubstituted or substituted aromatic ring
  MUTAGEN (6)..(6): Xaa stands for any amino acid
  MUTAGEN (8)..(8): Xaa stands for an amino acid having a side chain of unsubstituted or substituted aromatic ring
  MUTAGEN (9)..(9): Xaa stands for any amino acid
  MUTAGEN (10)..(10): Xaa stands for any basic amino acid
  MUTAGEN (11)..(11): Xaa stands for beta-cyclohexyl-L-alanine
XXXXXXYXXXXC

SEQ ID NO: 2 - protein, 13 aa, Artificial Sequence
  artificial peptide
  MUTAGEN (1)..(1): Xaa stands for N-methyl-alanine
  MUTAGEN (2)..(2): Xaa stands for N-methyl-phenylalanine
  MUTAGEN (4)..(4): Xaa stands for beta-cyclohexyl-L-alanine
  MUTAGEN (11)..(11): Xaa stands for beta-cyclohexyl-L-alanine
  MUTAGEN (13)..(13): Xaa stands for D-glutamic acid
  MOD_RES (13)..(13): AMIDATION
XXSXYSYYRRXCX

SEQ ID NO: 3 - protein, 12 aa, Artificial Sequence
  artificial peptide
  MUTAGEN (1)..(1): Xaa stands for N-methyl-glutamic acid
  MUTAGEN (2)..(2): Xaa stands for N-methyl-L-norleucine
  MUTAGEN (3)..(3): Xaa stands for alpha-methyl-alanine
  MUTAGEN (4)..(4): Xaa stands for beta-cyclohexyl-L-alanine
  MUTAGEN (5)..(5): Xaa stands for 4-fluoro-L-phenylalanine
  MUTAGEN (6)..(6): Xaa stands for alpha-methyl-alanine
  MUTAGEN (9)..(9): Xaa stands for 4-carboxy-L-phenylalanine
  MUTAGEN (10)..(10): Xaa stands for D-arginine
  MUTAGEN (11)..(11): Xaa stands for beta-cyclohexyl-L-alanine
  MOD_RES (12)..(12): AMIDATION
XXXXXXYYXXXC

SEQ ID NO: 4 - protein, 12 aa, Artificial Sequence
  artificial peptide
  MUTAGEN (1)..(1): Xaa stands for N-methyl-glutamic acid
  MUTAGEN (2)..(2): Xaa stands for N-methyl-L-norleucine
  MUTAGEN (3)..(3): Xaa stands for alpha-methyl-alanine
  MUTAGEN (4)..(4): Xaa stands for beta-cyclohexyl-L-alanine
  MUTAGEN (5)..(5): Xaa stands for 4-fluoro-L-phenylalanine
  MUTAGEN (6)..(6): Xaa stands for alpha-methyl-alanine
  MUTAGEN (9)..(9): Xaa stands for 4-carboxy-L-phenylalanine
  MUTAGEN (10)..(10): Xaa stands for (S)-2-amino-3-(piperidin-4-yl)propanoic acid
  MUTAGEN (11)..(11): Xaa stands for beta-cyclohexyl-L-alanine
  MOD_RES (12)..(12): AMIDATION
XXXXXXYYXXXC

SEQ ID NO: 5 - protein, 12 aa, Artificial Sequence
  artificial peptide
  MUTAGEN (1)..(1): Xaa stands for N-methyl-glutamic acid
  MUTAGEN (2)..(2): Xaa stands for N-methyl-L-norleucine
  MUTAGEN (3)..(3): Xaa stands for alpha-methyl-alanine
  MUTAGEN (4)..(4): Xaa stands for beta-cyclohexyl-L-alanine
  MUTAGEN (5)..(5): Xaa stands for 4-fluoro-L-phenylalanine
  MUTAGEN (6)..(6): Xaa stands for D-aspartic acid
  MUTAGEN (9)..(9): Xaa stands for 4-carboxy-L-phenylalanine
  MUTAGEN (10)..(10): Xaa stands for D-arginine
  MUTAGEN (11)..(11): Xaa stands for beta-cyclohexyl-L-alanine
  MOD_RES (12)..(12): AMIDATION
XXXXXXYYXXXC

SEQ ID NO: 6 - protein, 12 aa, Artificial Sequence
  artificial peptide
  MUTAGEN (1)..(1): Xaa stands for N-methyl-glutamic acid
  MUTAGEN (2)..(2): Xaa stands for N-methyl-L-norleucine
  MUTAGEN (3)..(3): Xaa stands for alpha-methyl-alanine
  MUTAGEN (4)..(4): Xaa stands for beta-cyclohexyl-L-alanine
  MUTAGEN (5)..(5): Xaa stands for 4-fluoro-L-phenylalanine
  MUTAGEN (6)..(6): Xaa stands for D-aspartic acid
  MUTAGEN (9)..(9): Xaa stands for 4-carboxy-L-phenylalanine
  MUTAGEN (10)..(10): Xaa stands for (S)-2-amino-3-(piperidin-4-yl)propanoic acid
  MUTAGEN (11)..(11): Xaa stands for beta-cyclohexyl-L-alanine
  MOD_RES (12)..(12): AMIDATION
XXXXXXYYXXXC

SEQ ID NO: 7 - protein, 12 aa, Artificial Sequence
  artificial peptide
  MUTAGEN (1)..(1): Xaa stands for N-methyl-glutamic acid
  MUTAGEN (2)..(2): Xaa stands for N-methyl-L-norleucine
  MUTAGEN (3)..(3): Xaa stands for alpha-methyl-alanine
  MUTAGEN (4)..(4): Xaa stands for beta-cyclohexyl-L-alanine
  MUTAGEN (5)..(5): Xaa stands for 4-fluoro-L-phenylalanine
  MUTAGEN (6)..(6): Xaa stands for N-methyl-glutamic acid
  MUTAGEN (9)..(9): Xaa stands for 4-carboxy-L-phenylalanine
  MUTAGEN (10)..(10): Xaa stands for D-arginine
  MUTAGEN (11)..(11): Xaa stands for beta-cyclohexyl-L-alanine
  MOD_RES (12)..(12): AMIDATION
XXXXXXYYXXXC

SEQ ID NO: 8 - protein, 12 aa, Artificial Sequence
  artificial peptide
  MUTAGEN (1)..(1): Xaa stands for N-methyl-glutamic acid
  MUTAGEN (2)..(2): Xaa stands for N-methyl-L-norleucine
  MUTAGEN (3)..(3): Xaa stands for alpha-methyl-alanine
  MUTAGEN (4)..(4): Xaa stands for beta-cyclohexyl-L-alanine
  MUTAGEN (5)..(5): Xaa stands for 4-fluoro-L-phenylalanine
  MUTAGEN (6)..(6): Xaa stands for N-methyl-glutamic acid
  MUTAGEN (8)..(8): Xaa stands for beta-(1-naphthyl)-L-alanine
  MUTAGEN (9)..(9): Xaa stands for 4-carboxy-L-phenylalanine
  MUTAGEN (10)..(10): Xaa stands for D-arginine
  MUTAGEN (11)..(11): Xaa stands for beta-cyclohexyl-L-alanine
  MOD_RES (12)..(12): AMIDATION
XXXXXXYXXXXC

SEQ ID NO: 9 - protein, 12 aa, Artificial Sequence
  artificial peptide
  MUTAGEN (1)..(1): Xaa stands for N-methyl-glutamic acid
  MUTAGEN (2)..(2): Xaa stands for N-methyl-L-norleucine
  MUTAGEN (3)..(3): Xaa stands for alpha-methyl-alanine
  MUTAGEN (4)..(4): Xaa stands for beta-cyclohexyl-L-alanine
  MUTAGEN (5)..(5): Xaa stands for 4-fluoro-L-phenylalanine
  MUTAGEN (6)..(6): Xaa stands for N-methyl-glutamic acid
  MUTAGEN (8)..(8): Xaa stands for beta-(1-naphthyl)-L-alanine
  MUTAGEN (9)..(9): Xaa stands for 4-carboxy-L-phenylalanine
  MUTAGEN (10)..(10): Xaa stands for (S)-2-amino-3-(piperidin-4-yl)propanoic acid
  MUTAGEN (11)..(11): Xaa stands for beta-cyclohexyl-L-alanine
  MOD_RES (12)..(12): AMIDATION
XXXXXXYXXXXC

SEQ ID NO: 10 - protein, 12 aa, Artificial Sequence
  artificial peptide
  MUTAGEN (1)..(1): Xaa stands for N-methyl-glutamic acid
  MUTAGEN (2)..(2): Xaa stands for N-methyl-L-norleucine
  MUTAGEN (3)..(3): Xaa stands for alpha-methyl-alanine
  MUTAGEN (4)..(4): Xaa stands for beta-cyclohexyl-L-alanine
  MUTAGEN (5)..(5): Xaa stands for 4-fluoro-L-phenylalanine
  MUTAGEN (6)..(6): Xaa stands for N-methyl-glutamic acid
  MUTAGEN (8)..(8): Xaa stands for beta-(1-naphthyl)-L-alanine
  MUTAGEN (10)..(10): Xaa stands for D-arginine
  MUTAGEN (11)..(11): Xaa stands for beta-cyclohexyl-L-alanine
  MOD_RES (12)..(12): AMIDATION
XXXXXXYXAXXC

SEQ ID NO: 11 - protein, 12 aa, Artificial Sequence
  artificial peptide
  MUTAGEN (1)..(1): Xaa stands for N-methyl-glutamic acid
  MUTAGEN (2)..(2): Xaa stands for N-methyl-L-norleucine
  MUTAGEN (3)..(3): Xaa stands for alpha-methyl-alanine
  MUTAGEN (4)..(4): Xaa stands for beta-cyclohexyl-L-alanine
  MUTAGEN (5)..(5): Xaa stands for 4-fluoro-L-phenylalanine
  MUTAGEN (6)..(6): Xaa stands for N-methyl-glutamic acid
  MUTAGEN (8)..(8): Xaa stands for beta-(1-naphthyl)-L-alanine
  MUTAGEN (10)..(10): Xaa stands for (S)-2-amino-3-(piperidin-4-yl)propanoic acid
  MUTAGEN (11)..(11): Xaa stands for beta-cyclohexyl-L-alanine
  MOD_RES (12)..(12): AMIDATION
XXXXXXYXAXXC

SEQ ID NO: 12 - protein, 12 aa, Artificial Sequence
  artificial peptide
  MUTAGEN (1)..(1): Xaa stands for N-methyl-glutamic acid
  MUTAGEN (2)..(2): Xaa stands for N-methyl-L-norleucine
  MUTAGEN (3)..(3): Xaa stands for alpha-methyl-alanine
  MUTAGEN (4)..(4): Xaa stands for beta-cyclohexyl-L-alanine
  MUTAGEN (5)..(5): Xaa stands for 4-fluoro-L-phenylalanine
  MUTAGEN (6)..(6): Xaa stands for N-methyl-glutamic acid
  MUTAGEN (9)..(9): Xaa stands for 4-carboxy-L-phenylalanine
  MUTAGEN (10)..(10): Xaa stands for (S)-2-amino-3-(piperidin-4-yl)propanoic acid
  MUTAGEN (11)..(11): Xaa stands for beta-cyclohexyl-L-alanine
  MOD_RES (12)..(12): AMIDATION
XXXXXXYYXXXC

SEQ ID NO: 13 - protein, 12 aa, Artificial Sequence
  artificial peptide
  MUTAGEN (1)..(1): Xaa stands for N-methyl-glutamic acid
  MUTAGEN (2)..(2): Xaa stands for N-methyl-L-norleucine
  MUTAGEN (3)..(3): Xaa stands for alpha-methyl-alanine
  MUTAGEN (4)..(4): Xaa stands for beta-cyclohexyl-L-alanine
  MUTAGEN (5)..(5): Xaa stands for 4-fluoro-L-phenylalanine
  MUTAGEN (6)..(6): Xaa stands for N-methyl-glutamic acid
  MUTAGEN (10)..(10): Xaa stands for D-arginine
  MUTAGEN (11)..(11): Xaa stands for beta-cyclohexyl-L-alanine
  MOD_RES (12)..(12): AMIDATION
XXXXXXYYAXXC

SEQ ID NO: 14 - protein, 12 aa, Artificial Sequence
  artificial peptide
  MUTAGEN (1)..(1): Xaa stands for N-methyl-glutamic acid
  MUTAGEN (2)..(2): Xaa stands for N-methyl-L-norleucine
  MUTAGEN (3)..(3): Xaa stands for alpha-methyl-alanine
  MUTAGEN (4)..(4): Xaa stands for beta-cyclohexyl-L-alanine
  MUTAGEN (5)..(5): Xaa stands for 4-fluoro-L-phenylalanine
  MUTAGEN (6)..(6): Xaa stands for N-methyl-glutamic acid
  MUTAGEN (10)..(10): Xaa stands for (S)-2-amino-3-(piperidin-4-yl)propanoic acid
  MUTAGEN (11)..(11): Xaa stands for beta-cyclohexyl-L-alanine
  MOD_RES (12)..(12): AMIDATION
XXXXXXYYAXXC

SEQ ID NO: 15 - protein, 13 aa, Artificial Sequence
  artificial peptide
  MUTAGEN (1)..(1): Xaa stands for N-methyl-alanine
  MUTAGEN (2)..(2): Xaa stands for N-methyl-phenylalanine
  MUTAGEN (4)..(4): Xaa stands for beta-cyclohexyl-L-alanine
  MUTAGEN (6)..(6): Xaa stands for D-aspartic acid
  MUTAGEN (9)..(9): Xaa stands for L-alpha,gamma-diamino-butyric acid
  MUTAGEN (11)..(11): Xaa stands for beta-cyclohexyl-L-alanine
  MUTAGEN (13)..(13): Xaa stands for D-glutamic acid
  MOD_RES (13)..(13): AMIDATION
XXSXYXYYXRXCX

SEQ ID NO: 16 - protein, 13 aa, Artificial Sequence
  artificial peptide
  MUTAGEN (1)..(1): Xaa stands for N-methyl-alanine
  MUTAGEN (2)..(2): Xaa stands for N-methyl-phenylalanine
  MUTAGEN (4)..(4): Xaa stands for beta-cyclohexyl-L-alanine
  MUTAGEN (6)..(6): Xaa stands for D-alpha,beta-diamino-propionic acid
  MUTAGEN (11)..(11): Xaa stands for beta-cyclohexyl-L-alanine
  MUTAGEN (13)..(13): Xaa stands for D-glutamic acid
  MOD_RES (13)..(13): AMIDATION
XXSXYXYYERXCX

SEQ ID NO: 17 - protein, 13 aa, Artificial Sequence
  artificial peptide
  MUTAGEN (1)..(1): Xaa stands for N-methyl-alanine
  MUTAGEN (2)..(2): Xaa stands for N-methyl-phenylalanine
  MUTAGEN (4)..(4): Xaa stands for beta-cyclohexyl-L-alanine
  MUTAGEN (9)..(9): Xaa stands for (S)-2-amino-heptanoic acid
  MUTAGEN (11)..(11): Xaa stands for beta-cyclohexyl-L-alanine
  MUTAGEN (13)..(13): Xaa stands for D-glutamic acid
  MOD_RES (13)..(13): AMIDATION
XXSXYKYYXRXCX

SEQ ID NO: 18 - protein, 13 aa, Artificial Sequence
  artificial peptide
  MUTAGEN (1)..(1): Xaa stands for N-methyl-glutamic acid
  MUTAGEN (2)..(2): Xaa stands for N-methyl-L-norleucine
  MUTAGEN (4)..(4): Xaa stands for beta-cyclohexyl-L-alanine
  MUTAGEN (5)..(5): Xaa stands for 4-fluoro-L-phenylalanine
  MUTAGEN (11)..(11): Xaa stands for beta-cyclohexyl-L-alanine
  MUTAGEN (13)..(13): Xaa stands for D-glutamic acid
XXSXXSYYARXCX

SEQ ID NO: 19 - protein, 13 aa, Artificial Sequence
  artificial peptide
  MUTAGEN (1)..(1): Xaa stands for N-methyl-glutamic acid
  MUTAGEN (2)..(2): Xaa stands for N-methyl-L-norleucine
  MUTAGEN (4)..(4): Xaa stands for beta-cyclohexyl-L-alanine
  MUTAGEN (5)..(5): Xaa stands for 4-fluoro-L-phenylalanine
  MUTAGEN (9)..(9): Xaa stands for 4-carboxy-L-phenylalanine
  MUTAGEN (11)..(11): Xaa stands for beta-cyclohexyl-L-alanine
  MUTAGEN (13)..(13): Xaa stands for D-glutamic acid
XXSXXSYYXRXCX

SEQ ID NO: 20 - protein, 13 aa, Artificial Sequence
  artificial peptide
  MUTAGEN (1)..(1): Xaa stands for N-methyl-glutamic acid
  MUTAGEN (2)..(2): Xaa stands for N-methyl-L-norleucine
  MUTAGEN (4)..(4): Xaa stands for beta-cyclohexyl-L-alanine
  MUTAGEN (5)..(5): Xaa stands for 4-fluoro-L-phenylalanine
  MUTAGEN (9)..(9): Xaa stands for (S)-2-amino-5-ureidopentanoic acid
  MUTAGEN (11)..(11): Xaa stands for beta-cyclohexyl-L-alanine
  MUTAGEN (13)..(13): Xaa stands for D-glutamic acid
XXSXXSYYXRXCX

SEQ ID NO: 21 - protein, 13 aa, Artificial Sequence
  artificial peptide
  MUTAGEN (1)..(1): Xaa stands for N-methyl-glutamic acid
  MUTAGEN (2)..(2): Xaa stands for N-methyl-L-norleucine
  MUTAGEN (3)..(3): Xaa stands for alpha-methyl-alanine
  MUTAGEN (4)..(4): Xaa stands for beta-cyclohexyl-L-alanine
  MUTAGEN (5)..(5): Xaa stands for 4-fluoro-L-phenylalanine
  MUTAGEN (6)..(6): Xaa stands for alpha-methyl-alanine
  MUTAGEN (9)..(9): Xaa stands for 4-carboxy-L-phenylalanine
  MUTAGEN (10)..(10): Xaa stands for D-arginine
  MUTAGEN (11)..(11): Xaa stands for beta-cyclohexyl-L-alanine
  MUTAGEN (13)..(13): Xaa stands for D-glutamic acid
  MOD_RES (13)..(13): AMIDATION
XXXXXXYYXXXCX

SEQ ID NO: 22 - protein, 13 aa, Artificial Sequence
  artificial peptide
  MUTAGEN (1)..(1): Xaa stands for N-methyl-glutamic acid
  MUTAGEN (2)..(2): Xaa stands for N-methyl-L-norleucine
  MUTAGEN (3)..(3): Xaa stands for alpha-methyl-alanine
  MUTAGEN (4)..(4): Xaa stands for beta-cyclohexyl-L-alanine
  MUTAGEN (5)..(5): Xaa stands for 4-fluoro-L-phenylalanine
  MUTAGEN (6)..(6): Xaa stands for alpha-methyl-alanine
  MUTAGEN (9)..(9): Xaa stands for 4-carboxy-L-phenylalanine
  MUTAGEN (10)..(10): Xaa stands for (S)-2-amino-3-(piperidin-4-yl)propanoic acid
  MUTAGEN (11)..(11): Xaa stands for beta-cyclohexyl-L-alanine
  MUTAGEN (13)..(13): Xaa stands for D-glutamic acid
  MOD_RES (13)..(13): AMIDATION
XXXXXXYYXXXCX

SEQ ID NO: 23 - protein, 13 aa, Artificial Sequence
  artificial peptide
  MUTAGEN (1)..(1): Xaa stands for N-methyl-glutamic acid
  MUTAGEN (2)..(2): Xaa stands for N-methyl-L-norleucine
  MUTAGEN (3)..(3): Xaa stands for alpha-methyl-alanine
  MUTAGEN (4)..(4): Xaa stands for beta-cyclohexyl-L-alanine
  MUTAGEN (5)..(5): Xaa stands for 4-fluoro-L-phenylalanine
  MUTAGEN (6)..(6): Xaa stands for D-aspartic acid
  MUTAGEN (8)..(8): Xaa stands for beta-(1-naphthyl)-L-alanine
  MUTAGEN (9)..(9): Xaa stands for (S)-2-amino-5-ureidopentanoic acid
  MUTAGEN (10)..(10): Xaa stands for D-arginine
  MUTAGEN (11)..(11): Xaa stands for beta-cyclohexyl-L-alanine
  MUTAGEN (13)..(13): Xaa stands for D-glutamic acid
XXXXXXYXXXXCX

SEQ ID NO: 24 - protein, 13 aa, Artificial Sequence
  artificial peptide
  MUTAGEN (1)..(1): Xaa stands for N-methyl-glutamic acid
  MUTAGEN (2)..(2): Xaa stands for N-methyl-L-norleucine
  MUTAGEN (3)..(3): Xaa stands for alpha-methyl-alanine
  MUTAGEN (4)..(4): Xaa stands for beta-cyclohexyl-L-alanine
  MUTAGEN (5)..(5): Xaa stands for 4-fluoro-L-phenylalanine
  MUTAGEN (6)..(6): Xaa stands for D-aspartic acid
  MUTAGEN (8)..(8): Xaa stands for beta-(1-naphthyl)-L-alanine
  MUTAGEN (9)..(9): Xaa stands for (S)-2-amino-5-ureidopentanoic acid
  MUTAGEN (10)..(10): Xaa stands for D-lysine
  MUTAGEN (11)..(11): Xaa stands for beta-cyclohexyl-L-alanine
  MUTAGEN (13)..(13): Xaa stands for D-glutamic acid
XXXXXXYXXXXCX

SEQ ID NO: 25 - protein, 13 aa, Artificial Sequence
  artificial peptide
  MUTAGEN (1)..(1): Xaa stands for N-methyl-glutamic acid
  MUTAGEN (2)..(2): Xaa stands for N-methyl-L-norleucine
  MUTAGEN (3)..(3): Xaa stands for alpha-methyl-alanine
  MUTAGEN (4)..(4): Xaa stands for beta-cyclohexyl-L-alanine
  MUTAGEN (5)..(5): Xaa stands for 4-fluoro-L-phenylalanine
  MUTAGEN (6)..(6): Xaa stands for D-aspartic acid
  MUTAGEN (8)..(8): Xaa stands for beta-(1-naphthyl)-L-alanine
  MUTAGEN (10)..(10): Xaa stands for D-arginine
  MUTAGEN (11)..(11): Xaa stands for beta-cyclohexyl-L-alanine
  MUTAGEN (13)..(13): Xaa stands for D-glutamic acid
XXXXXXYXKXXCX

SEQ ID NO: 26 - protein, 13 aa, Artificial Sequence
  artificial peptide
  MUTAGEN (1)..(1): Xaa stands for N-methyl-glutamic acid
  MUTAGEN (2)..(2): Xaa stands for N-methyl-L-norleucine
  MUTAGEN (3)..(3): Xaa stands for alpha-methyl-alanine
  MUTAGEN (4)..(4): Xaa stands for beta-cyclohexyl-L-alanine
  MUTAGEN (5)..(5): Xaa stands for 4-fluoro-L-phenylalanine
  MUTAGEN (6)..(6): Xaa stands for D-aspartic acid
  MUTAGEN (8)..(8): Xaa stands for beta-(1-naphthyl)-L-alanine
  MUTAGEN (10)..(10): Xaa stands for D-lysine
  MUTAGEN (11)..(11): Xaa stands for beta-cyclohexyl-L-alanine
  MUTAGEN (13)..(13): Xaa stands for D-glutamic acid
XXXXXXYXKXXCX

SEQ ID NO: 27 - protein, 13 aa, Artificial Sequence
  artificial peptide
  MUTAGEN (1)..(1): Xaa stands for N-methyl-glutamic acid
  MUTAGEN (2)..(2): Xaa stands for N-methyl-L-norleucine
  MUTAGEN (3)..(3): Xaa stands for alpha-methyl-alanine
  MUTAGEN (4)..(4): Xaa stands for beta-cyclohexyl-L-alanine
  MUTAGEN (5)..(5): Xaa stands for 4-fluoro-L-phenylalanine
  MUTAGEN (6)..(6): Xaa stands for D-aspartic acid
  MUTAGEN (9)..(9): Xaa stands for 4-carboxy-L-phenylalanine
  MUTAGEN (10)..(10): Xaa stands for D-arginine
  MUTAGEN (11)..(11): Xaa stands for beta-cyclohexyl-L-alanine
  MUTAGEN (13)..(13): Xaa stands for D-glutamic acid
  MOD_RES (13)..(13): AMIDATION
XXXXXXYYXXXCX

SEQ ID NO: 28 - protein, 13 aa, Artificial Sequence
  artificial peptide
  MUTAGEN (1)..(1): Xaa stands for N-methyl-glutamic acid
  MUTAGEN (2)..(2): Xaa stands for N-methyl-L-norleucine
  MUTAGEN (3)..(3): Xaa stands for alpha-methyl-alanine
  MUTAGEN (4)..(4): Xaa stands for beta-cyclohexyl-L-alanine
  MUTAGEN (5)..(5): Xaa stands for 4-fluoro-L-phenylalanine
  MUTAGEN (6)..(6): Xaa stands for D-aspartic acid
  MUTAGEN (9)..(9): Xaa stands for 4-carboxy-L-phenylalanine
  MUTAGEN (10)..(10): Xaa stands for (S)-2-amino-3-(piperidin-4-yl)propanoic acid
  MUTAGEN (11)..(11): Xaa stands for beta-cyclohexyl-L-alanine
  MUTAGEN (13)..(13): Xaa stands for D-glutamic acid
  MOD_RES (13)..(13): AMIDATION
XXXXXXYYXXXCX

SEQ ID NO: 29 - protein, 13 aa, Artificial Sequence
  artificial peptide
  MUTAGEN (1)..(1): Xaa stands for N-methyl-glutamic acid
  MUTAGEN (2)..(2): Xaa stands for N-methyl-L-norleucine
  MUTAGEN (3)..(3): Xaa stands for alpha-methyl-alanine
  MUTAGEN (4)..(4): Xaa stands for beta-cyclohexyl-L-alanine
  MUTAGEN (5)..(5): Xaa stands for 4-fluoro-L-phenylalanine
  MUTAGEN (6)..(6): Xaa stands for D-aspartic acid
  MUTAGEN (9)..(9): Xaa stands for (S)-2-amino-5-ureidopentanoic acid
  MUTAGEN (10)..(10): Xaa stands for D-arginine
  MUTAGEN (11)..(11): Xaa stands for beta-cyclohexyl-L-alanine
  MUTAGEN (13)..(13): Xaa stands for D-glutamic acid
XXXXXXYYXXXCX

SEQ ID NO: 30 - protein, 13 aa, Artificial Sequence
  artificial peptide
  MUTAGEN (1)..(1): Xaa stands for N-methyl-glutamic acid
  MUTAGEN (2)..(2): Xaa stands for N-methyl-L-norleucine
  MUTAGEN (3)..(3): Xaa stands for alpha-methyl-alanine
  MUTAGEN (4)..(4): Xaa stands for beta-cyclohexyl-L-alanine
  MUTAGEN (5)..(5): Xaa stands for 4-fluoro-L-phenylalanine
  MUTAGEN (6)..(6): Xaa stands for D-aspartic acid
  MUTAGEN (9)..(9): Xaa stands for (S)-2-amino-5-ureidopentanoic acid
  MUTAGEN (10)..(10): Xaa stands for D-lysine
  MUTAGEN (11)..(11): Xaa stands for beta-cyclohexyl-L-alanine
  MUTAGEN (13)..(13): Xaa stands for D-glutamic acid
XXXXXXYYXXXCX

SEQ ID NO: 31 - protein, 13 aa, Artificial Sequence
  artificial peptide
  MUTAGEN (1)..(1): Xaa stands for N-methyl-glutamic acid
  MUTAGEN (2)..(2): Xaa stands for N-methyl-L-norleucine
  MUTAGEN (3)..(3): Xaa stands for alpha-methyl-alanine
  MUTAGEN (4)..(4): Xaa stands for beta-cyclohexyl-L-alanine
  MUTAGEN (5)..(5): Xaa stands for 4-fluoro-L-phenylalanine
  MUTAGEN (6)..(6): Xaa stands for N-methyl-glutamic acid
  MUTAGEN (8)..(8): Xaa stands for beta-(1-naphthyl)-L-alanine
  MUTAGEN (10)..(10): Xaa stands for D-arginine
  MUTAGEN (11)..(11): Xaa stands for beta-cyclohexyl-L-alanine
  MUTAGEN (13)..(13): Xaa stands for D-glutamic acid
  MOD_RES (13)..(13): AMIDATION
XXXXXXYXAXXCX

SEQ ID NO: 32 - protein, 13 aa, Artificial Sequence
  artificial peptide
  MUTAGEN (1)..(1): Xaa stands for N-methyl-glutamic acid
  MUTAGEN (2)..(2): Xaa stands for N-methyl-L-norleucine
  MUTAGEN (3)..(3): Xaa stands for alpha-methyl-alanine
  MUTAGEN (4)..(4): Xaa stands for beta-cyclohexyl-L-alanine
  MUTAGEN (5)..(5): Xaa stands for 4-fluoro-L-phenylalanine
  MUTAGEN (6)..(6): Xaa stands for N-methyl-glutamic acid
  MUTAGEN (8)..(8): Xaa stands for beta-(1-naphthyl)-L-alanine
  MUTAGEN (10)..(10): Xaa stands for (S)-2-amino-3-(piperidin-4-yl)propanoic acid
  MUTAGEN (11)..(11): Xaa stands for beta-cyclohexyl-L-alanine
  MUTAGEN (13)..(13): Xaa stands for D-glutamic acid
  MOD_RES (13)..(13): AMIDATION
XXXXXXYXAXXCX

SEQ ID NO: 33 - protein, 13 aa, Artificial Sequence
  artificial peptide
  MUTAGEN (1)..(1): Xaa stands for N-methyl-glutamic acid
  MUTAGEN (2)..(2): Xaa stands for N-methyl-L-norleucine
  MUTAGEN (3)..(3): Xaa stands for alpha-methyl-alanine
  MUTAGEN (4)..(4): Xaa stands for beta-cyclohexyl-L-alanine
  MUTAGEN (5)..(5): Xaa stands for 4-fluoro-L-phenylalanine
  MUTAGEN (6)..(6): Xaa stands for N-methyl-glutamic acid
  MUTAGEN (8)..(8): Xaa stands for beta-(1-naphthyl)-L-alanine
  MUTAGEN (9)..(9): Xaa stands for 4-carboxy-L-phenylalanine
  MUTAGEN (10)..(10): Xaa stands for D-arginine
  MUTAGEN (11)..(11): Xaa stands for beta-cyclohexyl-L-alanine
  MUTAGEN (13)..(13): Xaa stands for D-glutamic acid
  MOD_RES (13)..(13): AMIDATION
XXXXXXYXXXXCX

SEQ ID NO: 34 - protein, 13 aa, Artificial Sequence
  artificial peptide
  MUTAGEN (1)..(1): Xaa stands for N-methyl-glutamic acid
  MUTAGEN (2)..(2): Xaa stands for N-methyl-L-norleucine
  MUTAGEN (3)..(3): Xaa stands for alpha-methyl-alanine
  MUTAGEN (4)..(4): Xaa stands for beta-cyclohexyl-L-alanine
  MUTAGEN (5)..(5): Xaa stands for 4-fluoro-L-phenylalanine
  MUTAGEN (6)..(6): Xaa stands for N-methyl-glutamic acid
  MUTAGEN (8)..(8): Xaa stands for beta-(1-naphthyl)-L-alanine
  MUTAGEN (9)..(9): Xaa stands for 4-carboxy-L-phenylalanine
  MUTAGEN (10)..(10): Xaa stands for (S)-2-amino-3-(piperidin-4-yl)propanoic acid
  MUTAGEN (11)..(11): Xaa stands for beta-cyclohexyl-L-alanine
  MUTAGEN (13)..(13): Xaa stands for D-glutamic acid
  MOD_RES (13)..(13): AMIDATION
XXXXXXYXXXXCX

SEQ ID NO: 35 - protein, 13 aa, Artificial Sequence
  artificial peptide
  MUTAGEN (1)..(1): Xaa stands for N-methyl-glutamic acid
  MUTAGEN (2)..(2): Xaa stands for N-methyl-L-norleucine
  MUTAGEN (3)..(3): Xaa stands for alpha-methyl-alanine
  MUTAGEN (4)..(4): Xaa stands for beta-cyclohexyl-L-alanine
  MUTAGEN (5)..(5): Xaa stands for 4-fluoro-L-phenylalanine
  MUTAGEN (6)..(6): Xaa stands for N-methyl-glutamic acid
  MUTAGEN (8)..(8): Xaa stands for beta-(1-naphthyl)-L-alanine
  MUTAGEN (10)..(10): Xaa stands for D-arginine
  MUTAGEN (11)..(11): Xaa stands for beta-cyclohexyl-L-alanine
  MUTAGEN (13)..(13): Xaa stands for D-glutamic acid
XXXXXXYXKXXCX

SEQ ID NO: 36 - protein, 13 aa, Artificial Sequence
  artificial peptide
  MUTAGEN (1)..(1): Xaa stands for N-methyl-glutamic acid
  MUTAGEN (2)..(2): Xaa stands for N-methyl-L-norleucine
  MUTAGEN (3)..(3): Xaa stands for alpha-methyl-alanine
  MUTAGEN (4)..(4): Xaa stands for beta-cyclohexyl-L-alanine
  MUTAGEN (5)..(5): Xaa stands for 4-fluoro-L-phenylalanine
  MUTAGEN (6)..(6): Xaa stands for N-methyl-glutamic acid
  MUTAGEN (8)..(8): Xaa stands for beta-(1-naphthyl)-L-alanine
  MUTAGEN (9)..(9): Xaa stands for (S)-2-amino-5-ureidopentanoic acid
  MUTAGEN (10)..(10): Xaa stands for D-arginine
  MUTAGEN (11)..(11): Xaa stands for beta-cyclohexyl-L-alanine
  MUTAGEN (13)..(13): Xaa stands for D-glutamic acid
XXXXXXYXXXXCX

SEQ ID NO: 37 - protein, 13 aa, Artificial Sequence
  artificial peptide
  MUTAGEN (1)..(1): Xaa stands for N-methyl-glutamic acid
  MUTAGEN (2)..(2): Xaa stands for N-methyl-L-norleucine
  MUTAGEN (3)..(3): Xaa stands for alpha-methyl-alanine
  MUTAGEN (4)..(4): Xaa stands for beta-cyclohexyl-L-alanine
  MUTAGEN (5)..(5): Xaa stands for 4-fluoro-L-phenylalanine
  MUTAGEN (6)..(6): Xaa stands for N-methyl-glutamic acid
  MUTAGEN (11)..(11): Xaa stands for beta-cyclohexyl-L-alanine
  MUTAGEN (13)..(13): Xaa stands for D-glutamic acid
XXXXXXYYARXCX

SEQ ID NO: 38 - protein, 13 aa, Artificial Sequence
  artificial peptide
  MUTAGEN (1)..(1): Xaa stands for N-methyl-glutamic acid
  MUTAGEN (2)..(2): Xaa stands for N-methyl-L-norleucine
  MUTAGEN (3)..(3): Xaa stands for alpha-methyl-alanine
  MUTAGEN (4)..(4): Xaa stands for beta-cyclohexyl-L-alanine
  MUTAGEN (5)..(5): Xaa stands for 4-fluoro-L-phenylalanine
  MUTAGEN (6)..(6): Xaa stands for N-methyl-glutamic acid
  MUTAGEN (10)..(10): Xaa stands for D-arginine
  MUTAGEN (11)..(11): Xaa stands for beta-cyclohexyl-L-alanine
  MUTAGEN (13)..(13): Xaa stands for D-glutamic acid
  MOD_RES (13)..(13): AMIDATION
XXXXXXYYAXXCX

SEQ ID NO: 39 - protein, 13 aa, Artificial Sequence
  artificial peptide
  MUTAGEN (1)..(1): Xaa stands for N-methyl-glutamic acid
  MUTAGEN (2)..(2): Xaa stands for N-methyl-L-norleucine
  MUTAGEN (3)..(3): Xaa stands for alpha-methyl-alanine
  MUTAGEN (4)..(4): Xaa stands for beta-cyclohexyl-L-alanine
  MUTAGEN (5)..(5): Xaa stands for 4-fluoro-L-phenylalanine
  MUTAGEN (6)..(6): Xaa stands for N-methyl-glutamic acid
  MUTAGEN (10)..(10): Xaa stands for (S)-2-amino-3-(piperidin-4-yl)propanoic acidd
  MUTAGEN (11)..(11): Xaa stands for beta-cyclohexyl-L-alanine
  MUTAGEN (13)..(13): Xaa stands for D-glutamic acid
  MOD_RES (13)..(13): AMIDATION
XXXXXXYYAXXCX

SEQ ID NO: 40 - protein, 13 aa, Artificial Sequence
  artificial peptide
  MUTAGEN (1)..(1): Xaa stands for N-methyl-glutamic acid
  MUTAGEN (2)..(2): Xaa stands for N-methyl-L-norleucine
  MUTAGEN (3)..(3): Xaa stands for alpha-methyl-alanine
  MUTAGEN (4)..(4): Xaa stands for beta-cyclohexyl-L-alanine
  MUTAGEN (5)..(5): Xaa stands for 4-fluoro-L-phenylalanine
  MUTAGEN (6)..(6): Xaa stands for N-methyl-glutamic acid
  MUTAGEN (9)..(9): Xaa stands for 4-carboxy-L-phenylalanine
  MUTAGEN (11)..(11): Xaa stands for beta-cyclohexyl-L-alanine
  MUTAGEN (13)..(13): Xaa stands for D-glutamic acid
XXXXXXYYXRXCX

SEQ ID NO: 41 - protein, 13 aa, Artificial Sequence
  artificial peptide
  MUTAGEN (1)..(1): Xaa stands for N-methyl-glutamic acid
  MUTAGEN (2)..(2): Xaa stands for N-methyl-L-norleucine
  MUTAGEN (3)..(3): Xaa stands for alpha-methyl-alanine
  MUTAGEN (4)..(4): Xaa stands for beta-cyclohexyl-L-alanine
  MUTAGEN (5)..(5): Xaa stands for 4-fluoro-L-phenylalanine
  MUTAGEN (6)..(6): Xaa stands for N-methyl-glutamic acid
  MUTAGEN (9)..(9): Xaa stands for 4-carboxy-L-phenylalanine
  MUTAGEN (10)..(10): Xaa stands for D-arginine
  MUTAGEN (11)..(11): Xaa stands for beta-cyclohexyl-L-alanine
  MUTAGEN (13)..(13): Xaa stands for D-glutamic acid
  MOD_RES (13)..(13): AMIDATION
XXXXXXYYXXXCX

SEQ ID NO: 42 - protein, 13 aa, Artificial Sequence
  artificial peptide
  MUTAGEN (1)..(1): Xaa stands for N-methyl-glutamic acid
  MUTAGEN (2)..(2): Xaa stands for N-methyl-L-norleucine
  MUTAGEN (3)..(3): Xaa stands for alpha-methyl-alanine
  MUTAGEN (4)..(4): Xaa stands for beta-cyclohexyl-L-alanine
  MUTAGEN (5)..(5): Xaa stands for 4-fluoro-L-phenylalanine
  MUTAGEN (6)..(6): Xaa stands for N-methyl-glutamic acid
  MUTAGEN (9)..(9): Xaa stands for 4-carboxy-L-phenylalanine
  MUTAGEN (10)..(10): Xaa stands for (S)-2-amino-3-(piperidin-4-yl)propanoic acid
  MUTAGEN (11)..(11): Xaa stands for beta-cyclohexyl-L-alanine
  MUTAGEN (13)..(13): Xaa stands for D-glutamic acid
  MOD_RES (13)..(13): AMIDATION
XXXXXXYYXXXCX

SEQ ID NO: 43 - protein, 13 aa, Artificial Sequence
  artificial peptide
  MUTAGEN (1)..(1): Xaa stands for N-methyl-glutamic acid
  MUTAGEN (2)..(2): Xaa stands for N-methyl-L-norleucine
  MUTAGEN (3)..(3): Xaa stands for alpha-methyl-alanine
  MUTAGEN (4)..(4): Xaa stands for beta-cyclohexyl-L-alanine
  MUTAGEN (5)..(5): Xaa stands for 4-fluoro-L-phenylalanine
  MUTAGEN (6)..(6): Xaa stands for N-methyl-glutamic acid
  MUTAGEN (9)..(9): Xaa stands for (S)-2-amino-5-ureidopentanoic acid
  MUTAGEN (11)..(11): Xaa stands for beta-cyclohexyl-L-alanine
  MUTAGEN (13)..(13): Xaa stands for D-glutamic acid
XXXXXXYYXRXCX

SEQ ID NO: 44 - protein, 13 aa, Artificial Sequence
  artificial peptide
  MUTAGEN (1)..(1): Xaa stands for N-methyl-glutamic acid
  MUTAGEN (2)..(2): Xaa stands for N-methyl-L-norleucine
  MUTAGEN (3)..(3): Xaa stands for alpha-methyl-alanine
  MUTAGEN (4)..(4): Xaa stands for beta-cyclohexyl-L-alanine
  MUTAGEN (5)..(5): Xaa stands for 4-fluoro-L-phenylalanine
  MUTAGEN (6)..(6): Xaa stands for N-methyl-glutamic acid
  MUTAGEN (9)..(9): Xaa stands for (S)-2-amino-5-ureidopentanoic acid
  MUTAGEN (10)..(10): Xaa stands for D-arginine
  MUTAGEN (11)..(11): Xaa stands for beta-cyclohexyl-L-alanine
  MUTAGEN (13)..(13): Xaa stands for D-glutamic acid
XXXXXXYYXXXCX

SEQ ID NO: 45 - protein, 13 aa, Artificial Sequence
  artificial peptide
  MUTAGEN (1)..(1): Xaa stands for N-methyl-glutamic acid
  MUTAGEN (2)..(2): Xaa stands for N-methyl-L-norleucine
  MUTAGEN (3)..(3): Xaa stands for alpha-methyl-alanine
  MUTAGEN (4)..(4): Xaa stands for beta-cyclohexyl-L-alanine
  MUTAGEN (5)..(5): Xaa stands for 4-fluoro-L-phenylalanine
  MUTAGEN (6)..(6): Xaa stands for N-methyl-glutamic acid
  MUTAGEN (9)..(9): Xaa stands for (S)-2-amino-5-ureidopentanoic acid
  MUTAGEN (10)..(10): Xaa stands for D-lysine
  MUTAGEN (11)..(11): Xaa stands for beta-cyclohexyl-L-alanine
  MUTAGEN (13)..(13): Xaa stands for D-glutamic acid
XXXXXXYYXXXCX

SEQ ID NO: 46 - protein, 13 aa, Artificial Sequence
  artificial peptide
  MUTAGEN (1)..(1): Xaa stands for N-methyl-glutamic acid
  MUTAGEN (2)..(2): Xaa stands for N-methyl-L-norleucine
  MUTAGEN (3)..(3): Xaa stands for alpha-methyl-alanine
  MUTAGEN (4)..(4): Xaa stands for beta-cyclohexyl-L-alanine
  MUTAGEN (5)..(5): Xaa stands for 4-fluoro-L-phenylalanine
  MUTAGEN (6)..(6): Xaa stands for N-methyl-glutamic acid
  MUTAGEN (8)..(8): Xaa stands for beta-(1-naphthyl)-L-alanine
  MUTAGEN (10)..(10): Xaa stands for D-lysine
  MUTAGEN (11)..(11): Xaa stands for beta-cyclohexyl-L-alanine
  MUTAGEN (13)..(13): Xaa stands for D-glutamic acid
XXXXXXYXKXXCX

SEQ ID NO: 47 - protein, 13 aa, Artificial Sequence
  artificial peptide
  MUTAGEN (1)..(1): Xaa stands for N-methyl-glutamic acid
  MUTAGEN (2)..(2): Xaa stands for N-methyl-L-norleucine
  MUTAGEN (3)..(3): Xaa stands for alpha-methyl-alanine
  MUTAGEN (4)..(4): Xaa stands for beta-cyclohexyl-L-alanine
  MUTAGEN (5)..(5): Xaa stands for 4-fluoro-L-phenylalanine
  MUTAGEN (6)..(6): Xaa stands for N-methyl-glutamic acid
  MUTAGEN (8)..(8): Xaa stands for beta-(1-naphthyl)-L-alanine
  MUTAGEN (9)..(9): Xaa stands for (S)-2-amino-5-ureidopentanoic acid
  MUTAGEN (10)..(10): Xaa stands for D-lysine
  MUTAGEN (11)..(11): Xaa stands for beta-cyclohexyl-L-alanine
  MUTAGEN (13)..(13): Xaa stands for D-glutamic acid
XXXXXXYXXXXCX

SEQ ID NO: 48 - protein, 13 aa, Artificial Sequence
  artificial peptide
  MUTAGEN (1)..(1): Xaa stands for N-methyl-glutamic acid
  MUTAGEN (2)..(2): Xaa stands for N-methyl-phenylalanine
  MUTAGEN (4)..(4): Xaa stands for beta-cyclohexyl-L-alanine
  MUTAGEN (5)..(5): Xaa stands for 4-fluoro-L-phenylalanine
  MUTAGEN (6)..(6): Xaa stands for alpha-methyl-alanine
  MUTAGEN (8)..(8): Xaa stands for beta-(1-naphthyl)-L-alanine
  MUTAGEN (11)..(11): Xaa stands for beta-cyclohexyl-L-alanine
  MUTAGEN (13)..(13): Xaa stands for D-glutamic acid
XXSXXXYXARXCX

SEQ ID NO: 49 - protein, 13 aa, Artificial Sequence
  artificial peptide
  MUTAGEN (1)..(1): Xaa stands for N-methyl-glutamic acid
  MUTAGEN (2)..(2): Xaa stands for N-methyl-phenylalanine
  MUTAGEN (4)..(4): Xaa stands for beta-cyclohexyl-L-alanine
  MUTAGEN (5)..(5): Xaa stands for 4-fluoro-L-phenylalanine
  MUTAGEN (6)..(6): Xaa stands for alpha-methyl-alanine
  MUTAGEN (8)..(8): Xaa stands for beta-(1-naphthyl)-L-alanine
  MUTAGEN (9)..(9): Xaa stands for (S)-2-amino-5-ureidopentanoic acid
  MUTAGEN (11)..(11): Xaa stands for beta-cyclohexyl-L-alanine
  MUTAGEN (13)..(13): Xaa stands for D-glutamic acid
XXSXXXYXXRXCX

SEQ ID NO: 50 - protein, 13 aa, Artificial Sequence
  artificial peptide
  MUTAGEN (1)..(1): Xaa stands for N-methyl-glutamic acid
  MUTAGEN (2)..(2): Xaa stands for N-methyl- phenylalanine
  MUTAGEN (4)..(4): Xaa stands for beta-cyclohexyl-L-alanine
  MUTAGEN (5)..(5): Xaa stands for 4-fluoro-L-phenylalanine
  MUTAGEN (6)..(6): Xaa stands for alpha-methyl-alanine
  MUTAGEN (11)..(11): Xaa stands for beta-cyclohexyl-L-alanine
  MUTAGEN (13)..(13): Xaa stands for D-glutamic acid
XXSXXXYYARXCX

SEQ ID NO: 51 - protein, 13 aa, Artificial Sequence
  artificial peptide
  MUTAGEN (1)..(1): Xaa stands for N-methyl-glutamic acid
  MUTAGEN (2)..(2): Xaa stands for N-methyl-phenylalanine
  MUTAGEN (4)..(4): Xaa stands for beta-cyclohexyl-L-alanine
  MUTAGEN (5)..(5): Xaa stands for 4-fluoro-L-phenylalanine
  MUTAGEN (6)..(6): Xaa stands for alpha-methyl-alanine
  MUTAGEN (9)..(9): Xaa stands for 4-carboxy-L-phenylalanine
  MUTAGEN (11)..(11): Xaa stands for beta-cyclohexyl-L-alanine
  MUTAGEN (13)..(13): Xaa stands for D-glutamic acid
XXSXXXYYXRXCX

SEQ ID NO: 52 - protein, 13 aa, Artificial Sequence
  artificial peptide
  MUTAGEN (1)..(1): Xaa stands for N-methyl-glutamic acid
  MUTAGEN (2)..(2): Xaa stands for N-methyl-phenylalanine
  MUTAGEN (4)..(4): Xaa stands for beta-cyclohexyl-L-alanine
  MUTAGEN (5)..(5): Xaa stands for 4-fluoro-L-phenylalanine
  MUTAGEN (6)..(6): Xaa stands for alpha-methyl-alanine
  MUTAGEN (9)..(9): Xaa stands for (S)-2-amino-5-ureidopentanoic acid
  MUTAGEN (11)..(11): Xaa stands for beta-cyclohexyl-L-alanine
  MUTAGEN (13)..(13): Xaa stands for D-glutamic acid
XXSXXXYYXRXCX

SEQ ID NO: 53 - protein, 13 aa, Artificial Sequence
  artificial peptide
  MUTAGEN (1)..(1): Xaa stands for N-methyl-glutamic acid
  MUTAGEN (2)..(2): Xaa stands for N-methyl-phenylalanine
  MUTAGEN (4)..(4): Xaa stands for beta-cyclohexyl-L-alanine
  MUTAGEN (5)..(5): Xaa stands for 4-fluoro-L-phenylalanine
  MUTAGEN (8)..(8): Xaa stands for beta-(1-naphthyl)-L-alanine
  MUTAGEN (11)..(11): Xaa stands for beta-cyclohexyl-L-alanine
  MUTAGEN (13)..(13): Xaa stands for D-glutamic acid
XXSXXEYXARXCX

SEQ ID NO: 54 - protein, 13 aa, Artificial Sequence
  artificial peptide
  MUTAGEN (1)..(1): Xaa stands for N-methyl-glutamic acid
  MUTAGEN (2)..(2): Xaa stands for N-methyl-phenylalanine
  MUTAGEN (4)..(4): Xaa stands for beta-cyclohexyl-L-alanine
  MUTAGEN (5)..(5): Xaa stands for 4-fluoro-L-phenylalanine
  MUTAGEN (8)..(8): Xaa stands for beta-(1-naphthyl)-L-alanine
  MUTAGEN (9)..(9): Xaa stands for (S)-2-amino-5-ureidopentanoic acid
  MUTAGEN (11)..(11): Xaa stands for beta-cyclohexyl-L-alanine
  MUTAGEN (13)..(13): Xaa stands for D-glutamic acid
XXSXXEYXXRXCX

SEQ ID NO: 55 - protein, 13 aa, Artificial Sequence
  artificial peptide
  MUTAGEN (1)..(1): Xaa stands for N-methyl-glutamic acid
  MUTAGEN (2)..(2): Xaa stands for N-methyl-phenylalanine
  MUTAGEN (4)..(4): Xaa stands for beta-cyclohexyl-L-alanine
  MUTAGEN (5)..(5): Xaa stands for 4-fluoro-L-phenylalanine
  MUTAGEN (11)..(11): Xaa stands for beta-cyclohexyl-L-alanine
  MUTAGEN (13)..(13): Xaa stands for D-glutamic acid
XXSXXEYYARXCX

SEQ ID NO: 56 - protein, 13 aa, Artificial Sequence
  artificial peptide
  MUTAGEN (1)..(1): Xaa stands for N-methyl-glutamic acid
  MUTAGEN (2)..(2): Xaa stands for N-methyl-phenylalanine
  MUTAGEN (4)..(4): Xaa stands for beta-cyclohexyl-L-alanine
  MUTAGEN (5)..(5): Xaa stands for 4-fluoro-L-phenylalanine
  MUTAGEN (9)..(9): Xaa stands for 4-carboxy-L-phenylalanine
  MUTAGEN (11)..(11): Xaa stands for beta-cyclohexyl-L-alanine
  MUTAGEN (13)..(13): Xaa stands for D-glutamic acid
XXSXXEYYXRXCX

SEQ ID NO: 57 - protein, 13 aa, Artificial Sequence
  artificial peptide
  MUTAGEN (1)..(1): Xaa stands for N-methyl-glutamic acid
  MUTAGEN (2)..(2): Xaa stands for N-methyl-phenylalanine
  MUTAGEN (4)..(4): Xaa stands for beta-cyclohexyl-L-alanine
  MUTAGEN (5)..(5): Xaa stands for 4-fluoro-L-phenylalanine
  MUTAGEN (9)..(9): Xaa stands for (S)-2-amino-5-ureidopentanoic acid
  MUTAGEN (11)..(11): Xaa stands for beta-cyclohexyl-L-alanine
  MUTAGEN (13)..(13): Xaa stands for D-glutamic acid
XXSXXEYYXRXCX

SEQ ID NO: 58 - protein, 13 aa, Artificial Sequence
  artificial peptide
  MUTAGEN (1)..(1): Xaa stands for N-methyl-glutamic acid
  MUTAGEN (2)..(2): Xaa stands for N-methyl-phenylalanine
  MUTAGEN (4)..(4): Xaa stands for beta-cyclohexyl-L-alanine
  MUTAGEN (5)..(5): Xaa stands for 4-fluoro-L-phenylalanine
  MUTAGEN (8)..(8): Xaa stands for 3-pyridyl-L-alanine
  MUTAGEN (9)..(9): Xaa stands for (S)-2-amino-5-ureidopentanoic acid
  MUTAGEN (11)..(11): Xaa stands for beta-cyclohexyl-L-alanine
  MUTAGEN (13)..(13): Xaa stands for D-glutamic acid
XXSXXSYXXRXCX

SEQ ID NO: 59 - protein, 13 aa, Artificial Sequence
  artificial peptide
  MUTAGEN (1)..(1): Xaa stands for N-methyl-glutamic acid
  MUTAGEN (2)..(2): Xaa stands for N-methyl-phenylalanine
  MUTAGEN (4)..(4): Xaa stands for beta-cyclohexyl-L-alanine
  MUTAGEN (5)..(5): Xaa stands for 4-fluoro-L-phenylalanine
  MUTAGEN (8)..(8): Xaa stands for 3-pyridyl-L-alanine
  MUTAGEN (11)..(11): Xaa stands for beta-cyclohexyl-L-alanine
  MUTAGEN (13)..(13): Xaa stands for D-glutamic acid
XXSXXSYXARXCX

SEQ ID NO: 60 - protein, 13 aa, Artificial Sequence
  artificial peptide
  MUTAGEN (1)..(1): Xaa stands for N-methyl-glutamic acid
  MUTAGEN (2)..(2): Xaa stands for N-methyl-phenylalanine
  MUTAGEN (4)..(4): Xaa stands for beta-cyclohexyl-L-alanine
  MUTAGEN (5)..(5): Xaa stands for 4-fluoro-L-phenylalanine
  MUTAGEN (8)..(8): Xaa stands for beta-(1-naphthyl)-L-alanine
  MUTAGEN (11)..(11): Xaa stands for beta-cyclohexyl-L-alanine
  MUTAGEN (13)..(13): Xaa stands for D-glutamic acid
XXSXXSYXARXCX

SEQ ID NO: 61 - protein, 13 aa, Artificial Sequence
  artificial peptide
  MUTAGEN (1)..(1): Xaa stands for N-methyl-glutamic acid
  MUTAGEN (2)..(2): Xaa stands for N-methyl-phenylalanine
  MUTAGEN (4)..(4): Xaa stands for beta-cyclohexyl-L-alanine
  MUTAGEN (5)..(5): Xaa stands for 4-fluoro-L-phenylalanine
  MUTAGEN (8)..(8): Xaa stands for beta-(1-naphthyl)-L-alanine
  MUTAGEN (9)..(9): Xaa stands for (S)-2-amino-5-ureidopentanoic acid
  MUTAGEN (11)..(11): Xaa stands for beta-cyclohexyl-L-alanine
  MUTAGEN (13)..(13): Xaa stands for D-glutamic acid
XXSXXSYXXRXCX

SEQ ID NO: 62 - protein, 13 aa, Artificial Sequence
  artificial peptide
  MUTAGEN (1)..(1): Xaa stands for N-methyl-glutamic acid
  MUTAGEN (2)..(2): Xaa stands for N-methyl-phenylalanine
  MUTAGEN (4)..(4): Xaa stands for beta-cyclohexyl-L-alanine
  MUTAGEN (5)..(5): Xaa stands for 4-fluoro-L-phenylalanine
  MUTAGEN (11)..(11): Xaa stands for beta-cyclohexyl-L-alanine
  MUTAGEN (13)..(13): Xaa stands for D-glutamic acid
XXSXXSYYARXCX

SEQ ID NO: 63 - protein, 13 aa, Artificial Sequence
  artificial peptide
  MUTAGEN (1)..(1): Xaa stands for N-methyl-glutamic acid
  MUTAGEN (2)..(2): Xaa stands for N-methyl-phenylalanine
  MUTAGEN (4)..(4): Xaa stands for beta-cyclohexyl-L-alanine
  MUTAGEN (5)..(5): Xaa stands for 4-fluoro-L-phenylalanine
  MUTAGEN (11)..(11): Xaa stands for beta-cyclohexyl-L-alanine
  MUTAGEN (13)..(13): Xaa stands for D-glutamic acid
  MOD_RES (13)..(13): AMIDATION
XXSXXSYYARXCX

SEQ ID NO: 64 - protein, 13 aa, Artificial Sequence
  artificial peptide
  MUTAGEN (1)..(1): Xaa stands for N-methyl-glutamic acid
  MUTAGEN (2)..(2): Xaa stands for N-methyl-phenylalanine
  MUTAGEN (4)..(4): Xaa stands for beta-cyclohexyl-L-alanine
  MUTAGEN (5)..(5): Xaa stands for 4-fluoro-L-phenylalanine
  MUTAGEN (11)..(11): Xaa stands for beta-cyclohexyl-L-alanine
  MUTAGEN (13)..(13): Xaa stands for D-glutamic acid
XXSXXSYYAKXCX

SEQ ID NO: 65 - protein, 13 aa, Artificial Sequence
  artificial peptide
  MUTAGEN (1)..(1): Xaa stands for N-methyl-glutamic acid
  MUTAGEN (2)..(2): Xaa stands for N-methyl-phenylalanine
  MUTAGEN (4)..(4): Xaa stands for beta-cyclohexyl-L-alanine
  MUTAGEN (5)..(5): Xaa stands for 4-fluoro-L-phenylalanine
  MUTAGEN (11)..(11): Xaa stands for beta-cyclohexyl-L-alanine
  MUTAGEN (13)..(13): Xaa stands for D-glutamic acid
  MOD_RES (13)..(13): AMIDATION
XXSXXSYYAKXCX

SEQ ID NO: 66 - protein, 13 aa, Artificial Sequence
  artificial peptide
  MUTAGEN (1)..(1): Xaa stands for N-methyl-glutamic acid
  MUTAGEN (2)..(2): Xaa stands for N-methyl-phenylalanine
  MUTAGEN (4)..(4): Xaa stands for beta-cyclohexyl-L-alanine
  MUTAGEN (5)..(5): Xaa stands for 4-fluoro-L-phenylalanine
  MUTAGEN (10)..(10): Xaa stands for (S)-2-amino-3-(piperidin-4-yl)propanoic acid
  MUTAGEN (11)..(11): Xaa stands for beta-cyclohexyl-L-alanine
  MUTAGEN (13)..(13): Xaa stands for D-glutamic acid
XXSXXSYYAXXCX

SEQ ID NO: 67 - protein, 13 aa, Artificial Sequence
  artificial peptide
  MUTAGEN (1)..(1): Xaa stands for N-methyl-glutamic acid
  MUTAGEN (2)..(2): Xaa stands for N-methyl-phenylalanine
  MUTAGEN (4)..(4): Xaa stands for beta-cyclohexyl-L-alanine
  MUTAGEN (5)..(5): Xaa stands for 4-fluoro-L-phenylalanine
  MUTAGEN (9)..(9): Xaa stands for 4-carboxy-L-phenylalanine
  MUTAGEN (11)..(11): Xaa stands for beta-cyclohexyl-L-alanine
  MUTAGEN (13)..(13): Xaa stands for D-glutamic acid
XXSXXSYYXRXCX

SEQ ID NO: 68 - protein, 13 aa, Artificial Sequence
  artificial peptide
  MUTAGEN (1)..(1): Xaa stands for N-methyl-glutamic acid
  MUTAGEN (2)..(2): Xaa stands for N-methyl-phenylalanine
  MUTAGEN (4)..(4): Xaa stands for beta-cyclohexyl-L-alanine
  MUTAGEN (5)..(5): Xaa stands for 4-fluoro-L-phenylalanine
  MUTAGEN (9)..(9): Xaa stands for 4-carboxy-L-phenylalanine
  MUTAGEN (11)..(11): Xaa stands for beta-cyclohexyl-L-alanine
  MUTAGEN (13)..(13): Xaa stands for D-glutamic acid
  MOD_RES (13)..(13): AMIDATION
XXSXXSYYXRXCX

SEQ ID NO: 69 - protein, 13 aa, Artificial Sequence
  artificial peptide
  MUTAGEN (1)..(1): Xaa stands for N-methyl-glutamic acid
  MUTAGEN (2)..(2): Xaa stands for N-methyl-phenylalanine
  MUTAGEN (4)..(4): Xaa stands for beta-cyclohexyl-L-alanine
  MUTAGEN (5)..(5): Xaa stands for 4-fluoro-L-phenylalanine
  MUTAGEN (9)..(9): Xaa stands for 4-carboxy-L-phenylalanine
  MUTAGEN (11)..(11): Xaa stands for beta-cyclohexyl-L-alanine
  MUTAGEN (13)..(13): Xaa stands for D-glutamic acid
XXSXXSYYXKXCX

SEQ ID NO: 70 - protein, 13 aa, Artificial Sequence
  artificial peptide
  MUTAGEN (1)..(1): Xaa stands for N-methyl-glutamic acid
  MUTAGEN (2)..(2): Xaa stands for N-methyl-phenylalanine
  MUTAGEN (4)..(4): Xaa stands for beta-cyclohexyl-L-alanine
  MUTAGEN (5)..(5): Xaa stands for 4-fluoro-L-phenylalanine
  MUTAGEN (9)..(9): Xaa stands for 4-carboxy-L-phenylalanine
  MUTAGEN (11)..(11): Xaa stands for beta-cyclohexyl-L-alanine
  MUTAGEN (13)..(13): Xaa stands for D-glutamic acid
  MOD_RES (13)..(13): AMIDATION
XXSXXSYYXKXCX

SEQ ID NO: 71 - protein, 13 aa, Artificial Sequence
  artificial peptide
  MUTAGEN (1)..(1): Xaa stands for N-methyl-glutamic acid
  MUTAGEN (2)..(2): Xaa stands for N-methyl-phenylalanine
  MUTAGEN (4)..(4): Xaa stands for beta-cyclohexyl-L-alanine
  MUTAGEN (5)..(5): Xaa stands for 4-fluoro-L-phenylalanine
  MUTAGEN (9)..(9): Xaa stands for (S)-2-amino-5-ureidopentanoic acid
  MUTAGEN (11)..(11): Xaa stands for beta-cyclohexyl-L-alanine
  MUTAGEN (13)..(13): Xaa stands for D-glutamic acid
XXSXXSYYXRXCX

SEQ ID NO: 72 - protein, 13 aa, Artificial Sequence
  artificial peptide
  MUTAGEN (1)..(1): Xaa stands for N-methyl-glutamic acid
  MUTAGEN (2)..(2): Xaa stands for N-methyl-phenylalanine
  MUTAGEN (4)..(4): Xaa stands for beta-cyclohexyl-L-alanine
  MUTAGEN (5)..(5): Xaa stands for 4-fluoro-L-phenylalanine
  MUTAGEN (9)..(9): Xaa stands for (S)-2-amino-5-ureidopentanoic acid
  MUTAGEN (11)..(11): Xaa stands for beta-cyclohexyl-L-alanine
  MUTAGEN (13)..(13): Xaa stands for D-glutamic acid
  MOD_RES (13)..(13): AMIDATION
XXSXXSYYXRXCX

SEQ ID NO: 73 - protein, 13 aa, Artificial Sequence
  artificial peptide
  MUTAGEN (1)..(1): Xaa stands for N-methyl-glutamic acid
  MUTAGEN (2)..(2): Xaa stands for N-methyl-phenylalanine
  MUTAGEN (4)..(4): Xaa stands for beta-cyclohexyl-L-alanine
  MUTAGEN (5)..(5): Xaa stands for 4-fluoro-L-phenylalanine
  MUTAGEN (9)..(9): Xaa stands for (S)-2-amino-5-ureidopentanoic acid
  MUTAGEN (11)..(11): Xaa stands for beta-cyclohexyl-L-alanine
  MUTAGEN (13)..(13): Xaa stands for D-glutamic acid
XXSXXSYYXKXCX

SEQ ID NO: 74 - protein, 13 aa, Artificial Sequence
  artificial peptide
  MUTAGEN (1)..(1): Xaa stands for N-methyl-glutamic acid
  MUTAGEN (2)..(2): Xaa stands for N-methyl-phenylalanine
  MUTAGEN (4)..(4): Xaa stands for beta-cyclohexyl-L-alanine
  MUTAGEN (5)..(5): Xaa stands for 4-fluoro-L-phenylalanine
  MUTAGEN (9)..(9): Xaa stands for (S)-2-amino-5-ureidopentanoic acid
  MUTAGEN (11)..(11): Xaa stands for beta-cyclohexyl-L-alanine
  MUTAGEN (13)..(13): Xaa stands for D-glutamic acid
  MOD_RES (13)..(13): AMIDATION
XXSXXSYYXKXCX

SEQ ID NO: 75 - protein, 13 aa, Artificial Sequence
  artificial peptide
  MUTAGEN (1)..(1): Xaa stands for N-methyl-glutamic acid
  MUTAGEN (2)..(2): Xaa stands for N-methyl-phenylalanine
  MUTAGEN (4)..(4): Xaa stands for beta-cyclohexyl-L-alanine
  MUTAGEN (5)..(5): Xaa stands for 4-fluoro-L-phenylalanine
  MUTAGEN (9)..(9): Xaa stands for (S)-2-amino-5-ureidopentanoic acid
  MUTAGEN (10)..(10): Xaa stands for (S)-2-amino-3-(piperidin-4-yl)propanoic acid
  MUTAGEN (11)..(11): Xaa stands for beta-cyclohexyl-L-alanine
  MUTAGEN (13)..(13): Xaa stands for D-glutamic acid
XXSXXSYYXXXCX

SEQ ID NO: 76 - protein, 13 aa, Artificial Sequence
  artificial peptide
  MUTAGEN (1)..(1): Xaa stands for N-methyl-glutamic acid
  MUTAGEN (2)..(2): Xaa stands for N-methyl-phenylalanine
  MUTAGEN (4)..(4): Xaa stands for beta-cyclohexyl-L-alanine
  MUTAGEN (5)..(5): Xaa stands for 4-fluoro-L-phenylalanine
  MUTAGEN (6)..(6): Xaa stands for D-serine
  MUTAGEN (8)..(8): Xaa stands for beta-(1-naphthyl)-L-alanine
  MUTAGEN (11)..(11): Xaa stands for beta-cyclohexyl-L-alanine
  MUTAGEN (13)..(13): Xaa stands for D-glutamic acid
XXSXXXYXARXCX

SEQ ID NO: 77 - protein, 13 aa, Artificial Sequence
  artificial peptide
  MUTAGEN (1)..(1): Xaa stands for N-methyl-glutamic acid
  MUTAGEN (2)..(2): Xaa stands for N-methyl-phenylalanine
  MUTAGEN (4)..(4): Xaa stands for beta-cyclohexyl-L-alanine
  MUTAGEN (5)..(5): Xaa stands for 4-fluoro-L-phenylalanine
  MUTAGEN (6)..(6): Xaa stands for D-serine
  MUTAGEN (8)..(8): Xaa stands for beta-(1-naphthyl)-L-alanine
  MUTAGEN (9)..(9): Xaa stands for (S)-2-amino-5-ureidopentanoic acid
  MUTAGEN (11)..(11): Xaa stands for beta-cyclohexyl-L-alanine
  MUTAGEN (13)..(13): Xaa stands for D-glutamic acid
XXSXXXYXXRXCX

SEQ ID NO: 78 - protein, 13 aa, Artificial Sequence
  artificial peptide
  MUTAGEN (1)..(1): Xaa stands for N-methyl-glutamic acid
  MUTAGEN (2)..(2): Xaa stands for N-methyl-phenylalanine
  MUTAGEN (4)..(4): Xaa stands for beta-cyclohexyl-L-alanine
  MUTAGEN (5)..(5): Xaa stands for 4-fluoro-L-phenylalanine
  MUTAGEN (6)..(6): Xaa stands for D-serine
  MUTAGEN (11)..(11): Xaa stands for beta-cyclohexyl-L-alanine
  MUTAGEN (13)..(13): Xaa stands for D-glutamic acid
XXSXXXYYARXCX

SEQ ID NO: 79 - protein, 13 aa, Artificial Sequence
  artificial peptide
  MUTAGEN (1)..(1): Xaa stands for N-methyl-glutamic acid
  MUTAGEN (2)..(2): Xaa stands for N-methyl-phenylalanine
  MUTAGEN (4)..(4): Xaa stands for beta-cyclohexyl-L-alanine
  MUTAGEN (5)..(5): Xaa stands for 4-fluoro-L-phenylalanine
  MUTAGEN (6)..(6): Xaa stands for D-serine
  MUTAGEN (9)..(9): Xaa stands for 4-carboxy-L-phenylalanine
  MUTAGEN (11)..(11): Xaa stands for beta-cyclohexyl-L-alanine
  MUTAGEN (13)..(13): Xaa stands for D-glutamic acid
XXSXXXYYXRXCX

SEQ ID NO: 80 - protein, 13 aa, Artificial Sequence
  artificial peptide
  MUTAGEN (1)..(1): Xaa stands for N-methyl-glutamic acid
  MUTAGEN (2)..(2): Xaa stands for N-methyl-phenylalanine
  MUTAGEN (4)..(4): Xaa stands for beta-cyclohexyl-L-alanine
  MUTAGEN (5)..(5): Xaa stands for 4-fluoro-L-phenylalanine
  MUTAGEN (6)..(6): Xaa stands for D-serine
  MUTAGEN (9)..(9): Xaa stands for (S)-2-amino-5-ureidopentanoic acid
  MUTAGEN (11)..(11): Xaa stands for beta-cyclohexyl-L-alanine
  MUTAGEN (13)..(13): Xaa stands for D-glutamic acid
XXSXXXYYXRXCX

SEQ ID NO: 81 - protein, 13 aa, Artificial Sequence
  artificial peptide
  MUTAGEN (1)..(1): Xaa stands for N-methyl-glutamic acid
  MUTAGEN (2)..(2): Xaa stands for N-methyl-phenylalanine
  MUTAGEN (4)..(4): Xaa stands for beta-cyclohexyl-L-alanine
  MUTAGEN (5)..(5): Xaa stands for 4-fluoro-L-phenylalanine
  MUTAGEN (6)..(6): Xaa stands for N-methyl-glutamic acid
  MUTAGEN (8)..(8): Xaa stands for beta-(1-naphthyl)-L-alanine
  MUTAGEN (11)..(11): Xaa stands for beta-cyclohexyl-L-alanine
  MUTAGEN (13)..(13): Xaa stands for D-glutamic acid
XXSXXXYXARXCX

SEQ ID NO: 82 - protein, 13 aa, Artificial Sequence
  artificial peptide
  MUTAGEN (1)..(1): Xaa stands for N-methyl-glutamic acid
  MUTAGEN (2)..(2): Xaa stands for N-methyl-phenylalanine
  MUTAGEN (4)..(4): Xaa stands for beta-cyclohexyl-L-alanine
  MUTAGEN (5)..(5): Xaa stands for 4-fluoro-L-phenylalanine
  MUTAGEN (6)..(6): Xaa stands for N-methyl-glutamic acid
  MUTAGEN (8)..(8): Xaa stands for beta-(1-naphthyl)-L-alanine
  MUTAGEN (9)..(9): Xaa stands for (S)-2-amino-5-ureidopentanoic acid
  MUTAGEN (11)..(11): Xaa stands for beta-cyclohexyl-L-alanine
  MUTAGEN (13)..(13): Xaa stands for D-glutamic acid
XXSXXXYXXRXCX

SEQ ID NO: 83 - protein, 13 aa, Artificial Sequence
  artificial peptide
  MUTAGEN (1)..(1): Xaa stands for N-methyl-glutamic acid
  MUTAGEN (2)..(2): Xaa stands for N-methyl-phenylalanine
  MUTAGEN (4)..(4): Xaa stands for beta-cyclohexyl-L-alanine
  MUTAGEN (5)..(5): Xaa stands for 4-fluoro-L-phenylalanine
  MUTAGEN (6)..(6): Xaa stands for N-methyl-glutamic acid
  MUTAGEN (11)..(11): Xaa stands for beta-cyclohexyl-L-alanine
  MUTAGEN (13)..(13): Xaa stands for D-glutamic acid
XXSXXXYYARXCX

SEQ ID NO: 84 - protein, 13 aa, Artificial Sequence
  artificial peptide
  MUTAGEN (1)..(1): Xaa stands for N-methyl-glutamic acid
  MUTAGEN (2)..(2): Xaa stands for N-methyl-phenylalanine
  MUTAGEN (4)..(4): Xaa stands for beta-cyclohexyl-L-alanine
  MUTAGEN (5)..(5): Xaa stands for 4-fluoro-L-phenylalanine
  MUTAGEN (6)..(6): Xaa stands for N-methyl-glutamic acid
  MUTAGEN (11)..(11): Xaa stands for beta-cyclohexyl-L-alanine
  MUTAGEN (13)..(13): Xaa stands for D-glutamic acid
  MOD_RES (13)..(13): AMIDATION
XXSXXXYYARXCX

SEQ ID NO: 85 - protein, 13 aa, Artificial Sequence
  artificial peptide
  MUTAGEN (1)..(1): Xaa stands for N-methyl-glutamic acid
  MUTAGEN (2)..(2): Xaa stands for N-methyl-phenylalanine
  MUTAGEN (4)..(4): Xaa stands for beta-cyclohexyl-L-alanine
  MUTAGEN (5)..(5): Xaa stands for 4-fluoro-L-phenylalanine
  MUTAGEN (6)..(6): Xaa stands for N-methyl-glutamic acid
  MUTAGEN (11)..(11): Xaa stands for beta-cyclohexyl-L-alanine
  MUTAGEN (13)..(13): Xaa stands for D-glutamic acid
XXSXXXYYAKXCX

SEQ ID NO: 86 - protein, 13 aa, Artificial Sequence
  artificial peptide
  MUTAGEN (1)..(1): Xaa stands for N-methyl-glutamic acid
  MUTAGEN (2)..(2): Xaa stands for N-methyl-phenylalanine
  MUTAGEN (4)..(4): Xaa stands for beta-cyclohexyl-L-alanine
  MUTAGEN (5)..(5): Xaa stands for 4-fluoro-L-phenylalanine
  MUTAGEN (6)..(6): Xaa stands for N-methyl-glutamic acid
  MUTAGEN (11)..(11): Xaa stands for beta-cyclohexyl-L-alanine
  MUTAGEN (13)..(13): Xaa stands for D-glutamic acid
  MOD_RES (13)..(13): AMIDATION
XXSXXXYYAKXCX

SEQ ID NO: 87 - protein, 13 aa, Artificial Sequence
  artificial peptide
  MUTAGEN (1)..(1): Xaa stands for N-methyl-glutamic acid
  MUTAGEN (2)..(2): Xaa stands for N-methyl-phenylalanine
  MUTAGEN (4)..(4): Xaa stands for beta-cyclohexyl-L-alanine
  MUTAGEN (5)..(5): Xaa stands for 4-fluoro-L-phenylalanine
  MUTAGEN (6)..(6): Xaa stands for N-methyl-glutamic acid
  MUTAGEN (9)..(9): Xaa stands for 4-carboxy-L-phenylalanine
  MUTAGEN (11)..(11): Xaa stands for beta-cyclohexyl-L-alanine
  MUTAGEN (13)..(13): Xaa stands for D-glutamic acid
XXSXXXYYXRXCX

SEQ ID NO: 88 - protein, 13 aa, Artificial Sequence
  artificial peptide
  MUTAGEN (1)..(1): Xaa stands for N-methyl-glutamic acid
  MUTAGEN (2)..(2): Xaa stands for N-methyl-phenylalanine
  MUTAGEN (4)..(4): Xaa stands for beta-cyclohexyl-L-alanine
  MUTAGEN (5)..(5): Xaa stands for 4-fluoro-L-phenylalanine
  MUTAGEN (6)..(6): Xaa stands for N-methyl-glutamic acid
  MUTAGEN (9)..(9): Xaa stands for 4-carboxy-L-phenylalanine
  MUTAGEN (11)..(11): Xaa stands for beta-cyclohexyl-L-alanine
  MUTAGEN (13)..(13): Xaa stands for D-glutamic acid
  MOD_RES (13)..(13): AMIDATION
XXSXXXYYXRXCX

SEQ ID NO: 89 - protein, 13 aa, Artificial Sequence
  artificial peptide
  MUTAGEN (1)..(1): Xaa stands for N-methyl-glutamic acid
  MUTAGEN (2)..(2): Xaa stands for N-methyl-phenylalanine
  MUTAGEN (4)..(4): Xaa stands for beta-cyclohexyl-L-alanine
  MUTAGEN (5)..(5): Xaa stands for 4-fluoro-L-phenylalanine
  MUTAGEN (6)..(6): Xaa stands for N-methyl-glutamic acid
  MUTAGEN (9)..(9): Xaa stands for 4-carboxy-L-phenylalanine
  MUTAGEN (11)..(11): Xaa stands for beta-cyclohexyl-L-alanine
  MUTAGEN (13)..(13): Xaa stands for D-glutamic acid
XXSXXXYYXKXCX

SEQ ID NO: 90 - protein, 13 aa, Artificial Sequence
  artificial peptide
  MUTAGEN (1)..(1): Xaa stands for N-methyl-glutamic acid
  MUTAGEN (2)..(2): Xaa stands for N-methyl-phenylalanine
  MUTAGEN (4)..(4): Xaa stands for beta-cyclohexyl-L-alanine
  MUTAGEN (5)..(5): Xaa stands for 4-fluoro-L-phenylalanine
  MUTAGEN (6)..(6): Xaa stands for N-methyl-glutamic acid
  MUTAGEN (9)..(9): Xaa stands for 4-carboxy-L-phenylalanine
  MUTAGEN (11)..(11): Xaa stands for beta-cyclohexyl-L-alanine
  MUTAGEN (13)..(13): Xaa stands for D-glutamic acid
  MOD_RES (13)..(13): AMIDATION
XXSXXXYYXKXCX

SEQ ID NO: 91 - protein, 13 aa, Artificial Sequence
  artificial peptide
  MUTAGEN (1)..(1): Xaa stands for N-methyl-glutamic acid
  MUTAGEN (2)..(2): Xaa stands for N-methyl-phenylalanine
  MUTAGEN (4)..(4): Xaa stands for beta-cyclohexyl-L-alanine
  MUTAGEN (5)..(5): Xaa stands for 4-fluoro-L-phenylalanine
  MUTAGEN (6)..(6): Xaa stands for N-methyl-glutamic acid
  MUTAGEN (9)..(9): Xaa stands for (S)-2-amino-5-ureidopentanoic acid
  MUTAGEN (11)..(11): Xaa stands for beta-cyclohexyl-L-alanine
  MUTAGEN (13)..(13): Xaa stands for D-glutamic acid
XXSXXXYYXRXCX

SEQ ID NO: 92 - protein, 13 aa, Artificial Sequence
  artificial peptide
  MUTAGEN (1)..(1): Xaa stands for N-methyl-glutamic acid
  MUTAGEN (2)..(2): Xaa stands for N-methyl-phenylalanine
  MUTAGEN (4)..(4): Xaa stands for beta-cyclohexyl-L-alanine
  MUTAGEN (5)..(5): Xaa stands for 4-fluoro-L-phenylalanine
  MUTAGEN (6)..(6): Xaa stands for N-methyl-glutamic acid
  MUTAGEN (9)..(9): Xaa stands for (S)-2-amino-5-ureidopentanoic acid
  MUTAGEN (11)..(11): Xaa stands for beta-cyclohexyl-L-alanine
  MUTAGEN (13)..(13): Xaa stands for D-glutamic acid
  MOD_RES (13)..(13): AMIDATION
XXSXXXYYXRXCX

SEQ ID NO: 93 - protein, 13 aa, Artificial Sequence
  artificial peptide
  MUTAGEN (1)..(1): Xaa stands for N-methyl-glutamic acid
  MUTAGEN (2)..(2): Xaa stands for N-methyl-phenylalanine
  MUTAGEN (4)..(4): Xaa stands for beta-cyclohexyl-L-alanine
  MUTAGEN (5)..(5): Xaa stands for 4-fluoro-L-phenylalanine
  MUTAGEN (6)..(6): Xaa stands for N-methyl-glutamic acid
  MUTAGEN (9)..(9): Xaa stands for (S)-2-amino-5-ureidopentanoic acid
  MUTAGEN (11)..(11): Xaa stands for beta-cyclohexyl-L-alanine
  MUTAGEN (13)..(13): Xaa stands for D-glutamic acid
XXSXXXYYXKXCX

SEQ ID NO: 94 - protein, 13 aa, Artificial Sequence
  artificial peptide
  MUTAGEN (1)..(1): Xaa stands for N-methyl-glutamic acid
  MUTAGEN (2)..(2): Xaa stands for N-methyl-phenylalanine
  MUTAGEN (4)..(4): Xaa stands for beta-cyclohexyl-L-alanine
  MUTAGEN (5)..(5): Xaa stands for 4-fluoro-L-phenylalanine
  MUTAGEN (6)..(6): Xaa stands for N-methyl-glutamic acid
  MUTAGEN (9)..(9): Xaa stands for (S)-2-amino-5-ureidopentanoic acid
  MUTAGEN (11)..(11): Xaa stands for beta-cyclohexyl-L-alanine
  MUTAGEN (13)..(13): Xaa stands for D-glutamic acid
  MOD_RES (13)..(13): AMIDATION
XXSXXXYYXKXCX

SEQ ID NO: 95 - protein, 13 aa, Artificial Sequence
  artificial peptide
  MUTAGEN (1)..(1): Xaa stands for N-methyl-glutamic acid
  MUTAGEN (2)..(2): Xaa stands for N-methyl-phenylalanine
  MUTAGEN (3)..(3): Xaa stands for alpha-methyl-alanine
  MUTAGEN (4)..(4): Xaa stands for beta-cyclohexyl-L-alanine
  MUTAGEN (5)..(5): Xaa stands for 4-fluoro-L-phenylalanine
  MUTAGEN (6)..(6): Xaa stands for alpha-methyl-alanine
  MUTAGEN (8)..(8): Xaa stands for (S)-2-amino-3-(4-(2-aminoethoxy)-phenyl) propanoic acid
  MUTAGEN (11)..(11): Xaa stands for beta-cyclohexyl-L-alanine
  MUTAGEN (13)..(13): Xaa stands for D-glutamic acid
  MOD_RES (13)..(13): AMIDATION
XXXXXXYXARXCX

SEQ ID NO: 96 - protein, 13 aa, Artificial Sequence
  artificial peptide
  MUTAGEN (1)..(1): Xaa stands for N-methyl-glutamic acid
  MUTAGEN (2)..(2): Xaa stands for N-methyl-phenylalanine
  MUTAGEN (3)..(3): Xaa stands for alpha-methyl-alanine
  MUTAGEN (4)..(4): Xaa stands for beta-cyclohexyl-L-alanine
  MUTAGEN (5)..(5): Xaa stands for 4-fluoro-L-phenylalanine
  MUTAGEN (6)..(6): Xaa stands for alpha-methyl-alanine
  MUTAGEN (8)..(8): Xaa stands for (S)-2-amino-3-(4-(2-aminoethoxy)-phenyl) propanoic acid
  MUTAGEN (9)..(9): Xaa stands for (S)-2-amino-5-ureidopentanoic acid
  MUTAGEN (11)..(11): Xaa stands for beta-cyclohexyl-L-alanine
  MUTAGEN (13)..(13): Xaa stands for D-glutamic acid
  MOD_RES (13)..(13): AMIDATION
XXXXXXYXXRXCX

SEQ ID NO: 97 - protein, 13 aa, Artificial Sequence
  artificial peptide
  MUTAGEN (1)..(1): Xaa stands for N-methyl-glutamic acid
  MUTAGEN (2)..(2): Xaa stands for N-methyl-phenylalanine
  MUTAGEN (3)..(3): Xaa stands for alpha-methyl-alanine
  MUTAGEN (4)..(4): Xaa stands for beta-cyclohexyl-L-alanine
  MUTAGEN (5)..(5): Xaa stands for 4-fluoro-L-phenylalanine
  MUTAGEN (6)..(6): Xaa stands for alpha-methyl-alanine
  MUTAGEN (8)..(8): Xaa stands for 3-pyridyl-L-alanine
  MUTAGEN (11)..(11): Xaa stands for beta-cyclohexyl-L-alanine
  MUTAGEN (13)..(13): Xaa stands for D-glutamic acid
  MOD_RES (13)..(13): AMIDATION
XXXXXXYXARXCX

SEQ ID NO: 98 - protein, 13 aa, Artificial Sequence
  artificial peptide
  MUTAGEN (1)..(1): Xaa stands for N-methyl-glutamic acid
  MUTAGEN (2)..(2): Xaa stands for N-methyl-phenylalanine
  MUTAGEN (3)..(3): Xaa stands for alpha-methyl-alanine
  MUTAGEN (4)..(4): Xaa stands for beta-cyclohexyl-L-alanine
  MUTAGEN (5)..(5): Xaa stands for 4-fluoro-L-phenylalanine
  MUTAGEN (6)..(6): Xaa stands for alpha-methyl-alanine
  MUTAGEN (8)..(8): Xaa stands for 3-pyridyl-L-alanine
  MUTAGEN (9)..(9): Xaa stands for (S)-2-amino-5-ureidopentanoic acid
  MUTAGEN (11)..(11): Xaa stands for beta-cyclohexyl-L-alanine
  MUTAGEN (13)..(13): Xaa stands for D-glutamic acid
  MOD_RES (13)..(13): AMIDATION
XXXXXXYXXRXCX

SEQ ID NO: 99 - protein, 13 aa, Artificial Sequence
  artificial peptide
  MUTAGEN (1)..(1): Xaa stands for N-methyl-glutamic acid
  MUTAGEN (2)..(2): Xaa stands for N-methyl-phenylalanine
  MUTAGEN (3)..(3): Xaa stands for alpha-methyl-alanine
  MUTAGEN (4)..(4): Xaa stands for beta-cyclohexyl-L-alanine
  MUTAGEN (5)..(5): Xaa stands for 4-fluoro-L-phenylalanine
  MUTAGEN (6)..(6): Xaa stands for alpha-methyl-alanine
  MUTAGEN (9)..(9): Xaa stands for (S)-2-amino-5-ureidopentanoic acid
  MUTAGEN (11)..(11): Xaa stands for beta-cyclohexyl-L-alanine
  MUTAGEN (13)..(13): Xaa stands for D-glutamic acid
XXXXXXYYXRXCX

SEQ ID NO: 100 - protein, 13 aa, Artificial Sequence
  artificial peptide
  MUTAGEN (1)..(1): Xaa stands for N-methyl-glutamic acid
  MUTAGEN (2)..(2): Xaa stands for N-methyl-phenylalanine
  MUTAGEN (3)..(3): Xaa stands for alpha-methyl-alanine
  MUTAGEN (4)..(4): Xaa stands for beta-cyclohexyl-L-alanine
  MUTAGEN (5)..(5): Xaa stands for 4-fluoro-L-phenylalanine
  MUTAGEN (6)..(6): Xaa stands for alpha-methyl-alanine
  MUTAGEN (9)..(9): Xaa stands for (S)-2-amino-5-ureidopentanoic acid
  MUTAGEN (11)..(11): Xaa stands for beta-cyclohexyl-L-alanine
  MUTAGEN (13)..(13): Xaa stands for D-glutamic acid
XXXXXXYYXKXCX

SEQ ID NO: 101 - protein, 13 aa, Artificial Sequence
  artificial peptide
  MUTAGEN (1)..(1): Xaa stands for N-methyl-glutamic acid
  MUTAGEN (2)..(2): Xaa stands for N-methyl-phenylalanine
  MUTAGEN (3)..(3): Xaa stands for alpha-methyl-alanine
  MUTAGEN (4)..(4): Xaa stands for beta-cyclohexyl-L-alanine
  MUTAGEN (5)..(5): Xaa stands for 4-fluoro-L-phenylalanine
  MUTAGEN (6)..(6): Xaa stands for alpha-methyl-alanine
  MUTAGEN (9)..(9): Xaa stands for (S)-2-amino-5-ureidopentanoic acid
  MUTAGEN (10)..(10): Xaa stands for D-arginine
  MUTAGEN (11)..(11): Xaa stands for beta-cyclohexyl-L-alanine
  MUTAGEN (13)..(13): Xaa stands for D-glutamic acid
XXXXXXYYXXXCX

SEQ ID NO: 102 - protein, 13 aa, Artificial Sequence
  artificial peptide
  MUTAGEN (1)..(1): Xaa stands for N-methyl-glutamic acid
  MUTAGEN (2)..(2): Xaa stands for N-methyl-phenylalanine
  MUTAGEN (3)..(3): Xaa stands for alpha-methyl-alanine
  MUTAGEN (4)..(4): Xaa stands for beta-cyclohexyl-L-alanine
  MUTAGEN (5)..(5): Xaa stands for 4-fluoro-L-phenylalanine
  MUTAGEN (6)..(6): Xaa stands for alpha-methyl-alanine
  MUTAGEN (9)..(9): Xaa stands for (S)-2-amino-5-ureidopentanoic acid
  MUTAGEN (10)..(10): Xaa stands for D-lysine
  MUTAGEN (11)..(11): Xaa stands for beta-cyclohexyl-L-alanine
  MUTAGEN (13)..(13): Xaa stands for D-glutamic acid
XXXXXXYYXXXCX

SEQ ID NO: 103 - protein, 13 aa, Artificial Sequence
  artificial peptide
  MUTAGEN (1)..(1): Xaa stands for N-methyl-glutamic acid
  MUTAGEN (2)..(2): Xaa stands for N-methyl-phenylalanine
  MUTAGEN (3)..(3): Xaa stands for alpha-methyl-alanine
  MUTAGEN (4)..(4): Xaa stands for beta-cyclohexyl-L-alanine
  MUTAGEN (5)..(5): Xaa stands for 4-fluoro-L-phenylalanine
  MUTAGEN (6)..(6): Xaa stands for D-aspartic acid
  MUTAGEN (8)..(8): Xaa stands for beta-(1-naphthyl)-L-alanine
  MUTAGEN (9)..(9): Xaa stands for (S)-2-amino-5-ureidopentanoic acid
  MUTAGEN (11)..(11): Xaa stands for beta-cyclohexyl-L-alanine
  MUTAGEN (13)..(13): Xaa stands for D-glutamic acid
XXXXXXYXXRXCX

SEQ ID NO: 104 - protein, 13 aa, Artificial Sequence
  artificial peptide
  MUTAGEN (1)..(1): Xaa stands for N-methyl-glutamic acid
  MUTAGEN (2)..(2): Xaa stands for N-methyl-phenylalanine
  MUTAGEN (3)..(3): Xaa stands for alpha-methyl-alanine
  MUTAGEN (4)..(4): Xaa stands for beta-cyclohexyl-L-alanine
  MUTAGEN (5)..(5): Xaa stands for 4-fluoro-L-phenylalanine
  MUTAGEN (6)..(6): Xaa stands for D-aspartic acid
  MUTAGEN (8)..(8): Xaa stands for beta-(1-naphthyl)-L-alanine
  MUTAGEN (9)..(9): Xaa stands for (S)-2-amino-5-ureidopentanoic acid
  MUTAGEN (11)..(11): Xaa stands for beta-cyclohexyl-L-alanine
  MUTAGEN (13)..(13): Xaa stands for D-glutamic acid
XXXXXXYXXKXCX

SEQ ID NO: 105 - protein, 13 aa, Artificial Sequence
  artificial peptide
  MUTAGEN (1)..(1): Xaa stands for N-methyl-glutamic acid
  MUTAGEN (2)..(2): Xaa stands for N-methyl-phenylalanine
  MUTAGEN (3)..(3): Xaa stands for alpha-methyl-alanine
  MUTAGEN (4)..(4): Xaa stands for beta-cyclohexyl-L-alanine
  MUTAGEN (5)..(5): Xaa stands for 4-fluoro-L-phenylalanine
  MUTAGEN (6)..(6): Xaa stands for D-aspartic acid
  MUTAGEN (8)..(8): Xaa stands for beta-(1-naphthyl)-L-alanine
  MUTAGEN (9)..(9): Xaa stands for (S)-2-amino-5-ureidopentanoic acid
  MUTAGEN (10)..(10): Xaa stands for D-arginine
  MUTAGEN (11)..(11): Xaa stands for beta-cyclohexyl-L-alanine
  MUTAGEN (13)..(13): Xaa stands for D-glutamic acid
XXXXXXYXXXXCX

SEQ ID NO: 106 - protein, 13 aa, Artificial Sequence
  artificial peptide
  MUTAGEN (1)..(1): Xaa stands for N-methyl-glutamic acid
  MUTAGEN (2)..(2): Xaa stands for N-methyl-phenylalanine
  MUTAGEN (3)..(3): Xaa stands for alpha-methyl-alanine
  MUTAGEN (4)..(4): Xaa stands for beta-cyclohexyl-L-alanine
  MUTAGEN (5)..(5): Xaa stands for 4-fluoro-L-phenylalanine
  MUTAGEN (6)..(6): Xaa stands for D-aspartic acid
  MUTAGEN (8)..(8): Xaa stands for beta-(1-naphthyl)-L-alanine
  MUTAGEN (9)..(9): Xaa stands for (S)-2-amino-5-ureidopentanoic acid
  MUTAGEN (10)..(10): Xaa stands for D-lysine
  MUTAGEN (11)..(11): Xaa stands for beta-cyclohexyl-L-alanine
  MUTAGEN (13)..(13): Xaa stands for D-glutamic acid
XXXXXXYXXXXCX

SEQ ID NO: 107 - protein, 13 aa, Artificial Sequence
  artificial peptide
  MUTAGEN (1)..(1): Xaa stands for N-methyl-glutamic acid
  MUTAGEN (2)..(2): Xaa stands for N-methyl-phenylalanine
  MUTAGEN (3)..(3): Xaa stands for alpha-methyl-alanine
  MUTAGEN (4)..(4): Xaa stands for beta-cyclohexyl-L-alanine
  MUTAGEN (5)..(5): Xaa stands for 4-fluoro-L-phenylalanine
  MUTAGEN (8)..(8): Xaa stands for beta-(1-naphthyl)-L-alanine
  MUTAGEN (11)..(11): Xaa stands for beta-cyclohexyl-L-alaninee
  MUTAGEN (13)..(13): Xaa stands for D-glutamic acid
XXXXXSYXARXCX

SEQ ID NO: 108 - protein, 13 aa, Artificial Sequence
  artificial peptide
  MUTAGEN (1)..(1): Xaa stands for N-methyl-glutamic acid
  MUTAGEN (2)..(2): Xaa stands for N-methyl-phenylalanine
  MUTAGEN (3)..(3): Xaa stands for alpha-methyl-alanine
  MUTAGEN (4)..(4): Xaa stands for beta-cyclohexyl-L-alanine
  MUTAGEN (5)..(5): Xaa stands for 4-fluoro-L-phenylalanine
  MUTAGEN (8)..(8): Xaa stands for beta-(1-naphthyl)-L-alanine
  MUTAGEN (9)..(9): Xaa stands for (S)-2-amino-5-ureidopentanoic acid
  MUTAGEN (11)..(11): Xaa stands for beta-cyclohexyl-L-alanine
  MUTAGEN (13)..(13): Xaa stands for D-glutamic acid
XXXXXSYXXRXCX

SEQ ID NO: 109 - protein, 13 aa, Artificial Sequence
  artificial peptide
  MUTAGEN (1)..(1): Xaa stands for N-methyl-glutamic acid
  MUTAGEN (2)..(2): Xaa stands for N-methyl-phenylalanine
  MUTAGEN (3)..(3): Xaa stands for alpha-methyl-alanine
  MUTAGEN (4)..(4): Xaa stands for beta-cyclohexyl-L-alanine
  MUTAGEN (5)..(5): Xaa stands for 4-fluoro-L-phenylalanine
  MUTAGEN (11)..(11): Xaa stands for beta-cyclohexyl-L-alanine
  MUTAGEN (13)..(13): Xaa stands for D-glutamic acid
XXXXXSYYARXCX

SEQ ID NO: 110 - protein, 13 aa, Artificial Sequence
  artificial peptide
  MUTAGEN (1)..(1): Xaa stands for N-methyl-glutamic acid
  MUTAGEN (2)..(2): Xaa stands for N-methyl-phenylalanine
  MUTAGEN (3)..(3): Xaa stands for alpha-methyl-alanine
  MUTAGEN (4)..(4): Xaa stands for beta-cyclohexyl-L-alanine
  MUTAGEN (5)..(5): Xaa stands for 4-fluoro-L-phenylalanine
  MUTAGEN (9)..(9): Xaa stands for 4-carboxy-L-phenylalanine
  MUTAGEN (11)..(11): Xaa stands for beta-cyclohexyl-L-alanine
  MUTAGEN (13)..(13): Xaa stands for D-glutamic acid
XXXXXSYYXRXCX

SEQ ID NO: 111 - protein, 13 aa, Artificial Sequence
  artificial peptide
  MUTAGEN (1)..(1): Xaa stands for N-methyl-glutamic acid
  MUTAGEN (2)..(2): Xaa stands for N-methyl-phenylalanine
  MUTAGEN (3)..(3): Xaa stands for alpha-methyl-alanine
  MUTAGEN (4)..(4): Xaa stands for beta-cyclohexyl-L-alanine
  MUTAGEN (5)..(5): Xaa stands for 4-fluoro-L-phenylalanine
  MUTAGEN (9)..(9): Xaa stands for (S)-2-amino-5-ureidopentanoic acid
  MUTAGEN (11)..(11): Xaa stands for beta-cyclohexyl-L-alanine
  MUTAGEN (13)..(13): Xaa stands for D-glutamic acid
XXXXXSYYXRXCX

SEQ ID NO: 112 - protein, 13 aa, Artificial Sequence
  artificial peptide
  MUTAGEN (1)..(1): Xaa stands for N-methyl-glutamic acid
  MUTAGEN (2)..(2): Xaa stands for N-methyl-phenylalanine
  MUTAGEN (3)..(3): Xaa stands for alpha-methyl-alanine
  MUTAGEN (4)..(4): Xaa stands for beta-cyclohexyl-L-alanine
  MUTAGEN (5)..(5): Xaa stands for 4-fluoro-L-phenylalanine
  MUTAGEN (6)..(6): Xaa stands for N-methyl-glutamic acid
  MUTAGEN (8)..(8): Xaa stands for beta-(1-naphthyl)-L-alanine
  MUTAGEN (9)..(9): Xaa stands for (S)-2-amino-5-ureidopentanoic acid
  MUTAGEN (11)..(11): Xaa stands for beta-cyclohexyl-L-alanine
  MUTAGEN (13)..(13): Xaa stands for D-glutamic acid
XXXXXXYXXRXCX

SEQ ID NO: 113 - protein, 13 aa, Artificial Sequence
  artificial peptide
  MUTAGEN (1)..(1): Xaa stands for N-methyl-glutamic acid
  MUTAGEN (2)..(2): Xaa stands for N-methyl-phenylalanine
  MUTAGEN (3)..(3): Xaa stands for alpha-methyl-alanine
  MUTAGEN (4)..(4): Xaa stands for beta-cyclohexyl-L-alanine
  MUTAGEN (5)..(5): Xaa stands for 4-fluoro-L-phenylalanine
  MUTAGEN (6)..(6): Xaa stands for N-methyl-glutamic acid
  MUTAGEN (8)..(8): Xaa stands for beta-(1-naphthyl)-L-alanine
  MUTAGEN (9)..(9): Xaa stands for (S)-2-amino-5-ureidopentanoic acid
  MUTAGEN (11)..(11): Xaa stands for beta-cyclohexyl-L-alanine
  MUTAGEN (13)..(13): Xaa stands for D-glutamic acid
XXXXXXYXXKXCX

SEQ ID NO: 114 - protein, 13 aa, Artificial Sequence
  artificial peptide
  MUTAGEN (1)..(1): Xaa stands for N-methyl-glutamic acid
  MUTAGEN (2)..(2): Xaa stands for N-methyl-phenylalanine
  MUTAGEN (3)..(3): Xaa stands for alpha-methyl-alanine
  MUTAGEN (4)..(4): Xaa stands for beta-cyclohexyl-L-alanine
  MUTAGEN (5)..(5): Xaa stands for 4-fluoro-L-phenylalanine
  MUTAGEN (6)..(6): Xaa stands for N-methyl-glutamic acid
  MUTAGEN (8)..(8): Xaa stands for beta-(1-naphthyl)-L-alanine
  MUTAGEN (9)..(9): Xaa stands for (S)-2-amino-5-ureidopentanoic acid
  MUTAGEN (10)..(10): Xaa stands for D-arginine
  MUTAGEN (11)..(11): Xaa stands for beta-cyclohexyl-L-alanine
  MUTAGEN (13)..(13): Xaa stands for D-glutamic acid
XXXXXXYXXXXCX

SEQ ID NO: 115 - protein, 13 aa, Artificial Sequence
  artificial peptide
  MUTAGEN (1)..(1): Xaa stands for N-methyl-glutamic acid
  MUTAGEN (2)..(2): Xaa stands for N-methyl-phenylalanine
  MUTAGEN (3)..(3): Xaa stands for alpha-methyl-alanine
  MUTAGEN (4)..(4): Xaa stands for beta-cyclohexyl-L-alanine
  MUTAGEN (5)..(5): Xaa stands for 4-fluoro-L-phenylalanine
  MUTAGEN (6)..(6): Xaa stands for N-methyl-glutamic acid
  MUTAGEN (8)..(8): Xaa stands for beta-(1-naphthyl)-L-alanine
  MUTAGEN (9)..(9): Xaa stands for (S)-2-amino-5-ureidopentanoic acid
  MUTAGEN (10)..(10): Xaa stands for D-lysine
  MUTAGEN (11)..(11): Xaa stands for beta-cyclohexyl-L-alanine
  MUTAGEN (13)..(13): Xaa stands for D-glutamic acid
XXXXXXYXXXXCX

SEQ ID NO: 116 - protein, 13 aa, Artificial Sequence
  artificial peptide
  MUTAGEN (1)..(1): Xaa stands for N-methyl-glutamic acid
  MUTAGEN (2)..(2): Xaa stands for N-methyl-phenylalanine
  MUTAGEN (3)..(3): Xaa stands for alpha-methyl-alanine
  MUTAGEN (4)..(4): Xaa stands for beta-cyclohexyl-L-alanine
  MUTAGEN (5)..(5): Xaa stands for 4-fluoro-L-phenylalanine
  MUTAGEN (6)..(6): Xaa stands for N-methyl-glutamic acid
  MUTAGEN (11)..(11): Xaa stands for beta-cyclohexyl-L-alanine
  MUTAGEN (13)..(13): Xaa stands for D-glutamic acid
XXXXXXYYARXCX

SEQ ID NO: 117 - protein, 13 aa, Artificial Sequence
  artificial peptide
  MUTAGEN (1)..(1): Xaa stands for N-methyl-glutamic acid
  MUTAGEN (2)..(2): Xaa stands for N-methyl-phenylalanine
  MUTAGEN (3)..(3): Xaa stands for alpha-methyl-alanine
  MUTAGEN (4)..(4): Xaa stands for beta-cyclohexyl-L-alanine
  MUTAGEN (5)..(5): Xaa stands for 4-fluoro-L-phenylalanine
  MUTAGEN (6)..(6): Xaa stands for N-methyl-glutamic acid
  MUTAGEN (11)..(11): Xaa stands for beta-cyclohexyl-L-alanine
  MUTAGEN (13)..(13): Xaa stands for D-glutamic acid
XXXXXXYYAKXCX

SEQ ID NO: 118 - protein, 13 aa, Artificial Sequence
  artificial peptide
  MUTAGEN (1)..(1): Xaa stands for N-methyl-glutamic acid
  MUTAGEN (2)..(2): Xaa stands for N-methyl-phenylalanine
  MUTAGEN (3)..(3): Xaa stands for alpha-methyl-alanine
  MUTAGEN (4)..(4): Xaa stands for beta-cyclohexyl-L-alanine
  MUTAGEN (5)..(5): Xaa stands for 4-fluoro-L-phenylalanine
  MUTAGEN (6)..(6): Xaa stands for N-methyl-glutamic acid
  MUTAGEN (10)..(10): Xaa stands for (S)-2-amino-3-(piperidin-4-yl)propanoic acid
  MUTAGEN (11)..(11): Xaa stands for beta-cyclohexyl-L-alanine
  MUTAGEN (13)..(13): Xaa stands for D-glutamic acid
XXXXXXYYAXXCX

SEQ ID NO: 119 - protein, 13 aa, Artificial Sequence
  artificial peptide
  MUTAGEN (1)..(1): Xaa stands for N-methyl-glutamic acid
  MUTAGEN (2)..(2): Xaa stands for N-methyl-phenylalanine
  MUTAGEN (3)..(3): Xaa stands for alpha-methyl-alanine
  MUTAGEN (4)..(4): Xaa stands for beta-cyclohexyl-L-alanine
  MUTAGEN (5)..(5): Xaa stands for 4-fluoro-L-phenylalanine
  MUTAGEN (6)..(6): Xaa stands for N-methyl-glutamic acid
  MUTAGEN (9)..(9): Xaa stands for 4-carboxy-L-phenylalanine
  MUTAGEN (11)..(11): Xaa stands for beta-cyclohexyl-L-alanine
  MUTAGEN (13)..(13): Xaa stands for D-glutamic acid
XXXXXXYYXRXCX

SEQ ID NO: 120 - protein, 13 aa, Artificial Sequence
  artificial peptide
  MUTAGEN (1)..(1): Xaa stands for N-methyl-glutamic acid
  MUTAGEN (2)..(2): Xaa stands for N-methyl-phenylalanine
  MUTAGEN (3)..(3): Xaa stands for alpha-methyl-alanine
  MUTAGEN (4)..(4): Xaa stands for beta-cyclohexyl-L-alanine
  MUTAGEN (5)..(5): Xaa stands for 4-fluoro-L-phenylalanine
  MUTAGEN (6)..(6): Xaa stands for N-methyl-glutamic acid
  MUTAGEN (9)..(9): Xaa stands for 4-carboxy-L-phenylalanine
  MUTAGEN (11)..(11): Xaa stands for beta-cyclohexyl-L-alanine
  MUTAGEN (13)..(13): Xaa stands for D-glutamic acid
XXXXXXYYXKXCX

SEQ ID NO: 121 - protein, 13 aa, Artificial Sequence
  artificial peptide
  MUTAGEN (1)..(1): Xaa stands for N-methyl-glutamic acid
  MUTAGEN (2)..(2): Xaa stands for N-methyl-phenylalanine
  MUTAGEN (3)..(3): Xaa stands for alpha-methyl-alanine
  MUTAGEN (4)..(4): Xaa stands for beta-cyclohexyl-L-alanine
  MUTAGEN (5)..(5): Xaa stands for 4-fluoro-L-phenylalanine
  MUTAGEN (6)..(6): Xaa stands for N-methyl-glutamic acid
  MUTAGEN (9)..(9): Xaa stands for 4-carboxy-L-phenylalanine
  MUTAGEN (10)..(10): Xaa stands for (S)-2-amino-3-(piperidin-4-yl)propanoic acid
  MUTAGEN (11)..(11): Xaa stands for beta-cyclohexyl-L-alanine
  MUTAGEN (13)..(13): Xaa stands for D-glutamic acid
XXXXXXYYXXXCX

SEQ ID NO: 122 - protein, 13 aa, Artificial Sequence
  artificial peptide
  MUTAGEN (1)..(1): Xaa stands for N-methyl-glutamic acid
  MUTAGEN (2)..(2): Xaa stands for N-methyl-phenylalanine
  MUTAGEN (3)..(3): Xaa stands for alpha-methyl-alanine
  MUTAGEN (4)..(4): Xaa stands for beta-cyclohexyl-L-alanine
  MUTAGEN (5)..(5): Xaa stands for 4-fluoro-L-phenylalanine
  MUTAGEN (6)..(6): Xaa stands for N-methyl-glutamic acid
  MUTAGEN (9)..(9): Xaa stands for (S)-2-amino-5-ureidopentanoic acid
  MUTAGEN (11)..(11): Xaa stands for beta-cyclohexyl-L-alanine
  MUTAGEN (13)..(13): Xaa stands for D-glutamic acid
XXXXXXYYXRXCX

SEQ ID NO: 123 - protein, 13 aa, Artificial Sequence
  artificial peptide
  MUTAGEN (1)..(1): Xaa stands for N-methyl-glutamic acid
  MUTAGEN (2)..(2): Xaa stands for N-methyl-phenylalanine
  MUTAGEN (3)..(3): Xaa stands for alpha-methyl-alanine
  MUTAGEN (4)..(4): Xaa stands for beta-cyclohexyl-L-alanine
  MUTAGEN (5)..(5): Xaa stands for 4-fluoro-L-phenylalanine
  MUTAGEN (6)..(6): Xaa stands for N-methyl-glutamic acid
  MUTAGEN (9)..(9): Xaa stands for (S)-2-amino-5-ureidopentanoic acid
  MUTAGEN (11)..(11): Xaa stands for beta-cyclohexyl-L-alanine
  MUTAGEN (13)..(13): Xaa stands for D-glutamic acid
XXXXXXYYXKXCX

SEQ ID NO: 124 - protein, 13 aa, Artificial Sequence
  artificial peptide
  MUTAGEN (1)..(1): Xaa stands for N-methyl-glutamic acid
  MUTAGEN (2)..(2): Xaa stands for N-methyl-phenylalanine
  MUTAGEN (3)..(3): Xaa stands for alpha-methyl-alanine
  MUTAGEN (4)..(4): Xaa stands for beta-cyclohexyl-L-alanine
  MUTAGEN (5)..(5): Xaa stands for 4-fluoro-L-phenylalanine
  MUTAGEN (6)..(6): Xaa stands for N-methyl-glutamic acid
  MUTAGEN (9)..(9): Xaa stands for (S)-2-amino-5-ureidopentanoic acid
  MUTAGEN (10)..(10): Xaa stands for D-arginine
  MUTAGEN (11)..(11): Xaa stands for beta-cyclohexyl-L-alanine
  MUTAGEN (13)..(13): Xaa stands for D-glutamic acid
XXXXXXYYXXXCX

SEQ ID NO: 125 - protein, 13 aa, Artificial Sequence
  artificial peptide
  MUTAGEN (1)..(1): Xaa stands for N-methyl-glutamic acid
  MUTAGEN (2)..(2): Xaa stands for N-methyl-phenylalanine
  MUTAGEN (3)..(3): Xaa stands for alpha-methyl-alanine
  MUTAGEN (4)..(4): Xaa stands for beta-cyclohexyl-L-alanine
  MUTAGEN (5)..(5): Xaa stands for 4-fluoro-L-phenylalanine
  MUTAGEN (6)..(6): Xaa stands for N-methyl-glutamic acid
  MUTAGEN (9)..(9): Xaa stands for (S)-2-amino-5-ureidopentanoic acid
  MUTAGEN (10)..(10): Xaa stands for D-lysine
  MUTAGEN (11)..(11): Xaa stands for beta-cyclohexyl-L-alanine
  MUTAGEN (13)..(13): Xaa stands for D-glutamic acid
XXXXXXYYXXXCX

SEQ ID NO: 126 - protein, 13 aa, Artificial Sequence
  artificial peptide
  MUTAGEN (1)..(1): Xaa stands for N-methyl-glutamic acid
  MUTAGEN (2)..(2): Xaa stands for N-methyl-phenylalanine
  MUTAGEN (3)..(3): Xaa stands for alpha-methyl-alanine
  MUTAGEN (4)..(4): Xaa stands for beta-cyclohexyl-L-alanine
  MUTAGEN (5)..(5): Xaa stands for 4-fluoro-L-phenylalanine
  MUTAGEN (6)..(6): Xaa stands for N-methyl-glutamic acid
  MUTAGEN (9)..(9): Xaa stands for (S)-2-amino-5-ureidopentanoic acid
  MUTAGEN (10)..(10): Xaa stands for (S)-2-amino-3-(piperidin-4-yl)propanoic acid
  MUTAGEN (11)..(11): Xaa stands for beta-cyclohexyl-L-alanine
  MUTAGEN (13)..(13): Xaa stands for D-glutamic acid
XXXXXXYYXXXCX

SEQ ID NO: 127 - DNA, 26 bp, Artificial Sequence
  primer for RT-PCR
acaggtacgttaatagttaatagcgt

SEQ ID NO: 128 - DNA, 22 bp, Artificial Sequence
  primer for RT-PCR
atattgcagcagtacgcacaca

SEQ ID NO: 129 - DNA, 26 bp, Artificial Sequence
  probe
acactagccatccttactgcgcttcg

SEQ ID NO: 130 - DNA, 20 bp, Artificial Sequence
  N-2 forward primer for RT-PCR
ttacaaacattggccgcaaa

SEQ ID NO: 131 - DNA, 18 bp, Artificial Sequence
  N-2 reverse primer for RT-PCR
gcgcgacattccgaagaa

SEQ ID NO: 132 - protein, 13 aa, Artificial Sequence
  artificial peptide
  MUTAGEN (1)..(1): Xaa stands for N-methyl-glutamic acid
  MUTAGEN (2)..(2): Xaa stands for N-methyl-L-norleucine
  MUTAGEN (4)..(4): Xaa stands for beta-cyclohexyl-L-alanine
  MUTAGEN (5)..(5): Xaa stands for 4-fluoro-L-phenylalanine
  MUTAGEN (6)..(6): Xaa stands for alpha-methyl-alanine
  MUTAGEN (10)..(10): Xaa stands for D-arginine
  MUTAGEN (11)..(11): Xaa stands for beta-cyclohexyl-L-alanine
  MUTAGEN (13)..(13): Xaa stands for D-glutamic acid
XXSXXXYYAXXCX

SEQ ID NO: 133 - protein, 13 aa, Artificial Sequence
  artificial peptide
  MUTAGEN (1)..(1): Xaa stands for N-methyl-glutamic acid
  MUTAGEN (2)..(2): Xaa stands for N-methyl-L-norleucine
  MUTAGEN (4)..(4): Xaa stands for beta-cyclohexyl-L-alanine
  MUTAGEN (5)..(5): Xaa stands for 4-fluoro-L-phenylalanine
  MUTAGEN (6)..(6): Xaa stands for alpha-methyl-alanine
  MUTAGEN (10)..(10): Xaa stands for D-lysine
  MUTAGEN (11)..(11): Xaa stands for beta-cyclohexyl-L-alanine
  MUTAGEN (13)..(13): Xaa stands for D-glutamic acid
XXSXXXYYAXXCX

SEQ ID NO: 134 - protein, 13 aa, Artificial Sequence
  artificial peptide
  MUTAGEN (1)..(1): Xaa stands for N-methyl-glutamic acid
  MUTAGEN (2)..(2): Xaa stands for N-methyl-L-norleucine
  MUTAGEN (4)..(4): Xaa stands for beta-cyclohexyl-L-alanine
  MUTAGEN (5)..(5): Xaa stands for 4-fluoro-L-phenylalanine
  MUTAGEN (6)..(6): Xaa stands for alpha-methyl-alanine
  MUTAGEN (10)..(10): Xaa stands for D-arginine
  MUTAGEN (11)..(11): Xaa stands for beta-cyclohexyl-L-alanine
  MUTAGEN (13)..(13): Xaa stands for D-glutamic acid
  MOD_RES (13)..(13): AMIDATION
XXSXXXYYAXXCX

SEQ ID NO: 135 - protein, 13 aa, Artificial Sequence
  artificial peptide
  MUTAGEN (1)..(1): Xaa stands for N-methyl-glutamic acid
  MUTAGEN (2)..(2): Xaa stands for N-methyl-L-norleucine
  MUTAGEN (4)..(4): Xaa stands for beta-cyclohexyl-L-alanine
  MUTAGEN (5)..(5): Xaa stands for 4-fluoro-L-phenylalanine
  MUTAGEN (6)..(6): Xaa stands for alpha-methyl-alanine
  MUTAGEN (10)..(10): Xaa stands for D-lysine
  MUTAGEN (11)..(11): Xaa stands for beta-cyclohexyl-L-alanine
  MUTAGEN (13)..(13): Xaa stands for D-glutamic acid
  MOD_RES (13)..(13): AMIDATION
XXSXXXYYAXXCX

SEQ ID NO: 136 - protein, 13 aa, Artificial Sequence
  artificial peptide
  MUTAGEN (1)..(1): Xaa stands for N-methyl-glutamic acid
  MUTAGEN (2)..(2): Xaa stands for N-methyl-phenylalanine
  MUTAGEN (3)..(3): Xaa stands for alpha-methyl-alanine
  MUTAGEN (4)..(4): Xaa stands for beta-cyclohexyl-L-alanine
  MUTAGEN (5)..(5): Xaa stands for 4-fluoro-L-phenylalanine
  MUTAGEN (6)..(6): Xaa stands for N-methyl-glutamic acid
  MUTAGEN (9)..(9): Xaa stands for 4-carboxy-L-phenylalanine
  MUTAGEN (10)..(10): Xaa stands for D-arginine
  MUTAGEN (11)..(11): Xaa stands for beta-cyclohexyl-L-alanine
  MUTAGEN (13)..(13): Xaa stands for D-glutamic acid
XXXXXXYYXXXCX

SEQ ID NO: 137 - protein, 13 aa, Artificial Sequence
  artificial peptide
  MUTAGEN (1)..(1): Xaa stands for N-methyl-glutamic acid
  MUTAGEN (2)..(2): Xaa stands for N-methyl-L-norleucine
  MUTAGEN (3)..(3): Xaa stands for alpha-methyl-alanine
  MUTAGEN (4)..(4): Xaa stands for beta-cyclohexyl-L-alanine
  MUTAGEN (5)..(5): Xaa stands for 4-fluoro-L-phenylalanine
  MUTAGEN (6)..(6): Xaa stands for N-methyl-glutamic acid
  MUTAGEN (9)..(9): Xaa stands for 4-carboxy-L-phenylalanine
  MUTAGEN (10)..(10): Xaa stands for D-arginine
  MUTAGEN (11)..(11): Xaa stands for beta-cyclohexyl-L-alanine
  MUTAGEN (13)..(13): Xaa stands for D-glutamic acid
XXXXXXYYXXXCX

SEQ ID NO: 138 - protein, 13 aa, Artificial Sequence
  artificial peptide
  MUTAGEN (1)..(1): Xaa stands for N-methyl-glutamic acid
  MUTAGEN (2)..(2): Xaa stands for N-methyl-phenylalanine
  MUTAGEN (4)..(4): Xaa stands for beta-cyclohexyl-L-alanine
  MUTAGEN (5)..(5): Xaa stands for 4-fluoro-L-phenylalanine
  MUTAGEN (6)..(6): Xaa stands for N-methyl-glutamic acid
  MUTAGEN (9)..(9): Xaa stands for 4-carboxy-L-phenylalanine
  MUTAGEN (10)..(10): Xaa stands for D-arginine
  MUTAGEN (11)..(11): Xaa stands for beta-cyclohexyl-L-alanine
  MUTAGEN (13)..(13): Xaa stands for D-glutamic acid
  MOD_RES (13)..(13): AMIDATION
XXSXXXYYXXXCX

SEQ ID NO: 139 - protein, 13 aa, Artificial Sequence
  artificial peptide
  MUTAGEN (1)..(1): Xaa stands for N-methyl-glutamic acid
  MUTAGEN (2)..(2): Xaa stands for N-methyl-phenylalanine
  MUTAGEN (3)..(3): Xaa stands for alpha-methyl-alanine
  MUTAGEN (4)..(4): Xaa stands for beta-cyclohexyl-L-alanine
  MUTAGEN (5)..(5): Xaa stands for 4-fluoro-L-phenylalanine
  MUTAGEN (6)..(6): Xaa stands for N-methyl-glutamic acid
  MUTAGEN (9)..(9): Xaa stands for 4-carboxy-L-phenylalanine
  MUTAGEN (10)..(10): Xaa stands for D-arginine
  MUTAGEN (11)..(11): Xaa stands for beta-cyclohexyl-L-alanine
  MUTAGEN (13)..(13): Xaa stands for D-glutamic acid
  MOD_RES (13)..(13): AMIDATION
XXXXXXYYXXXCX

SEQ ID NO: 140 - protein, 13 aa, Artificial Sequence
  artificial peptide
  MUTAGEN (1)..(1): Xaa stands for N-methyl-glutamic acid
  MUTAGEN (2)..(2): Xaa stands for N-methyl-phenylalanine
  MUTAGEN (4)..(4): Xaa stands for beta-cyclohexyl-L-alanine
  MUTAGEN (5)..(5): Xaa stands for 4-fluoro-L-phenylalanine
  MUTAGEN (6)..(6): Xaa stands for N-methyl-glutamic acid
  MUTAGEN (9)..(9): Xaa stands for 4-carboxy-L-phenylalanine
  MUTAGEN (10)..(10): Xaa stands for D-arginine
  MUTAGEN (11)..(11): Xaa stands for beta-cyclohexyl-L-alanine
  MUTAGEN (13)..(13): Xaa stands for D-glutamic acid
XXSXXXYYXXXCX

SEQ ID NO: 141 - protein, 13 aa, Artificial Sequence
  artificial peptide
  MUTAGEN (1)..(1): Xaa stands for N-methyl-glutamic acid
  MUTAGEN (2)..(2): Xaa stands for N-methyl-L-norleucine
  MUTAGEN (3)..(3): Xaa stands for alpha-methyl-alanine
  MUTAGEN (4)..(4): Xaa stands for beta-cyclohexyl-L-alanine
  MUTAGEN (5)..(5): Xaa stands for 4-fluoro-L-phenylalanine
  MUTAGEN (6)..(6): Xaa stands for D-aspartic acid
  MUTAGEN (9)..(9): Xaa stands for 4-carboxy-L-phenylalanine
  MUTAGEN (10)..(10): Xaa stands for D-arginine
  MUTAGEN (11)..(11): Xaa stands for beta-cyclohexyl-L-alanine
  MUTAGEN (13)..(13): Xaa stands for D-glutamic acid
XXXXXXYYXXXCX

SEQ ID NO: 142 - protein, 13 aa, Artificial Sequence
  artificial peptide
  MUTAGEN (1)..(1): Xaa stands for N-methyl-glutamic acid
  MUTAGEN (2)..(2): Xaa stands for N-methyl-L-norleucine
  MUTAGEN (3)..(3): Xaa stands for alpha-methyl-alanine
  MUTAGEN (4)..(4): Xaa stands for beta-cyclohexyl-L-alanine
  MUTAGEN (5)..(5): Xaa stands for 4-fluoro-L-phenylalanine
  MUTAGEN (6)..(6): Xaa stands for D-aspartic acid
  MUTAGEN (9)..(9): Xaa stands for 4-carboxy-L-phenylalanine
  MUTAGEN (10)..(10): Xaa stands for D-lysine
  MUTAGEN (11)..(11): Xaa stands for beta-cyclohexyl-L-alanine
  MUTAGEN (13)..(13): Xaa stands for D-glutamic acid
XXXXXXYYXXXCX

SEQ ID NO: 143 - protein, 13 aa, Artificial Sequence
  artificial peptide
  MUTAGEN (1)..(1): Xaa stands for N-methyl-glutamic acid
  MUTAGEN (2)..(2): Xaa stands for N-methyl-phenylalanine
  MUTAGEN (3)..(3): Xaa stands for alpha-methyl-alanine
  MUTAGEN (4)..(4): Xaa stands for beta-cyclohexyl-L-alanine
  MUTAGEN (5)..(5): Xaa stands for 4-fluoro-L-phenylalanine
  MUTAGEN (6)..(6): Xaa stands for alpha-methyl-alanine
  MUTAGEN (9)..(9): Xaa stands for 4-carboxy-L-phenylalanine
  MUTAGEN (11)..(11): Xaa stands for beta-cyclohexyl-L-alanine
  MUTAGEN (13)..(13): Xaa stands for D-glutamic acid
XXXXXXYYXRXCX

SEQ ID NO: 144 - protein, 13 aa, Artificial Sequence
  artificial peptide
  MUTAGEN (1)..(1): Xaa stands for N-methyl-glutamic acid
  MUTAGEN (2)..(2): Xaa stands for N-methyl-phenylalanine
  MUTAGEN (3)..(3): Xaa stands for alpha-methyl-alanine
  MUTAGEN (4)..(4): Xaa stands for beta-cyclohexyl-L-alanine
  MUTAGEN (5)..(5): Xaa stands for 4-fluoro-L-phenylalanine
  MUTAGEN (6)..(6): Xaa stands for alpha-methyl-alanine
  MUTAGEN (9)..(9): Xaa stands for 4-carboxy-L-phenylalanine
  MUTAGEN (11)..(11): Xaa stands for beta-cyclohexyl-L-alanine
  MUTAGEN (13)..(13): Xaa stands for D-glutamic acid
XXXXXXYYXKXCX

SEQ ID NO: 145 - protein, 13 aa, Artificial Sequence
  artificial peptide
  MUTAGEN (1)..(1): Xaa stands for N-methyl-glutamic acid
  MUTAGEN (2)..(2): Xaa stands for N-methyl-phenylalanine
  MUTAGEN (3)..(3): Xaa stands for alpha-methyl-alanine
  MUTAGEN (4)..(4): Xaa stands for beta-cyclohexyl-L-alanine
  MUTAGEN (5)..(5): Xaa stands for 4-fluoro-L-phenylalanine
  MUTAGEN (6)..(6): Xaa stands for alpha-methyl-alanine
  MUTAGEN (9)..(9): Xaa stands for 4-carboxy-L-phenylalanine
  MUTAGEN (10)..(10): Xaa stands for D-arginine
  MUTAGEN (11)..(11): Xaa stands for beta-cyclohexyl-L-alanine
  MUTAGEN (13)..(13): Xaa stands for D-glutamic acid
XXXXXXYYXXXCX

SEQ ID NO: 146 - protein, 13 aa, Artificial Sequence
  artificial peptide
  MUTAGEN (1)..(1): Xaa stands for N-methyl-glutamic acid
  MUTAGEN (2)..(2): Xaa stands for N-methyl-phenylalanine
  MUTAGEN (3)..(3): Xaa stands for alpha-methyl-alanine
  MUTAGEN (4)..(4): Xaa stands for beta-cyclohexyl-L-alanine
  MUTAGEN (5)..(5): Xaa stands for 4-fluoro-L-phenylalanine
  MUTAGEN (6)..(6): Xaa stands for alpha-methyl-alanine
  MUTAGEN (9)..(9): Xaa stands for 4-carboxy-L-phenylalanine
  MUTAGEN (10)..(10): Xaa stands for D-lysine
  MUTAGEN (11)..(11): Xaa stands for beta-cyclohexyl-L-alanine
  MUTAGEN (13)..(13): Xaa stands for D-glutamic acid
XXXXXXYYXXXCX

SEQ ID NO: 147 - protein, 13 aa, Artificial Sequence
  artificial peptide
  MUTAGEN (1)..(1): Xaa stands for N-methyl-glutamic acid
  MUTAGEN (2)..(2): Xaa stands for N-methyl-phenylalanine
  MUTAGEN (3)..(3): Xaa stands for alpha-methyl-alanine
  MUTAGEN (4)..(4): Xaa stands for beta-cyclohexyl-L-alanine
  MUTAGEN (5)..(5): Xaa stands for 4-fluoro-L-phenylalanine
  MUTAGEN (6)..(6): Xaa stands for N-methyl-glutamic acid
  MUTAGEN (9)..(9): Xaa stands for 4-carboxy-L-phenylalanine
  MUTAGEN (10)..(10): Xaa stands for D-lysine
  MUTAGEN (11)..(11): Xaa stands for beta-cyclohexyl-L-alanine
  MUTAGEN (13)..(13): Xaa stands for D-glutamic acid
XXXXXXYYXXXCX

SEQ ID NO: 148 - protein, 13 aa, Artificial Sequence
  artificial peptide
  MUTAGEN (1)..(1): Xaa stands for N-methyl-glutamic acid
  MUTAGEN (2)..(2): Xaa stands for N-methyl-L-norleucine
  MUTAGEN (3)..(3): Xaa stands for alpha-methyl-alanine
  MUTAGEN (4)..(4): Xaa stands for beta-cyclohexyl-L-alanine
  MUTAGEN (5)..(5): Xaa stands for 4-fluoro-L-phenylalanine
  MUTAGEN (6)..(6): Xaa stands for N-methyl-glutamic acid
  MUTAGEN (9)..(9): Xaa stands for 4-carboxy-L-phenylalanine
  MUTAGEN (10)..(10): Xaa stands for D-lysine
  MUTAGEN (11)..(11): Xaa stands for beta-cyclohexyl-L-alanine
  MUTAGEN (13)..(13): Xaa stands for D-glutamic acid
XXXXXXYYXXXCX

SEQ ID NO: 149 - protein, 13 aa, Artificial Sequence
  artificial peptide
  MUTAGEN (1)..(1): Xaa stands for N-methyl-glutamic acid
  MUTAGEN (2)..(2): Xaa stands for N-methyl-L-norleucine
  MUTAGEN (4)..(4): Xaa stands for beta-cyclohexyl-L-alanine
  MUTAGEN (6)..(6): Xaa stands for D-aspartic acid
  MUTAGEN (9)..(9): Xaa stands for L-alpha,gamma-diamino-butyric acid
  MUTAGEN (11)..(11): Xaa stands for beta-cyclohexyl-L-alanine
  MUTAGEN (13)..(13): Xaa stands for D-glutamic acid
  MOD_RES (13)..(13): AMIDATION
XXSXYXYYXRXCX

SEQ ID NO: 150 - protein, 13 aa, Artificial Sequence
  artificial peptide
  MUTAGEN (1)..(1): Xaa stands for N-methyl-glutamic acid
  MUTAGEN (2)..(2): Xaa stands for N-methyl-L-norleucine
  MUTAGEN (3)..(3): Xaa stands for alpha-methyl-alanine
  MUTAGEN (4)..(4): Xaa stands for beta-cyclohexyl-L-alanine
  MUTAGEN (6)..(6): Xaa stands for D-aspartic acid
  MUTAGEN (9)..(9): Xaa stands for L-alpha,gamma-diamino-butyric acid
  MUTAGEN (11)..(11): Xaa stands for beta-cyclohexyl-L-alanine
  MUTAGEN (13)..(13): Xaa stands for D-glutamic acid
  MOD_RES (13)..(13): AMIDATION
XXXXYXYYXRXCX

SEQ ID NO: 151 - protein, 13 aa, Artificial Sequence
  artificial peptide
  MUTAGEN (1)..(1): Xaa stands for N-methyl-glutamic acid
  MUTAGEN (2)..(2): Xaa stands for N-methyl-L-norleucine
  MUTAGEN (4)..(4): Xaa stands for beta-cyclohexyl-L-alanine
  MUTAGEN (6)..(6): Xaa stands for D-aspartic acid
  MUTAGEN (9)..(9): Xaa stands for L-alpha,gamma-diamino-butyric acid
  MUTAGEN (10)..(10): Xaa stands for D-arginine
  MUTAGEN (11)..(11): Xaa stands for beta-cyclohexyl-L-alanine
  MUTAGEN (13)..(13): Xaa stands for D-glutamic acid
  MOD_RES (13)..(13): AMIDATION
XXSXYXYYXXXCX

SEQ ID NO: 152 - protein, 13 aa, Artificial Sequence
  artificial peptide
  MUTAGEN (1)..(1): Xaa stands for N-methyl-glutamic acid
  MUTAGEN (2)..(2): Xaa stands for N-methyl-L-norleucine
  MUTAGEN (3)..(3): Xaa stands for alpha-methyl-alanine
  MUTAGEN (4)..(4): Xaa stands for beta-cyclohexyl-L-alanine
  MUTAGEN (6)..(6): Xaa stands for D-aspartic acid
  MUTAGEN (9)..(9): Xaa stands for L-alpha,gamma-diamino-butyric acid
  MUTAGEN (10)..(10): Xaa stands for D-arginine
  MUTAGEN (11)..(11): Xaa stands for beta-cyclohexyl-L-alanine
  MUTAGEN (13)..(13): Xaa stands for D-glutamic acid
  MOD_RES (13)..(13): AMIDATION
XXXXYXYYXXXCX

SEQ ID NO: 153 - protein, 13 aa, Artificial Sequence
  artificial peptide
  MUTAGEN (1)..(1): Xaa stands for N-methyl-glutamic acid
  MUTAGEN (2)..(2): Xaa stands for N-methyl-L-norleucine
  MUTAGEN (3)..(3): Xaa stands for alpha-methyl-alanine
  MUTAGEN (4)..(4): Xaa stands for beta-cyclohexyl-L-alanine
  MUTAGEN (5)..(5): Xaa stands for 4-fluoro-L-phenylalanine
  MUTAGEN (6)..(6): Xaa stands for alpha-methyl-alanine
  MUTAGEN (9)..(9): Xaa stands for 4-carboxy-L-phenylalanine
  MUTAGEN (10)..(10): Xaa stands for D-lysine
  MUTAGEN (11)..(11): Xaa stands for beta-cyclohexyl-L-alanine
  MUTAGEN (13)..(13): Xaa stands for D-glutamic acid
  MOD_RES (13)..(13): AMIDATION
XXXXXXYYXXXCX

SEQ ID NO: 154 - protein, 13 aa, Artificial Sequence
  artificial peptide
  MUTAGEN (1)..(1): Xaa stands for N-methyl-glutamic acid
  MUTAGEN (2)..(2): Xaa stands for N-methyl-L-norleucine
  MUTAGEN (3)..(3): Xaa stands for alpha-methyl-alanine
  MUTAGEN (4)..(4): Xaa stands for beta-cyclohexyl-L-alanine
  MUTAGEN (5)..(5): Xaa stands for 4-fluoro-L-phenylalanine
  MUTAGEN (6)..(6): Xaa stands for alpha-methyl-alanine
  MUTAGEN (9)..(9): Xaa stands for (S)-2-amino-5-ureidopentanoic acid
  MUTAGEN (10)..(10): Xaa stands for (S)-2-amino-3-(piperidin-4-yl)-propanoic acid
  MUTAGEN (11)..(11): Xaa stands for beta-cyclohexyl-L-alanine
  MUTAGEN (13)..(13): Xaa stands for D-glutamic acid
  MOD_RES (13)..(13): AMIDATION
XXXXXXYYXXXCX

SEQ ID NO: 155 - protein, 13 aa, Artificial Sequence
  artificial peptide
  MUTAGEN (1)..(1): Xaa stands for N-methyl-glutamic acid
  MUTAGEN (2)..(2): Xaa stands for N-methyl-L-norleucine
  MUTAGEN (3)..(3): Xaa stands for alpha-methyl-alanine
  MUTAGEN (4)..(4): Xaa stands for beta-cyclohexyl-L-alanine
  MUTAGEN (5)..(5): Xaa stands for 4-fluoro-L-phenylalanine
  MUTAGEN (6)..(6): Xaa stands for alpha-methyl-alanine
  MUTAGEN (9)..(9): Xaa stands for 4-carboxy-L-phenylalanine
  MUTAGEN (10)..(10): Xaa stands for (S)-2-amino-3-(piperidin-4-yl)-propanoic acid
  MUTAGEN (11)..(11): Xaa stands for beta-cyclohexyl-L-alanine
  MUTAGEN (13)..(13): Xaa stands for D-glutamic acid
XXXXXXYYXXXCX

SEQ ID NO: 156 - protein, 13 aa, Artificial Sequence
  artificial peptide
  MUTAGEN (1)..(1): Xaa stands for N-methyl-glutamic acid
  MUTAGEN (2)..(2): Xaa stands for N-methyl-L-norleucine
  MUTAGEN (3)..(3): Xaa stands for alpha-methyl-alanine
  MUTAGEN (4)..(4): Xaa stands for beta-cyclohexyl-L-alanine
  MUTAGEN (5)..(5): Xaa stands for 4-fluoro-L-phenylalanine
  MUTAGEN (6)..(6): Xaa stands for D-aspartic acid
  MUTAGEN (9)..(9): Xaa stands for (S)-2-amino-5-ureidopentanoic acid
  MUTAGEN (10)..(10): Xaa stands for (S)-2-amino-3-(piperidin-4-yl)-propanoic acid
  MUTAGEN (11)..(11): Xaa stands for beta-cyclohexyl-L-alanine
  MUTAGEN (13)..(13): Xaa stands for D-glutamic acid
  MOD_RES (13)..(13): AMIDATION
XXXXXXYYXXXCX

SEQ ID NO: 157 - protein, 13 aa, Artificial Sequence
  artificial peptide
  MUTAGEN (1)..(1): Xaa stands for N-methyl-glutamic acid
  MUTAGEN (2)..(2): Xaa stands for N-methyl-L-norleucine
  MUTAGEN (3)..(3): Xaa stands for alpha-methyl-alanine
  MUTAGEN (4)..(4): Xaa stands for beta-cyclohexyl-L-alanine
  MUTAGEN (5)..(5): Xaa stands for 4-fluoro-L-phenylalanine
  MUTAGEN (6)..(6): Xaa stands for D-aspartic acid
  MUTAGEN (9)..(9): Xaa stands for 4-carboxy-L-phenylalanine
  MUTAGEN (10)..(10): Xaa stands for D-lysine
  MUTAGEN (11)..(11): Xaa stands for beta-cyclohexyl-L-alanine
  MUTAGEN (13)..(13): Xaa stands for D-glutamic acid
  MOD_RES (13)..(13): AMIDATION
XXXXXXYYXXXCX

SEQ ID NO: 158 - protein, 13 aa, Artificial Sequence
  artificial peptide
  MUTAGEN (1)..(1): Xaa stands for N-methyl-glutamic acid
  MUTAGEN (2)..(2): Xaa stands for N-methyl-L-norleucine
  MUTAGEN (3)..(3): Xaa stands for alpha-methyl-alanine
  MUTAGEN (4)..(4): Xaa stands for beta-cyclohexyl-L-alanine
  MUTAGEN (5)..(5): Xaa stands for 4-fluoro-L-phenylalanine
  MUTAGEN (6)..(6): Xaa stands for D-aspartic acid
  MUTAGEN (9)..(9): Xaa stands for 4-carboxy-L-phenylalanine
  MUTAGEN (10)..(10): Xaa stands for (S)-2-amino-3-(piperidin-4-yl)-propanoic acid
  MUTAGEN (11)..(11): Xaa stands for beta-cyclohexyl-L-alanine
  MUTAGEN (13)..(13): Xaa stands for D-glutamic acid
XXXXXXYYXXXCX

SEQ ID NO: 159 - protein, 13 aa, Artificial Sequence
  artificial peptide
  MUTAGEN (1)..(1): Xaa stands for N-methyl-glutamic acid
  MUTAGEN (2)..(2): Xaa stands for N-methyl-L-norleucine
  MUTAGEN (3)..(3): Xaa stands for alpha-methyl-alanine
  MUTAGEN (4)..(4): Xaa stands for beta-cyclohexyl-L-alanine
  MUTAGEN (5)..(5): Xaa stands for 4-fluoro-L-phenylalanine
  MUTAGEN (6)..(6): Xaa stands for alpha-methyl-alanine
  MUTAGEN (9)..(9): Xaa stands for (S)-2-amino-5-ureidopentanoic acid
  MUTAGEN (10)..(10): Xaa stands for D-lysine
  MUTAGEN (11)..(11): Xaa stands for beta-cyclohexyl-L-alanine
  MUTAGEN (13)..(13): Xaa stands for D-glutamic acid
  MOD_RES (13)..(13): AMIDATION
XXXXXXYYXXXCX

SEQ ID NO: 160 - protein, 13 aa, Artificial Sequence
  artificial peptide
  MUTAGEN (1)..(1): Xaa stands for N-methyl-glutamic acid
  MUTAGEN (2)..(2): Xaa stands for N-methyl-L-norleucine
  MUTAGEN (3)..(3): Xaa stands for alpha-methyl-alanine
  MUTAGEN (4)..(4): Xaa stands for beta-cyclohexyl-L-alanine
  MUTAGEN (5)..(5): Xaa stands for 4-fluoro-L-phenylalanine
  MUTAGEN (6)..(6): Xaa stands for alpha-methyl-alanine
  MUTAGEN (9)..(9): Xaa stands for (S)-2-amino-5-ureidopentanoic acid
  MUTAGEN (10)..(10): Xaa stands for (S)-2-amino-3-(piperidin-4-yl)-propanoic acid
  MUTAGEN (11)..(11): Xaa stands for beta-cyclohexyl-L-alanine
  MUTAGEN (13)..(13): Xaa stands for D-glutamic acid
XXXXXXYYXXXCX

SEQ ID NO: 161 - protein, 13 aa, Artificial Sequence
  artificial peptide
  MUTAGEN (1)..(1): Xaa stands for N-methyl-glutamic acid
  MUTAGEN (2)..(2): Xaa stands for N-methyl-L-norleucine
  MUTAGEN (3)..(3): Xaa stands for alpha-methyl-alanine
  MUTAGEN (4)..(4): Xaa stands for beta-cyclohexyl-L-alanine
  MUTAGEN (5)..(5): Xaa stands for 4-fluoro-L-phenylalanine
  MUTAGEN (6)..(6): Xaa stands for alpha-methyl-alanine
  MUTAGEN (9)..(9): Xaa stands for 4-carboxy-L-phenylalanine
  MUTAGEN (10)..(10): Xaa stands for D-lysine
  MUTAGEN (11)..(11): Xaa stands for beta-cyclohexyl-L-alanine
  MUTAGEN (13)..(13): Xaa stands for D-glutamic acid
XXXXXXYYXXXCX

SEQ ID NO: 162 - protein, 13 aa, Artificial Sequence
  artificial peptide
  MUTAGEN (1)..(1): Xaa stands for N-methyl-glutamic acid
  MUTAGEN (2)..(2): Xaa stands for N-methyl-L-norleucine
  MUTAGEN (3)..(3): Xaa stands for alpha-methyl-alanine
  MUTAGEN (4)..(4): Xaa stands for beta-cyclohexyl-L-alanine
  MUTAGEN (5)..(5): Xaa stands for 4-fluoro-L-phenylalanine
  MUTAGEN (6)..(6): Xaa stands for D-aspartic acid
  MUTAGEN (9)..(9): Xaa stands for (S)-2-amino-5-ureidopentanoic acid
  MUTAGEN (10)..(10): Xaa stands for D-lysine
  MUTAGEN (11)..(11): Xaa stands for beta-cyclohexyl-L-alanine
  MUTAGEN (13)..(13): Xaa stands for D-glutamic acid
  MOD_RES (13)..(13): AMIDATION
XXXXXXYYXXXCX

SEQ ID NO: 163 - protein, 13 aa, Artificial Sequence
  artificial peptide
  MUTAGEN (1)..(1): Xaa stands for N-methyl-glutamic acid
  MUTAGEN (2)..(2): Xaa stands for N-methyl-L-norleucine
  MUTAGEN (3)..(3): Xaa stands for alpha-methyl-alanine
  MUTAGEN (4)..(4): Xaa stands for beta-cyclohexyl-L-alanine
  MUTAGEN (5)..(5): Xaa stands for 4-fluoro-L-phenylalanine
  MUTAGEN (6)..(6): Xaa stands for D-aspartic acid
  MUTAGEN (9)..(9): Xaa stands for (S)-2-amino-5-ureidopentanoic acid
  MUTAGEN (10)..(10): Xaa stands for (S)-2-amino-3-(piperidin-4-yl)-propanoic acid
  MUTAGEN (11)..(11): Xaa stands for beta-cyclohexyl-L-alanine
  MUTAGEN (13)..(13): Xaa stands for D-glutamic acid
XXXXXXYYXXXCX

SEQ ID NO: 164 - protein, 13 aa, Artificial Sequence
  artificial peptide
  MUTAGEN (1)..(1): Xaa stands for N-methyl-glutamic acid
  MUTAGEN (2)..(2): Xaa stands for N-methyl-L-norleucine
  MUTAGEN (3)..(3): Xaa stands for alpha-methyl-alanine
  MUTAGEN (4)..(4): Xaa stands for beta-cyclohexyl-L-alanine
  MUTAGEN (5)..(5): Xaa stands for 4-fluoro-L-phenylalanine
  MUTAGEN (6)..(6): Xaa stands for alpha-methyl-alanine
  MUTAGEN (9)..(9): Xaa stands for (S)-2-amino-5-ureidopentanoic acid
  MUTAGEN (10)..(10): Xaa stands for D-lysine
  MUTAGEN (11)..(11): Xaa stands for beta-cyclohexyl-L-alanine
  MUTAGEN (13)..(13): Xaa stands for D-glutamic acid
XXXXXXYYXXXCX

SEQ ID NO: 165 - protein, 13 aa, Artificial Sequence
  artificial peptide
  MUTAGEN (1)..(1): Xaa stands for N-methyl-glutamic acid
  MUTAGEN (2)..(2): Xaa stands for N-methyl-L-norleucine
  MUTAGEN (3)..(3): Xaa stands for alpha-methyl-alanine
  MUTAGEN (4)..(4): Xaa stands for beta-cyclohexyl-L-alanine
  MUTAGEN (5)..(5): Xaa stands for 4-fluoro-L-phenylalanine
  MUTAGEN (6)..(6): Xaa stands for alpha-methyl-alanine
  MUTAGEN (9)..(9): Xaa stands for L-alpha,gamma-diamino-butyric acid
  MUTAGEN (11)..(11): Xaa stands for beta-cyclohexyl-L-alanine
  MUTAGEN (13)..(13): Xaa stands for D-glutamic acid
  MOD_RES (13)..(13): AMIDATION
XXXXXXYYXRXCX

SEQ ID NO: 166 - protein, 13 aa, Artificial Sequence
  artificial peptide
  MUTAGEN (1)..(1): Xaa stands for N-methyl-glutamic acid
  MUTAGEN (2)..(2): Xaa stands for N-methyl-L-norleucine
  MUTAGEN (3)..(3): Xaa stands for alpha-methyl-alanine
  MUTAGEN (4)..(4): Xaa stands for beta-cyclohexyl-L-alanine
  MUTAGEN (5)..(5): Xaa stands for 4-fluoro-L-phenylalanine
  MUTAGEN (6)..(6): Xaa stands for alpha-methyl-alanine
  MUTAGEN (9)..(9): Xaa stands for L-alpha,gamma-diamino-butyric acid
  MUTAGEN (10)..(10): Xaa stands for D-lysine
  MUTAGEN (11)..(11): Xaa stands for beta-cyclohexyl-L-alanine
  MUTAGEN (13)..(13): Xaa stands for D-glutamic acid
  MOD_RES (13)..(13): AMIDATION
XXXXXXYYXXXCX

SEQ ID NO: 167 - protein, 13 aa, Artificial Sequence
  artificial peptide
  MUTAGEN (1)..(1): Xaa stands for N-methyl-glutamic acid
  MUTAGEN (2)..(2): Xaa stands for N-methyl-L-norleucine
  MUTAGEN (3)..(3): Xaa stands for alpha-methyl-alanine
  MUTAGEN (4)..(4): Xaa stands for beta-cyclohexyl-L-alanine
  MUTAGEN (5)..(5): Xaa stands for 4-fluoro-L-phenylalanine
  MUTAGEN (6)..(6): Xaa stands for alpha-methyl-alanine
  MUTAGEN (9)..(9): Xaa stands for L-alpha,gamma-diamino-butyric acid
  MUTAGEN (10)..(10): Xaa stands for D-arginine
  MUTAGEN (11)..(11): Xaa stands for beta-cyclohexyl-L-alanine
  MUTAGEN (13)..(13): Xaa stands for D-glutamic acid
  MOD_RES (13)..(13): AMIDATION
XXXXXXYYXXXCX

SEQ ID NO: 168 - protein, 13 aa, Artificial Sequence
  artificial peptide
  MUTAGEN (1)..(1): Xaa stands for N-methyl-glutamic acid
  MUTAGEN (2)..(2): Xaa stands for N-methyl-L-norleucine
  MUTAGEN (3)..(3): Xaa stands for alpha-methyl-alanine
  MUTAGEN (4)..(4): Xaa stands for beta-cyclohexyl-L-alanine
  MUTAGEN (5)..(5): Xaa stands for 4-fluoro-L-phenylalanine
  MUTAGEN (6)..(6): Xaa stands for alpha-methyl-alanine
  MUTAGEN (9)..(9): Xaa stands for L-alpha,gamma-diamino-butyric acid
  MUTAGEN (10)..(10): Xaa stands for (S)-2-amino-3-(piperidin-4-yl)-propanoic acid
  MUTAGEN (11)..(11): Xaa stands for beta-cyclohexyl-L-alanine
  MUTAGEN (13)..(13): Xaa stands for D-glutamic acid
  MOD_RES (13)..(13): AMIDATION
XXXXXXYYXXXCX

SEQ ID NO: 169 - protein, 13 aa, Artificial Sequence
  artificial peptide
  MUTAGEN (1)..(1): Xaa stands for N-methyl-glutamic acid
  MUTAGEN (2)..(2): Xaa stands for N-methyl-L-norleucine
  MUTAGEN (3)..(3): Xaa stands for alpha-methyl-alanine
  MUTAGEN (4)..(4): Xaa stands for beta-cyclohexyl-L-alanine
  MUTAGEN (5)..(5): Xaa stands for 4-fluoro-L-phenylalanine
  MUTAGEN (6)..(6): Xaa stands for D-aspartic acid
  MUTAGEN (9)..(9): Xaa stands for L-alpha,gamma-diamino-butyric acid
  MUTAGEN (11)..(11): Xaa stands for beta-cyclohexyl-L-alanine
  MUTAGEN (13)..(13): Xaa stands for D-glutamic acid
  MOD_RES (13)..(13): AMIDATION
XXXXXXYYXRXCX

SEQ ID NO: 170 - protein, 13 aa, Artificial Sequence
  artificial peptide
  MUTAGEN (1)..(1): Xaa stands for N-methyl-glutamic acid
  MUTAGEN (2)..(2): Xaa stands for N-methyl-L-norleucine
  MUTAGEN (3)..(3): Xaa stands for alpha-methyl-alanine
  MUTAGEN (4)..(4): Xaa stands for beta-cyclohexyl-L-alanine
  MUTAGEN (5)..(5): Xaa stands for 4-fluoro-L-phenylalanine
  MUTAGEN (6)..(6): Xaa stands for D-aspartic acid
  MUTAGEN (9)..(9): Xaa stands for L-alpha,gamma-diamino-butyric acid
  MUTAGEN (10)..(10): Xaa stands for D-lysine
  MUTAGEN (11)..(11): Xaa stands for beta-cyclohexyl-L-alanine
  MUTAGEN (13)..(13): Xaa stands for D-glutamic acid
  MOD_RES (13)..(13): AMIDATION
XXXXXXYYXXXCX

SEQ ID NO: 171 - protein, 13 aa, Artificial Sequence
  artificial peptide
  MUTAGEN (1)..(1): Xaa stands for N-methyl-glutamic acid
  MUTAGEN (2)..(2): Xaa stands for N-methyl-L-norleucine
  MUTAGEN (3)..(3): Xaa stands for alpha-methyl-alanine
  MUTAGEN (4)..(4): Xaa stands for beta-cyclohexyl-L-alanine
  MUTAGEN (5)..(5): Xaa stands for 4-fluoro-L-phenylalanine
  MUTAGEN (6)..(6): Xaa stands for D-aspartic acid
  MUTAGEN (9)..(9): Xaa stands for L-alpha,gamma-diamino-butyric acid
  MUTAGEN (10)..(10): Xaa stands for D-arginine
  MUTAGEN (11)..(11): Xaa stands for beta-cyclohexyl-L-alanine
  MUTAGEN (13)..(13): Xaa stands for D-glutamic acid
  MOD_RES (13)..(13): AMIDATION
XXXXXXYYXXXCX

SEQ ID NO: 172 - protein, 13 aa, Artificial Sequence
  artificial peptide
  MUTAGEN (1)..(1): Xaa stands for N-methyl-glutamic acid
  MUTAGEN (2)..(2): Xaa stands for N-methyl-L-norleucine
  MUTAGEN (3)..(3): Xaa stands for alpha-methyl-alanine
  MUTAGEN (4)..(4): Xaa stands for beta-cyclohexyl-L-alanine
  MUTAGEN (5)..(5): Xaa stands for 4-fluoro-L-phenylalanine
  MUTAGEN (6)..(6): Xaa stands for D-aspartic acid
  MUTAGEN (9)..(9): Xaa stands for L-alpha,gamma-diamino-butyric acid
  MUTAGEN (10)..(10): Xaa stands for (S)-2-amino-3-(piperidin-4-yl)-propanoic acid
  MUTAGEN (11)..(11): Xaa stands for beta-cyclohexyl-L-alanine
  MUTAGEN (13)..(13): Xaa stands for D-glutamic acid
  MOD_RES (13)..(13): AMIDATION
XXXXXXYYXXXCX

SEQ ID NO: 173 - protein, 13 aa, Artificial Sequence
  artificial peptide
  MUTAGEN (1)..(1): Xaa stands for N-methyl-glutamic acid
  MUTAGEN (2)..(2): Xaa stands for N-methyl-L-norleucine
  MUTAGEN (3)..(3): Xaa stands for alpha-methyl-alanine
  MUTAGEN (4)..(4): Xaa stands for beta-cyclohexyl-L-alanine
  MUTAGEN (5)..(5): Xaa stands for 4-fluoro-L-phenylalanine
  MUTAGEN (6)..(6): Xaa stands for 4-amino-1-(carboxymethyl)piperidin-4-carboxylic acid
  MUTAGEN (9)..(9): Xaa stands for 4-carboxy-L-phenylalanine
  MUTAGEN (10)..(10): Xaa stands for (S)-2-amino-3-(piperidin-4-yl)-propanoic acid
  MUTAGEN (11)..(11): Xaa stands for beta-cyclohexyl-L-alanine
  MUTAGEN (13)..(13): Xaa stands for D-glutamic acid
  MOD_RES (13)..(13): AMIDATION
XXXXXXYYXXXCX

SEQ ID NO: 174 - protein, 13 aa, Artificial Sequence
  artificial peptide
  MUTAGEN (1)..(1): Xaa stands for N-methyl-glutamic acid
  MUTAGEN (2)..(2): Xaa stands for N-methyl-L-norleucine
  MUTAGEN (3)..(3): Xaa stands for alpha-methyl-alanine
  MUTAGEN (4)..(4): Xaa stands for beta-cyclohexyl-L-alanine
  MUTAGEN (5)..(5): Xaa stands for 4-fluoro-L-phenylalanine
  MUTAGEN (6)..(6): Xaa stands for N-methyl-glycine
  MUTAGEN (9)..(9): Xaa stands for 4-carboxy-L-phenylalanine
  MUTAGEN (10)..(10): Xaa stands for (S)-2-amino-3-(piperidin-4-yl)-propanoic acid
  MUTAGEN (11)..(11): Xaa stands for beta-cyclohexyl-L-alanine
  MUTAGEN (13)..(13): Xaa stands for D-glutamic acid
  MOD_RES (13)..(13): AMIDATION
XXXXXXYYXXXCX

SEQ ID NO: 175 - protein, 13 aa, Artificial Sequence
  artificial peptide
  MUTAGEN (1)..(1): Xaa stands for N-methyl-glutamic acid
  MUTAGEN (2)..(2): Xaa stands for N-methyl-L-norleucine
  MUTAGEN (3)..(3): Xaa stands for alpha-methyl-alanine
  MUTAGEN (4)..(4): Xaa stands for beta-cyclohexyl-L-alanine
  MUTAGEN (5)..(5): Xaa stands for 4-fluoro-L-phenylalanine
  MUTAGEN (6)..(6): Xaa stands for N-methyl-D-glutamic acid
  MUTAGEN (9)..(9): Xaa stands for 4-carboxy-L-phenylalanine
  MUTAGEN (10)..(10): Xaa stands for (S)-2-amino-3-(piperidin-4-yl)-propanoic acid
  MUTAGEN (11)..(11): Xaa stands for beta-cyclohexyl-L-alanine
  MUTAGEN (13)..(13): Xaa stands for D-glutamic acid
  MOD_RES (13)..(13): AMIDATION
XXXXXXYYXXXCX

SEQ ID NO: 176 - protein, 13 aa, Artificial Sequence
  artificial peptide
  MUTAGEN (1)..(1): Xaa stands for N-methyl-glutamic acid
  MUTAGEN (2)..(2): Xaa stands for N-methyl-L-norleucine
  MUTAGEN (3)..(3): Xaa stands for alpha-methyl-alanine
  MUTAGEN (4)..(4): Xaa stands for beta-cyclohexyl-L-alanine
  MUTAGEN (5)..(5): Xaa stands for 4-fluoro-L-phenylalanine
  MUTAGEN (6)..(6): Xaa stands for N-methyl-D-aspartic acid
  MUTAGEN (9)..(9): Xaa stands for 4-carboxy-L-phenylalanine
  MUTAGEN (10)..(10): Xaa stands for (S)-2-amino-3-(piperidin-4-yl)-propanoic acid
  MUTAGEN (11)..(11): Xaa stands for beta-cyclohexyl-L-alanine
  MUTAGEN (13)..(13): Xaa stands for D-glutamic acid
  MOD_RES (13)..(13): AMIDATION
XXXXXXYYXXXCX

SEQ ID NO: 177 - protein, 13 aa, Artificial Sequence
  artificial peptide
  MUTAGEN (1)..(1): Xaa stands for 3-pyridyl-L-alanine
  MUTAGEN (2)..(2): Xaa stands for N-methyl-L-norleucine
  MUTAGEN (3)..(3): Xaa stands for alpha-methyl-alanine
  MUTAGEN (4)..(4): Xaa stands for beta-cyclohexyl-L-alanine
  MUTAGEN (5)..(5): Xaa stands for 4-fluoro-L-phenylalanine
  MUTAGEN (6)..(6): Xaa stands for D-aspartic acid
  MUTAGEN (9)..(9): Xaa stands for (S)-2-amino-5-ureidopentanoic acid
  MUTAGEN (10)..(10): Xaa stands for D-lysine
  MUTAGEN (11)..(11): Xaa stands for beta-cyclohexyl-L-alanine
  MUTAGEN (13)..(13): Xaa stands for D-glutamic acid
  MOD_RES (13)..(13): AMIDATION
XXXXXXYYXXXCX

SEQ ID NO: 178 - protein, 13 aa, Artificial Sequence
  artificial peptide
  MUTAGEN (1)..(1): Xaa stands for 3-pyridyl-L-alanine
  MUTAGEN (2)..(2): Xaa stands for N-methyl-L-norleucine
  MUTAGEN (3)..(3): Xaa stands for alpha-methyl-alanine
  MUTAGEN (4)..(4): Xaa stands for (S)-2-amino-3-(2,3-dihydro-1H-indene-2-yl)-propanoic acid
  MUTAGEN (5)..(5): Xaa stands for 4-fluoro-L-phenylalanine
  MUTAGEN (6)..(6): Xaa stands for D-aspartic acid
  MUTAGEN (9)..(9): Xaa stands for (S)-2-amino-5-ureidopentanoic acid
  MUTAGEN (10)..(10): Xaa stands for D-lysine
  MUTAGEN (11)..(11): Xaa stands for beta-cyclohexyl-L-alanine
  MUTAGEN (13)..(13): Xaa stands for D-glutamic acid
  MOD_RES (13)..(13): AMIDATION
XXXXXXYYXXXCX

SEQ ID NO: 179 - protein, 13 aa, Artificial Sequence
  artificial peptide
  MUTAGEN (1)..(1): Xaa stands for 3-pyridyl-L-alanine
  MUTAGEN (2)..(2): Xaa stands for N-methyl-L-norleucine
  MUTAGEN (3)..(3): Xaa stands for alpha-methyl-alanine
  MUTAGEN (4)..(4): Xaa stands for (S)-2-amino-3-(2,3-dihydro-1H-indene-2-yl)-propanoic acid
  MUTAGEN (5)..(5): Xaa stands for 4-fluoro-L-phenylalanine
  MUTAGEN (6)..(6): Xaa stands for N-methyl-D-alanine
  MUTAGEN (9)..(9): Xaa stands for (S)-2-amino-5-ureidopentanoic acid
  MUTAGEN (10)..(10): Xaa stands for D-lysine
  MUTAGEN (11)..(11): Xaa stands for beta-cyclohexyl-L-alanine
  MUTAGEN (13)..(13): Xaa stands for D-glutamic acid
  MOD_RES (13)..(13): AMIDATION
XXXXXXYYXXXCX

SEQ ID NO: 180 - protein, 13 aa, Artificial Sequence
  artificial peptide
  MUTAGEN (1)..(1): Xaa stands for 3-pyridyl-L-alanine
  MUTAGEN (2)..(2): Xaa stands for N-methyl-L-norleucine
  MUTAGEN (3)..(3): Xaa stands for alpha-methyl-alanine
  MUTAGEN (4)..(4): Xaa stands for (S)-2-amino-3-(2,3-dihydro-1H-indene-2-yl)-propanoic acid
  MUTAGEN (5)..(5): Xaa stands for 4-fluoro-L-phenylalanine
  MUTAGEN (6)..(6): Xaa stands for N-methyl-D-alanine
  MUTAGEN (7)..(7): Xaa stands for (S)-2-amino-3-(4-hydroxy-methylphenyl) -propanoic acid
  MUTAGEN (9)..(9): Xaa stands for (S)-2-amino-5-ureidopentanoic acid
  MUTAGEN (10)..(10): Xaa stands for D-lysine
  MUTAGEN (11)..(11): Xaa stands for beta-cyclohexyl-L-alanine
  MUTAGEN (13)..(13): Xaa stands for D-glutamic acid
  MOD_RES (13)..(13): AMIDATION
XXXXXXXYXXXCX

SEQ ID NO: 181 - protein, 13 aa, Artificial Sequence
  artificial peptide
  MUTAGEN (1)..(1): Xaa stands for 3-pyridyl-L-alanine
  MUTAGEN (2)..(2): Xaa stands for N-methyl-L-norleucine
  MUTAGEN (3)..(3): Xaa stands for alpha-methyl-alanine
  MUTAGEN (4)..(4): Xaa stands for beta-cyclohexyl-L-alanine
  MUTAGEN (5)..(5): Xaa stands for 4-fluoro-L-phenylalanine
  MUTAGEN (6)..(6): Xaa stands for N-methyl-D-alanine
  MUTAGEN (9)..(9): Xaa stands for (S)-2-amino-5-ureidopentanoic acid
  MUTAGEN (10)..(10): Xaa stands for D-lysine
  MUTAGEN (11)..(11): Xaa stands for beta-cyclohexyl-L-alanine
  MUTAGEN (13)..(13): Xaa stands for D-glutamic acid
  MOD_RES (13)..(13): AMIDATION
XXXXXXYYXXXCX

SEQ ID NO: 182 - protein, 13 aa, Artificial Sequence
  artificial peptide
  MUTAGEN (1)..(1): Xaa stands for 3-pyridyl-L-alanine
  MUTAGEN (2)..(2): Xaa stands for N-methyl-L-norleucine
  MUTAGEN (3)..(3): Xaa stands for alpha-methyl-alanine
  MUTAGEN (4)..(4): Xaa stands for beta-cyclohexyl-L-alanine
  MUTAGEN (5)..(5): Xaa stands for 4-fluoro-L-phenylalanine
  MUTAGEN (6)..(6): Xaa stands for N-methyl-D-alanine
  MUTAGEN (7)..(7): Xaa stands for (S)-2-amino-3-(4-hydroxy-methylphenyl) -propanoic acid
  MUTAGEN (9)..(9): Xaa stands for (S)-2-amino-5-ureidopentanoic acid
  MUTAGEN (10)..(10): Xaa stands for D-lysine
  MUTAGEN (11)..(11): Xaa stands for beta-cyclohexyl-L-alanine
  MUTAGEN (13)..(13): Xaa stands for D-glutamic acid
  MOD_RES (13)..(13): AMIDATION
XXXXXXXYXXXCX

SEQ ID NO: 183 - protein, 13 aa, Artificial Sequence
  artificial peptide
  MUTAGEN (1)..(1): Xaa stands for N-methyl-glutamic acid
  MUTAGEN (2)..(2): Xaa stands for N-methyl-L-norleucine
  MUTAGEN (3)..(3): Xaa stands for alpha-methyl-alanine
  MUTAGEN (4)..(4): Xaa stands for (S)-2-amino-3-(2,3-dihydro-1H-indene-2-yl)-propanoic acid
  MUTAGEN (5)..(5): Xaa stands for 4-fluoro-L-phenylalanine
  MUTAGEN (6)..(6): Xaa stands for D-aspartic acid
  MUTAGEN (9)..(9): Xaa stands for (S)-2-amino-5-ureidopentanoic acid
  MUTAGEN (10)..(10): Xaa stands for D-lysine
  MUTAGEN (11)..(11): Xaa stands for beta-cyclohexyl-L-alanine
  MUTAGEN (13)..(13): Xaa stands for D-glutamic acid
  MOD_RES (13)..(13): AMIDATION
XXXXXXYYXXXCX

SEQ ID NO: 184 - protein, 13 aa, Artificial Sequence
  artificial peptide
  MUTAGEN (1)..(1): Xaa stands for N-methyl-glutamic acid
  MUTAGEN (2)..(2): Xaa stands for N-methyl-L-norleucine
  MUTAGEN (3)..(3): Xaa stands for alpha-methyl-alanine
  MUTAGEN (4)..(4): Xaa stands for (S)-2-amino-3-(2,3-dihydro-1H-indene-2-yl)-propanoic acid
  MUTAGEN (5)..(5): Xaa stands for 4-fluoro-L-phenylalanine
  MUTAGEN (6)..(6): Xaa stands for N-methyl-D-alanine
  MUTAGEN (9)..(9): Xaa stands for (S)-2-amino-5-ureidopentanoic acid
  MUTAGEN (10)..(10): Xaa stands for D-lysine
  MUTAGEN (11)..(11): Xaa stands for beta-cyclohexyl-L-alanine
  MUTAGEN (13)..(13): Xaa stands for D-glutamic acid
  MOD_RES (13)..(13): AMIDATION
XXXXXXYYXXXCX

SEQ ID NO: 185 - protein, 13 aa, Artificial Sequence
  artificial peptide
  MUTAGEN (1)..(1): Xaa stands for N-methyl-glutamic acid
  MUTAGEN (2)..(2): Xaa stands for N-methyl-L-norleucine
  MUTAGEN (3)..(3): Xaa stands for alpha-methyl-alanine
  MUTAGEN (4)..(4): Xaa stands for (S)-2-amino-3-(2,3-dihydro-1H-indene-2-yl)-propanoic acid
  MUTAGEN (5)..(5): Xaa stands for 4-fluoro-L-phenylalanine
  MUTAGEN (6)..(6): Xaa stands for N-methyl-D-alanine
  MUTAGEN (7)..(7): Xaa stands for (S)-2-amino-3-(4-hydroxy-methylphenyl) -propanoic acid
  MUTAGEN (9)..(9): Xaa stands for (S)-2-amino-5-ureidopentanoic acid
  MUTAGEN (10)..(10): Xaa stands for D-lysine
  MUTAGEN (11)..(11): Xaa stands for beta-cyclohexyl-L-alanine
  MUTAGEN (13)..(13): Xaa stands for D-glutamic acid
  MOD_RES (13)..(13): AMIDATION
XXXXXXXYXXXCX

SEQ ID NO: 186 - protein, 13 aa, Artificial Sequence
  artificial peptide
  MUTAGEN (1)..(1): Xaa stands for N-methyl-glutamic acid
  MUTAGEN (2)..(2): Xaa stands for N-methyl-L-norleucine
  MUTAGEN (3)..(3): Xaa stands for alpha-methyl-alanine
  MUTAGEN (4)..(4): Xaa stands for (S)-2-amino-3-(2,3-dihydro-1H-indene-2-yl)-propanoic acid
  MUTAGEN (5)..(5): Xaa stands for 4-fluoro-L-phenylalanine
  MUTAGEN (6)..(6): Xaa stands for N-methylglycine
  MUTAGEN (7)..(7): Xaa stands for (S)-2-amino-3-(4-hydroxy-methylphenyl) -propanoic acid
  MUTAGEN (9)..(9): Xaa stands for (S)-2-amino-5-ureidopentanoic acid
  MUTAGEN (10)..(10): Xaa stands for D-lysine
  MUTAGEN (11)..(11): Xaa stands for beta-cyclohexyl-L-alanine
  MUTAGEN (13)..(13): Xaa stands for D-glutamic acid
  MOD_RES (13)..(13): AMIDATION
XXXXXXXYXXXCX

SEQ ID NO: 187 - protein, 13 aa, Artificial Sequence
  artificial peptide
  MUTAGEN (1)..(1): Xaa stands for N-methyl-glutamic acid
  MUTAGEN (2)..(2): Xaa stands for N-methyl-L-norleucine
  MUTAGEN (3)..(3): Xaa stands for alpha-methyl-alanine
  MUTAGEN (4)..(4): Xaa stands for beta-cyclohexyl-L-alanine
  MUTAGEN (5)..(5): Xaa stands for 4-fluoro-L-phenylalanine
  MUTAGEN (6)..(6): Xaa stands for D-aspartic acid
  MUTAGEN (7)..(7): Xaa stands for (S)-2-amino-3-(4-hydroxy-methylphenyl) -propanoic acid
  MUTAGEN (9)..(9): Xaa stands for (S)-2-amino-5-ureidopentanoic acid
  MUTAGEN (10)..(10): Xaa stands for D-lysine
  MUTAGEN (11)..(11): Xaa stands for beta-cyclohexyl-L-alanine
  MUTAGEN (13)..(13): Xaa stands for D-glutamic acid
  MOD_RES (13)..(13): AMIDATION
XXXXXXXYXXXCX

SEQ ID NO: 188 - protein, 13 aa, Artificial Sequence
  artificial peptide
  MUTAGEN (1)..(1): Xaa stands for N-methyl-glutamic acid
  MUTAGEN (2)..(2): Xaa stands for N-methyl-L-norleucine
  MUTAGEN (3)..(3): Xaa stands for alpha-methyl-alanine
  MUTAGEN (4)..(4): Xaa stands for beta-cyclohexyl-L-alanine
  MUTAGEN (5)..(5): Xaa stands for 4-fluoro-L-phenylalanine
  MUTAGEN (9)..(9): Xaa stands for (S)-2-amino-5-ureidopentanoic acid
  MUTAGEN (10)..(10): Xaa stands for D-lysine
  MUTAGEN (11)..(11): Xaa stands for beta-cyclohexyl-L-alanine
  MUTAGEN (13)..(13): Xaa stands for D-glutamic acid
  MOD_RES (13)..(13): AMIDATION
XXXXXPYYXXXCX

SEQ ID NO: 189 - protein, 13 aa, Artificial Sequence
  artificial peptide
  MUTAGEN (1)..(1): Xaa stands for 3-pyridyl-L-alanine
  MUTAGEN (2)..(2): Xaa stands for N-methyl-L-norleucine
  MUTAGEN (3)..(3): Xaa stands for alpha-methyl-alanine
  MUTAGEN (4)..(4): Xaa stands for beta-cyclohexyl-L-alanine
  MUTAGEN (5)..(5): Xaa stands for 4-fluoro-L-phenylalanine
  MUTAGEN (6)..(6): Xaa stands for 4-amino-1-(carboxymethyl)piperidin-4-carboxylic acid
  MUTAGEN (9)..(9): Xaa stands for 4-carboxy-L-phenylalanine
  MUTAGEN (10)..(10): Xaa stands for (S)-2-amino-3-(piperidin-4-yl)-propanoic acid
  MUTAGEN (11)..(11): Xaa stands for beta-cyclohexyl-L-alanine
  MUTAGEN (13)..(13): Xaa stands for D-glutamic acid
  MOD_RES (13)..(13): AMIDATION
XXXXXXYYXXXCX

SEQ ID NO: 190 - protein, 13 aa, Artificial Sequence
  artificial peptide
  MUTAGEN (1)..(1): Xaa stands for 3-pyridyl-L-alanine
  MUTAGEN (2)..(2): Xaa stands for N-methyl-L-norleucine
  MUTAGEN (3)..(3): Xaa stands for alpha-methyl-alanine
  MUTAGEN (4)..(4): Xaa stands for beta-cyclohexyl-L-alanine
  MUTAGEN (5)..(5): Xaa stands for 4-fluoro-L-phenylalanine
  MUTAGEN (6)..(6): Xaa stands for 2-methyl-serine
  MUTAGEN (9)..(9): Xaa stands for 4-carboxy-L-phenylalanine
  MUTAGEN (10)..(10): Xaa stands for (S)-2-amino-3-(piperidin-4-yl)-propanoic acid
  MUTAGEN (11)..(11): Xaa stands for beta-cyclohexyl-L-alanine
  MUTAGEN (13)..(13): Xaa stands for D-glutamic acid
  MOD_RES (13)..(13): AMIDATION
XXXXXXYYXXXCX

SEQ ID NO: 191 - protein, 13 aa, Artificial Sequence
  artificial peptide
  MUTAGEN (1)..(1): Xaa stands for 3-pyridyl-L-alanine
  MUTAGEN (2)..(2): Xaa stands for N-methyl-L-norleucine
  MUTAGEN (3)..(3): Xaa stands for alpha-methyl-alanine
  MUTAGEN (4)..(4): Xaa stands for alpha-methyl-alanine
  MUTAGEN (5)..(5): Xaa stands for 4-fluoro-L-phenylalanine
  MUTAGEN (6)..(6): Xaa stands for N-methyl-glycine
  MUTAGEN (9)..(9): Xaa stands for 4-carboxy-L-phenylalanine
  MUTAGEN (10)..(10): Xaa stands for (S)-2-amino-3-(piperidin-4-yl)-propanoic acid
  MUTAGEN (11)..(11): Xaa stands for beta-cyclohexyl-L-alanine
  MUTAGEN (13)..(13): Xaa stands for D-glutamic acid
  MOD_RES (13)..(13): AMIDATION
XXXXXXYYXXXCX

SEQ ID NO: 192 - protein, 13 aa, Artificial Sequence
  artificial peptide
  MUTAGEN (1)..(1): Xaa stands for 3-pyridyl-L-alanine
  MUTAGEN (2)..(2): Xaa stands for N-methyl-L-norleucine
  MUTAGEN (3)..(3): Xaa stands for alpha-methyl-alanine
  MUTAGEN (4)..(4): Xaa stands for beta-cyclohexyl-L-alanine
  MUTAGEN (5)..(5): Xaa stands for 4-fluoro-L-phenylalanine
  MUTAGEN (6)..(6): Xaa stands for N-methyl-D-glutamic acid
  MUTAGEN (9)..(9): Xaa stands for 4-carboxy-L-phenylalanine
  MUTAGEN (10)..(10): Xaa stands for (S)-2-amino-3-(piperidin-4-yl)-propanoic acid
  MUTAGEN (11)..(11): Xaa stands for beta-cyclohexyl-L-alanine
  MUTAGEN (13)..(13): Xaa stands for D-glutamic acid
  MOD_RES (13)..(13): AMIDATION
XXXXXXYYXXXCX

SEQ ID NO: 193 - protein, 13 aa, Artificial Sequence
  artificial peptide
  MUTAGEN (1)..(1): Xaa stands for 3-pyridyl-L-alanine
  MUTAGEN (2)..(2): Xaa stands for N-methyl-L-norleucine
  MUTAGEN (3)..(3): Xaa stands for alpha-methyl-alanine
  MUTAGEN (4)..(4): Xaa stands for beta-cyclohexyl-L-alanine
  MUTAGEN (5)..(5): Xaa stands for 4-fluoro-L-phenylalanine
  MUTAGEN (6)..(6): Xaa stands for N-methyl-D-aspartic acid
  MUTAGEN (9)..(9): Xaa stands for 4-carboxy-L-phenylalanine
  MUTAGEN (10)..(10): Xaa stands for (S)-2-amino-3-(piperidin-4-yl)-propanoic acid
  MUTAGEN (11)..(11): Xaa stands for beta-cyclohexyl-L-alanine
  MUTAGEN (13)..(13): Xaa stands for D-glutamic acid
  MOD_RES (13)..(13): AMIDATION
XXXXXXYYXXXCX

SEQ ID NO: 194 - protein, 13 aa, Artificial Sequence
  artificial peptide
  MUTAGEN (1)..(1): Xaa stands for 3-pyridyl-L-alanine
  MUTAGEN (2)..(2): Xaa stands for N-methyl-L-norleucine
  MUTAGEN (3)..(3): Xaa stands for alpha-methyl-alanine
  MUTAGEN (4)..(4): Xaa stands for beta-cyclohexyl-L-alanine
  MUTAGEN (5)..(5): Xaa stands for 4-fluoro-L-phenylalanine
  MUTAGEN (9)..(9): Xaa stands for 4-carboxy-L-phenylalanine
  MUTAGEN (10)..(10): Xaa stands for (S)-2-amino-3-(piperidin-4-yl)-propanoic acid
  MUTAGEN (11)..(11): Xaa stands for beta-cyclohexyl-L-alanine
  MUTAGEN (13)..(13): Xaa stands for D-glutamic acid
  MOD_RES (13)..(13): AMIDATION
XXXXXPYYXXXCX

SEQ ID NO: 195 - protein, 13 aa, Artificial Sequence
  artificial peptide
  MUTAGEN (1)..(1): Xaa stands for 3-pyridyl-L-alanine
  MUTAGEN (2)..(2): Xaa stands for N-methyl-L-norleucine
  MUTAGEN (3)..(3): Xaa stands for alpha-methyl-alanine
  MUTAGEN (4)..(4): Xaa stands for beta-cyclohexyl-L-alanine
  MUTAGEN (5)..(5): Xaa stands for 4-fluoro-L-phenylalanine
  MUTAGEN (6)..(6): Xaa stands for D-aspartic acid
  MUTAGEN (9)..(9): Xaa stands for 4-carboxy-L-phenylalanine
  MUTAGEN (10)..(10): Xaa stands for (S)-2-amino-3-(piperidin-4-yl)-propanoic acid
  MUTAGEN (11)..(11): Xaa stands for beta-cyclohexyl-L-alanine
  MUTAGEN (13)..(13): Xaa stands for D-glutamic acid
  MOD_RES (13)..(13): AMIDATION
XXXXXXYYXXXCX

SEQ ID NO: 196 - protein, 13 aa, Artificial Sequence
  artificial peptide
  MUTAGEN (1)..(1): Xaa stands for N-methyl-glutamic acid
  MUTAGEN (2)..(2): Xaa stands for N-methyl-L-norleucine
  MUTAGEN (3)..(3): Xaa stands for alpha-methyl-alanine
  MUTAGEN (4)..(4): Xaa stands for (S)-2-amino-3-(2,3-dihydro-1H-indene-2-yl)-propanoic acid
  MUTAGEN (5)..(5): Xaa stands for 4-fluoro-L-phenylalanine
  MUTAGEN (6)..(6): Xaa stands for 4-amino-1-(carboxymethyl)piperidin-4-carboxylic acid
  MUTAGEN (9)..(9): Xaa stands for 4-carboxy-L-phenylalanine
  MUTAGEN (10)..(10): Xaa stands for (S)-2-amino-3-(piperidin-4-yl)-propanoic acid
  MUTAGEN (11)..(11): Xaa stands for beta-cyclohexyl-L-alanine
  MUTAGEN (13)..(13): Xaa stands for D-glutamic acid
  MOD_RES (13)..(13): AMIDATION
XXXXXXYYXXXCX

SEQ ID NO: 197 - protein, 13 aa, Artificial Sequence
  artificial peptide
  MUTAGEN (1)..(1): Xaa stands for N-methyl-glutamic acid
  MUTAGEN (2)..(2): Xaa stands for N-methyl-L-norleucine
  MUTAGEN (3)..(3): Xaa stands for alpha-methyl-alanine
  MUTAGEN (4)..(4): Xaa stands for (S)-2-amino-3-(2,3-dihydro-1H-indene-2-yl)-propanoic acid
  MUTAGEN (5)..(5): Xaa stands for 4-fluoro-L-phenylalanine
  MUTAGEN (6)..(6): Xaa stands for 2-methyl-serine
  MUTAGEN (9)..(9): Xaa stands for 4-carboxy-L-phenylalanine
  MUTAGEN (10)..(10): Xaa stands for (S)-2-amino-3-(piperidin-4-yl)-propanoic acid
  MUTAGEN (11)..(11): Xaa stands for beta-cyclohexyl-L-alanine
  MUTAGEN (13)..(13): Xaa stands for D-glutamic acid
  MOD_RES (13)..(13): AMIDATION
XXXXXXYYXXXCX

SEQ ID NO: 198 - protein, 13 aa, Artificial Sequence
  artificial peptide
  MUTAGEN (1)..(1): Xaa stands for N-methyl-glutamic acid
  MUTAGEN (2)..(2): Xaa stands for N-methyl-L-norleucine
  MUTAGEN (3)..(3): Xaa stands for alpha-methyl-alanine
  MUTAGEN (4)..(4): Xaa stands for (S)-2-amino-3-(2,3-dihydro-1H-indene-2-yl)-propanoic acid
  MUTAGEN (5)..(5): Xaa stands for 4-fluoro-L-phenylalanine
  MUTAGEN (6)..(6): Xaa stands for N-methyl-glycine
  MUTAGEN (9)..(9): Xaa stands for 4-carboxy-L-phenylalanine
  MUTAGEN (10)..(10): Xaa stands for (S)-2-amino-3-(piperidin-4-yl)-propanoic acid
  MUTAGEN (11)..(11): Xaa stands for beta-cyclohexyl-L-alanine
  MUTAGEN (13)..(13): Xaa stands for D-glutamic acid
  MOD_RES (13)..(13): AMIDATION
XXXXXXYYXXXCX

SEQ ID NO: 199 - protein, 13 aa, Artificial Sequence
  artificial peptide
  MUTAGEN (1)..(1): Xaa stands for N-methyl-glutamic acid
  MUTAGEN (2)..(2): Xaa stands for N-methyl-L-norleucine
  MUTAGEN (3)..(3): Xaa stands for alpha-methyl-alanine
  MUTAGEN (4)..(4): Xaa stands for (S)-2-amino-3-(2,3-dihydro-1H-indene-2-yl)-propanoic acid
  MUTAGEN (5)..(5): Xaa stands for 4-fluoro-L-phenylalanine
  MUTAGEN (6)..(6): Xaa stands for N-methyl-D-glutamic acid
  MUTAGEN (9)..(9): Xaa stands for 4-carboxy-L-phenylalanine
  MUTAGEN (10)..(10): Xaa stands for (S)-2-amino-3-(piperidin-4-yl)-propanoic acid
  MUTAGEN (11)..(11): Xaa stands for beta-cyclohexyl-L-alanine
  MUTAGEN (13)..(13): Xaa stands for D-glutamic acid
  MOD_RES (13)..(13): AMIDATION
XXXXXXYYXXXCX

SEQ ID NO: 200 - protein, 13 aa, Artificial Sequence
  artificial peptide
  MUTAGEN (1)..(1): Xaa stands for N-methyl-glutamic acid
  MUTAGEN (2)..(2): Xaa stands for N-methyl-L-norleucine
  MUTAGEN (3)..(3): Xaa stands for alpha-methyl-alanine
  MUTAGEN (4)..(4): Xaa stands for (S)-2-amino-3-(2,3-dihydro-1H-indene-2-yl)-propanoic acid
  MUTAGEN (5)..(5): Xaa stands for 4-fluoro-L-phenylalanine
  MUTAGEN (6)..(6): Xaa stands for N-methyl-D-aspartic acid
  MUTAGEN (9)..(9): Xaa stands for 4-carboxy-L-phenylalanine
  MUTAGEN (10)..(10): Xaa stands for (S)-2-amino-3-(piperidin-4-yl)-propanoic acid
  MUTAGEN (11)..(11): Xaa stands for beta-cyclohexyl-L-alanine
  MUTAGEN (13)..(13): Xaa stands for D-glutamic acid
  MOD_RES (13)..(13): AMIDATION
XXXXXXYYXXXCX

SEQ ID NO: 201 - protein, 13 aa, Artificial Sequence
  artificial peptide
  MUTAGEN (1)..(1): Xaa stands for N-methyl-glutamic acid
  MUTAGEN (2)..(2): Xaa stands for N-methyl-L-norleucine
  MUTAGEN (3)..(3): Xaa stands for alpha-methyl-alanine
  MUTAGEN (4)..(4): Xaa stands for (S)-2-amino-3-(2,3-dihydro-1H-indene-2-yl)-propanoic acid
  MUTAGEN (5)..(5): Xaa stands for 4-fluoro-L-phenylalanine
  MUTAGEN (9)..(9): Xaa stands for 4-carboxy-L-phenylalanine
  MUTAGEN (10)..(10): Xaa stands for (S)-2-amino-3-(piperidin-4-yl)-propanoic acid
  MUTAGEN (11)..(11): Xaa stands for beta-cyclohexyl-L-alanine
  MUTAGEN (13)..(13): Xaa stands for D-glutamic acid
  MOD_RES (13)..(13): AMIDATION
XXXXXPYYXXXCX

SEQ ID NO: 202 - protein, 13 aa, Artificial Sequence
  artificial peptide
  MUTAGEN (1)..(1): Xaa stands for N-methyl-glutamic acid
  MUTAGEN (2)..(2): Xaa stands for N-methyl-L-norleucine
  MUTAGEN (3)..(3): Xaa stands for alpha-methyl-alanine
  MUTAGEN (4)..(4): Xaa stands for (S)-2-amino-3-(2,3-dihydro-1H-indene-2-yl)-propanoic acid
  MUTAGEN (5)..(5): Xaa stands for 4-fluoro-L-phenylalanine
  MUTAGEN (6)..(6): Xaa stands for D-aspartic acid
  MUTAGEN (9)..(9): Xaa stands for 4-carboxy-L-phenylalanine
  MUTAGEN (10)..(10): Xaa stands for (S)-2-amino-3-(piperidin-4-yl)-propanoic acid
  MUTAGEN (11)..(11): Xaa stands for beta-cyclohexyl-L-alanine
  MUTAGEN (13)..(13): Xaa stands for D-glutamic acid
  MOD_RES (13)..(13): AMIDATION
XXXXXXYYXXXCX

SEQ ID NO: 203 - protein, 13 aa, Artificial Sequence
  artificial peptide
  MUTAGEN (1)..(1): Xaa stands for N-methyl-glutamic acid
  MUTAGEN (2)..(2): Xaa stands for N-methyl-L-norleucine
  MUTAGEN (3)..(3): Xaa stands for alpha-methyl-alanine
  MUTAGEN (4)..(4): Xaa stands for beta-cyclohexyl-L-alanine
  MUTAGEN (5)..(5): Xaa stands for 4-fluoro-L-phenylalanine
  MUTAGEN (6)..(6): Xaa stands for 2-methyl-serine
  MUTAGEN (9)..(9): Xaa stands for 4-carboxy-L-phenylalanine
  MUTAGEN (10)..(10): Xaa stands for (S)-2-amino-3-(piperidin-4-yl)-propanoic acid
  MUTAGEN (11)..(11): Xaa stands for beta-cyclohexyl-L-alanine
  MUTAGEN (13)..(13): Xaa stands for D-glutamic acid
  MOD_RES (13)..(13): AMIDATION
XXXXXXYYXXXCX

SEQ ID NO: 204 - protein, 13 aa, Artificial Sequence
  artificial peptide
  MUTAGEN (1)..(1): Xaa stands for 3-pyridyl-L-alanine
  MUTAGEN (2)..(2): Xaa stands for N-methyl-L-norleucine
  MUTAGEN (3)..(3): Xaa stands for alpha-methyl-alanine
  MUTAGEN (4)..(4): Xaa stands for beta-cyclohexyl-L-alanine
  MUTAGEN (5)..(5): Xaa stands for 4-fluoro-L-phenylalanine
  MUTAGEN (6)..(6): Xaa stands for 4-amino-1-(carboxymethyl)piperidin-4-carboxylic acid
  MUTAGEN (9)..(9): Xaa stands for (S)-2-amino-5-ureidopentanoic acid
  MUTAGEN (10)..(10): Xaa stands for D-lysine
  MUTAGEN (11)..(11): Xaa stands for beta-cyclohexyl-L-alanine
  MUTAGEN (13)..(13): Xaa stands for D-glutamic acid
  MOD_RES (13)..(13): AMIDATION
XXXXXXYYXXXCX

SEQ ID NO: 205 - protein, 13 aa, Artificial Sequence
  artificial peptide
  MUTAGEN (1)..(1): Xaa stands for 3-pyridyl-L-alanine
  MUTAGEN (2)..(2): Xaa stands for N-methyl-L-norleucine
  MUTAGEN (3)..(3): Xaa stands for alpha-methyl-alanine
  MUTAGEN (4)..(4): Xaa stands for beta-cyclohexyl-L-alanine
  MUTAGEN (5)..(5): Xaa stands for 4-fluoro-L-phenylalanine
  MUTAGEN (6)..(6): Xaa stands for 2-methyl-serine
  MUTAGEN (9)..(9): Xaa stands for (S)-2-amino-5-ureidopentanoic acid
  MUTAGEN (10)..(10): Xaa stands for D-lysine
  MUTAGEN (11)..(11): Xaa stands for beta-cyclohexyl-L-alanine
  MUTAGEN (13)..(13): Xaa stands for D-glutamic acid
  MOD_RES (13)..(13): AMIDATION
XXXXXXYYXXXCX

SEQ ID NO: 206 - protein, 13 aa, Artificial Sequence
  artificial peptide
  MUTAGEN (1)..(1): Xaa stands for 3-pyridyl-L-alanine
  MUTAGEN (2)..(2): Xaa stands for N-methyl-L-norleucine
  MUTAGEN (3)..(3): Xaa stands for alpha-methyl-alanine
  MUTAGEN (4)..(4): Xaa stands for beta-cyclohexyl-L-alanine
  MUTAGEN (5)..(5): Xaa stands for 4-fluoro-L-phenylalanine
  MUTAGEN (6)..(6): Xaa stands for N-methyl-glycine
  MUTAGEN (9)..(9): Xaa stands for (S)-2-amino-5-ureidopentanoic acid
  MUTAGEN (10)..(10): Xaa stands for D-lysine
  MUTAGEN (11)..(11): Xaa stands for beta-cyclohexyl-L-alanine
  MUTAGEN (13)..(13): Xaa stands for D-glutamic acid
  MOD_RES (13)..(13): AMIDATION
XXXXXXYYXXXCX

SEQ ID NO: 207 - protein, 13 aa, Artificial Sequence
  artificial peptide
  MUTAGEN (1)..(1): Xaa stands for 3-pyridyl-L-alanine
  MUTAGEN (2)..(2): Xaa stands for N-methyl-L-norleucine
  MUTAGEN (3)..(3): Xaa stands for alpha-methyl-alanine
  MUTAGEN (4)..(4): Xaa stands for beta-cyclohexyl-L-alanine
  MUTAGEN (5)..(5): Xaa stands for 4-fluoro-L-phenylalanine
  MUTAGEN (6)..(6): Xaa stands for N-methyl-D-glutamic acid
  MUTAGEN (9)..(9): Xaa stands for (S)-2-amino-5-ureidopentanoic acid
  MUTAGEN (10)..(10): Xaa stands for D-lysine
  MUTAGEN (11)..(11): Xaa stands for beta-cyclohexyl-L-alanine
  MUTAGEN (13)..(13): Xaa stands for D-glutamic acid
  MOD_RES (13)..(13): AMIDATION
XXXXXXYYXXXCX

SEQ ID NO: 208 - protein, 13 aa, Artificial Sequence
  artificial peptide
  MUTAGEN (1)..(1): Xaa stands for 3-pyridyl-L-alanine
  MUTAGEN (2)..(2): Xaa stands for N-methyl-L-norleucine
  MUTAGEN (3)..(3): Xaa stands for alpha-methyl-alanine
  MUTAGEN (4)..(4): Xaa stands for beta-cyclohexyl-L-alanine
  MUTAGEN (5)..(5): Xaa stands for 4-fluoro-L-phenylalanine
  MUTAGEN (6)..(6): Xaa stands for N-methyl-D-aspartic acid
  MUTAGEN (9)..(9): Xaa stands for (S)-2-amino-5-ureidopentanoic acid
  MUTAGEN (10)..(10): Xaa stands for D-lysine
  MUTAGEN (11)..(11): Xaa stands for beta-cyclohexyl-L-alanine
  MUTAGEN (13)..(13): Xaa stands for D-glutamic acid
  MOD_RES (13)..(13): AMIDATION
XXXXXXYYXXXCX

SEQ ID NO: 209 - protein, 13 aa, Artificial Sequence
  artificial peptide
  MUTAGEN (1)..(1): Xaa stands for 3-pyridyl-L-alanine
  MUTAGEN (2)..(2): Xaa stands for N-methyl-L-norleucine
  MUTAGEN (3)..(3): Xaa stands for alpha-methyl-alanine
  MUTAGEN (4)..(4): Xaa stands for beta-cyclohexyl-L-alanine
  MUTAGEN (5)..(5): Xaa stands for 4-fluoro-L-phenylalanine
  MUTAGEN (9)..(9): Xaa stands for (S)-2-amino-5-ureidopentanoic acid
  MUTAGEN (10)..(10): Xaa stands for D-lysine
  MUTAGEN (11)..(11): Xaa stands for beta-cyclohexyl-L-alanine
  MUTAGEN (13)..(13): Xaa stands for D-glutamic acid
  MOD_RES (13)..(13): AMIDATION
XXXXXPYYXXXCX

SEQ ID NO: 210 - protein, 13 aa, Artificial Sequence
  artificial peptide
  MUTAGEN (1)..(1): Xaa stands for N-methyl-glutamic acid
  MUTAGEN (2)..(2): Xaa stands for N-methyl-L-norleucine
  MUTAGEN (3)..(3): Xaa stands for alpha-methyl-alanine
  MUTAGEN (4)..(4): Xaa stands for (S)-2-amino-3-(2,3-dihydro-1H-indene-2-yl)-propanoic acid
  MUTAGEN (5)..(5): Xaa stands for 4-fluoro-L-phenylalanine
  MUTAGEN (6)..(6): Xaa stands for 4-amino-1-(carboxymethyl)piperidin-4-carboxylic acid
  MUTAGEN (9)..(9): Xaa stands for (S)-2-amino-5-ureidopentanoic acid
  MUTAGEN (10)..(10): Xaa stands for D-lysine
  MUTAGEN (11)..(11): Xaa stands for beta-cyclohexyl-L-alanine
  MUTAGEN (13)..(13): Xaa stands for D-glutamic acid
  MOD_RES (13)..(13): AMIDATION
XXXXXXYYXXXCX

SEQ ID NO: 211 - protein, 13 aa, Artificial Sequence
  artificial peptide
  MUTAGEN (1)..(1): Xaa stands for N-methyl-glutamic acid
  MUTAGEN (2)..(2): Xaa stands for N-methyl-L-norleucine
  MUTAGEN (3)..(3): Xaa stands for alpha-methyl-alanine
  MUTAGEN (4)..(4): Xaa stands for (S)-2-amino-3-(2,3-dihydro-1H-indene-2-yl)-propanoic acid
  MUTAGEN (5)..(5): Xaa stands for 4-fluoro-L-phenylalanine
  MUTAGEN (6)..(6): Xaa stands for 2-methyl-serine
  MUTAGEN (9)..(9): Xaa stands for (S)-2-amino-5-ureidopentanoic acid
  MUTAGEN (10)..(10): Xaa stands for D-lysine
  MUTAGEN (11)..(11): Xaa stands for beta-cyclohexyl-L-alanine
  MUTAGEN (13)..(13): Xaa stands for D-glutamic acid
  MOD_RES (13)..(13): AMIDATION
XXXXXXYYXXXCX

SEQ ID NO: 212 - protein, 13 aa, Artificial Sequence
  artificial peptide
  MUTAGEN (1)..(1): Xaa stands for N-methyl-glutamic acid
  MUTAGEN (2)..(2): Xaa stands for N-methyl-L-norleucine
  MUTAGEN (3)..(3): Xaa stands for alpha-methyl-alanine
  MUTAGEN (4)..(4): Xaa stands for (S)-2-amino-3-(2,3-dihydro-1H-indene-2-yl)-propanoic acid
  MUTAGEN (5)..(5): Xaa stands for 4-fluoro-L-phenylalanine
  MUTAGEN (6)..(6): Xaa stands for N-methyl-glycine
  MUTAGEN (9)..(9): Xaa stands for (S)-2-amino-5-ureidopentanoic acid
  MUTAGEN (10)..(10): Xaa stands for D-lysine
  MUTAGEN (11)..(11): Xaa stands for beta-cyclohexyl-L-alanine
  MUTAGEN (13)..(13): Xaa stands for D-glutamic acid
  MOD_RES (13)..(13): AMIDATION
XXXXXXYYXXXCX

SEQ ID NO: 213 - protein, 13 aa, Artificial Sequence
  artificial peptide
  MUTAGEN (1)..(1): Xaa stands for N-methyl-glutamic acid
  MUTAGEN (2)..(2): Xaa stands for N-methyl-L-norleucine
  MUTAGEN (3)..(3): Xaa stands for alpha-methyl-alanine
  MUTAGEN (4)..(4): Xaa stands for (S)-2-amino-3-(2,3-dihydro-1H-indene-2-yl)-propanoic acid
  MUTAGEN (5)..(5): Xaa stands for 4-fluoro-L-phenylalanine
  MUTAGEN (6)..(6): Xaa stands for N-methyl-D-glutamic acid
  MUTAGEN (9)..(9): Xaa stands for (S)-2-amino-5-ureidopentanoic acid
  MUTAGEN (10)..(10): Xaa stands for D-lysine
  MUTAGEN (11)..(11): Xaa stands for beta-cyclohexyl-L-alanine
  MUTAGEN (13)..(13): Xaa stands for D-glutamic acid
  MOD_RES (13)..(13): AMIDATION
XXXXXXYYXXXCX

SEQ ID NO: 214 - protein, 13 aa, Artificial Sequence
  artificial peptide
  MUTAGEN (1)..(1): Xaa stands for N-methyl-glutamic acid
  MUTAGEN (2)..(2): Xaa stands for N-methyl-L-norleucine
  MUTAGEN (3)..(3): Xaa stands for alpha-methyl-alanine
  MUTAGEN (4)..(4): Xaa stands for (S)-2-amino-3-(2,3-dihydro-1H-indene-2-yl)-propanoic acid
  MUTAGEN (5)..(5): Xaa stands for 4-fluoro-L-phenylalanine
  MUTAGEN (6)..(6): Xaa stands for N-methyl-D-aspartic acid
  MUTAGEN (9)..(9): Xaa stands for (S)-2-amino-5-ureidopentanoic acid
  MUTAGEN (10)..(10): Xaa stands for D-lysine
  MUTAGEN (11)..(11): Xaa stands for beta-cyclohexyl-L-alanine
  MUTAGEN (13)..(13): Xaa stands for D-glutamic acid
  MOD_RES (13)..(13): AMIDATION
XXXXXXYYXXXCX

SEQ ID NO: 215 - protein, 13 aa, Artificial Sequence
  artificial peptide
  MUTAGEN (1)..(1): Xaa stands for N-methyl-glutamic acid
  MUTAGEN (2)..(2): Xaa stands for N-methyl-L-norleucine
  MUTAGEN (3)..(3): Xaa stands for alpha-methyl-alanine
  MUTAGEN (4)..(4): Xaa stands for (S)-2-amino-3-(2,3-dihydro-1H-indene-2-yl)-propanoic acid
  MUTAGEN (5)..(5): Xaa stands for 4-fluoro-L-phenylalanine
  MUTAGEN (9)..(9): Xaa stands for (S)-2-amino-5-ureidopentanoic acid
  MUTAGEN (10)..(10): Xaa stands for D-lysine
  MUTAGEN (11)..(11): Xaa stands for beta-cyclohexyl-L-alanine
  MUTAGEN (13)..(13): Xaa stands for D-glutamic acid
  MOD_RES (13)..(13): AMIDATION
XXXXXPYYXXXCX

SEQ ID NO: 216 - protein, 13 aa, Artificial Sequence
  artificial peptide
  MUTAGEN (1)..(1): Xaa stands for N-methyl-glutamic acid
  MUTAGEN (2)..(2): Xaa stands for N-methyl-L-norleucine
  MUTAGEN (3)..(3): Xaa stands for alpha-methyl-alanine
  MUTAGEN (4)..(4): Xaa stands for beta-cyclohexyl-L-alanine
  MUTAGEN (5)..(5): Xaa stands for 4-fluoro-L-phenylalanine
  MUTAGEN (6)..(6): Xaa stands for 2-methyl-serine
  MUTAGEN (9)..(9): Xaa stands for (S)-2-amino-5-ureidopentanoic acid
  MUTAGEN (10)..(10): Xaa stands for D-lysine
  MUTAGEN (11)..(11): Xaa stands for beta-cyclohexyl-L-alanine
  MUTAGEN (13)..(13): Xaa stands for D-glutamic acid
  MOD_RES (13)..(13): AMIDATION
XXXXXXYYXXXCX

SEQ ID NO: 217 - protein, 13 aa, Artificial Sequence
  artificial peptide
  MUTAGEN (1)..(1): Xaa stands for N-methyl-glutamic acid
  MUTAGEN (2)..(2): Xaa stands for N-methyl-L-norleucine
  MUTAGEN (3)..(3): Xaa stands for alpha-methyl-alanine
  MUTAGEN (4)..(4): Xaa stands for beta-cyclohexyl-L-alanine
  MUTAGEN (5)..(5): Xaa stands for 4-fluoro-L-phenylalanine
  MUTAGEN (6)..(6): Xaa stands for N-methyl-D-aspartic acid
  MUTAGEN (9)..(9): Xaa stands for (S)-2-amino-5-ureidopentanoic acid
  MUTAGEN (10)..(10): Xaa stands for D-lysine
  MUTAGEN (11)..(11): Xaa stands for beta-cyclohexyl-L-alanine
  MUTAGEN (13)..(13): Xaa stands for D-glutamic acid
XXXXXXYYXXXCX

SEQ ID NO: 218 - protein, 13 aa, Artificial Sequence
  artificial peptide
  MUTAGEN (1)..(1): Xaa stands for N-methyl-glutamic acid
  MUTAGEN (2)..(2): Xaa stands for N-methyl-L-norleucine
  MUTAGEN (3)..(3): Xaa stands for alpha-methyl-alanine
  MUTAGEN (4)..(4): Xaa stands for beta-cyclohexyl-L-alanine
  MUTAGEN (5)..(5): Xaa stands for 4-fluoro-L-phenylalanine
  MUTAGEN (6)..(6): Xaa stands for D-glutamic acid
  MUTAGEN (9)..(9): Xaa stands for (S)-2-amino-5-ureidopentanoic acid
  MUTAGEN (10)..(10): Xaa stands for D-lysine
  MUTAGEN (11)..(11): Xaa stands for beta-cyclohexyl-L-alanine
  MUTAGEN (13)..(13): Xaa stands for D-glutamic acid
XXXXXXYYXXXCX